European Patent Application EP 4 574 975 A1, published June 25, 2025. Title: COMPOSITIONS AND METHODS FOR DELIVERING TRANSGENES. Applicant: Bayer AG. The sequence listing filed with the application follows.

SEQUENCE LISTING (186 sequences)

SEQ ID NO: 1 - DNA, 23 bp, synthetic construct
  misc_feature 1..23: note = spacer sequence for B-Gen.1 human albumin target 1
  source 1..23: mol_type = other DNA
ttctattgttcaacttttattct

SEQ ID NO: 2 - DNA, 23 bp, synthetic construct
  misc_feature 1..23: note = spacer sequence for B-Gen.1 human albumin target 2
  source 1..23: mol_type = other DNA
ttcaacttttattctattttccc

SEQ ID NO: 3 - DNA, 23 bp, synthetic construct
  misc_feature 1..23: note = spacer sequence for B-Gen.1 human albumin target 3
  source 1..23: mol_type = other DNA
tattttcccagtaaaataaagtt

SEQ ID NO: 4 - DNA, 23 bp, synthetic construct
  misc_feature 1..23: note = spacer sequence for B-Gen.1 human albumin target 4
  source 1..23: mol_type = other DNA
tcccagtaaaataaagttttagt

SEQ ID NO: 5 - DNA, 23 bp, synthetic construct
  misc_feature 1..23: note = spacer sequence for B-Gen.1 human albumin target 5
  source 1..23: mol_type = other DNA
tactgggaaaatagaataaaagt

SEQ ID NO: 6 - DNA, 23 bp, synthetic construct
  misc_feature 1..23: note = spacer sequence for B-Gen.1 human albumin target 6
  source 1..23: mol_type = other DNA
tttaaagatgcagagtttactaa

SEQ ID NO: 7 - DNA, 23 bp, synthetic construct
  misc_feature 1..23: note = spacer sequence for B-Gen.1 human albumin target 7
  source 1..23: mol_type = other DNA
ttttggcatttatttctaaaatg

SEQ ID NO: 8 - DNA, 23 bp, synthetic construct
  misc_feature 1..23: note = spacer sequence for B-Gen.1 human albumin target 8
  source 1..23: mol_type = other DNA
tggcatttatttctaaaatggca

SEQ ID NO: 9 - DNA, 23 bp, synthetic construct
  misc_feature 1..23: note = spacer sequence for B-Gen.1 human albumin target 9
  source 1..23: mol_type = other DNA
atttctaaaatggcatagtattt

SEQ ID NO: 10 - DNA, 23 bp, synthetic construct
  misc_feature 1..23: note = spacer sequence for B-Gen.1 human albumin target 10
  source 1..23: mol_type = other DNA
ctaaaatggcatagtattttgta

SEQ ID NO: 11 - DNA, 23 bp, synthetic construct
  misc_feature 1..23: note = spacer sequence for B-Gen.1 human albumin target 11
  source 1..23: mol_type = other DNA
tagaaataaatgccaaaataatt

SEQ ID NO: 12 - DNA, 23 bp, synthetic construct
  misc_feature 1..23: note = spacer sequence for B-Gen.1 human albumin target 12
  source 1..23: mol_type = other DNA
tgtatttgtgaagtcttacaagg

SEQ ID NO: 13 - DNA, 23 bp, synthetic construct
  misc_feature 1..23: note = spacer sequence for B-Gen.1 human albumin target 13
  source 1..23: mol_type = other DNA
gtgaagtcttacaaggttatctt

SEQ ID NO: 14 - DNA, 23 bp, synthetic construct
  misc_feature 1..23: note = spacer sequence for B-Gen.1 human albumin target 14
  source 1..23: mol_type = other DNA
ataaaattcaaacatcctaggta

SEQ ID NO: 15 - DNA, 23 bp, synthetic construct
  misc_feature 1..23: note = spacer sequence for B-Gen.1 human albumin target 15
  source 1..23: mol_type = other DNA
ataagataaccttgtaagacttc

SEQ ID NO: 16 - DNA, 23 bp, synthetic construct
  misc_feature 1..23: note = spacer sequence for B-Gen.1 human albumin target 16
  source 1..23: mol_type = other DNA
tgacctttttttttttttaccta

SEQ ID NO: 17 - DNA, 23 bp, synthetic construct
  misc_feature 1..23: note = spacer sequence for B-Gen.1 human albumin target 17
  source 1..23: mol_type = other DNA
tttagtgactgtaattttctttt

SEQ ID NO: 18 - DNA, 23 bp, synthetic construct
  misc_feature 1..23: note = spacer sequence for B-Gen.1 human albumin target 18
  source 1..23: mol_type = other DNA
cagtcactaaacaattctgacct

SEQ ID NO: 19 - DNA, 23 bp, synthetic construct
  misc_feature 1..23: note = spacer sequence for B-Gen.1 human albumin target 19
  source 1..23: mol_type = other DNA
tcttttgcgcactaaggaaagtg

SEQ ID NO: 20 - DNA, 23 bp, synthetic construct
  misc_feature 1..23: note = spacer sequence for B-Gen.1 human albumin target 20
  source 1..23: mol_type = other DNA
tgtgaagtttcagtcactctaag

SEQ ID NO: 21 - DNA, 23 bp, synthetic construct
  misc_feature 1..23: note = spacer sequence for B-Gen.1 human albumin target 21
  source 1..23: mol_type = other DNA
aattcataactatcccaaagacc

SEQ ID NO: 22 - DNA, 23 bp, synthetic construct
  misc_feature 1..23: note = spacer sequence for B-Gen.1 human albumin target 22
  source 1..23: mol_type = other DNA
aatcttcaaccctattctgtgaa

SEQ ID NO: 23 - DNA, 23 bp, synthetic construct
  misc_feature 1..23: note = spacer sequence for B-Gen.1 human albumin target 23
  source 1..23: mol_type = other DNA
ataactatcccaaagacctatcc

SEQ ID NO: 24 - DNA, 23 bp, synthetic construct
  misc_feature 1..23: note = spacer sequence for B-Gen.1 human albumin target 24
  source 1..23: mol_type = other DNA
cactatgctttatttaaaaacca

SEQ ID NO: 25 - DNA, 23 bp, synthetic construct
  misc_feature 1..23: note = spacer sequence for B-Gen.1 human albumin target 25
  source 1..23: mol_type = other DNA
aaaaaccacaaaacctgtgctgt

SEQ ID NO: 26 - DNA, 23 bp, synthetic construct
  misc_feature 1..23: note = spacer sequence for B-Gen.1 human albumin target 26
  source 1..23: mol_type = other DNA
atgagatcaacagcacaggtttt

SEQ ID NO: 27 - DNA, 23 bp, synthetic construct
  misc_feature 1..23: note = spacer sequence for B-Gen.1 human albumin target 27
  source 1..23: mol_type = other DNA
atatttattttcattttagtctg

SEQ ID NO: 28 - DNA, 23 bp, synthetic construct
  misc_feature 1..23: note = spacer sequence for B-Gen.1 human albumin target 28
  source 1..23: mol_type = other DNA
attttcattttagtctgtcttct

SEQ ID NO: 29 - DNA, 23 bp, synthetic construct
  misc_feature 1..23: note = spacer sequence for B-Gen.1 human albumin target 29
  source 1..23: mol_type = other DNA
tcattttagtctgtcttcttggt

SEQ ID NO: 30 - DNA, 23 bp, synthetic construct
  misc_feature 1..23: note = spacer sequence for B-Gen.1 human albumin target 30
  source 1..23: mol_type = other DNA
tagtctgtcttcttggttgctgt

SEQ ID NO: 31 - DNA, 23 bp, synthetic construct
  misc_feature 1..23: note = spacer sequence for B-Gen.1 human albumin target 31
  source 1..23: mol_type = other DNA
gatattatctaagtttgaatata

SEQ ID NO: 32 - DNA, 23 bp, synthetic construct
  misc_feature 1..23: note = spacer sequence for B-Gen.1 human albumin target 32
  source 1..23: mol_type = other DNA
tctaagtttgaatataaggctat

SEQ ID NO: 33 - DNA, 23 bp, synthetic construct
  misc_feature 1..23: note = spacer sequence for B-Gen.1 human albumin target 33
  source 1..23: mol_type = other DNA
atagccttatattcaaacttaga

SEQ ID NO: 34 - DNA, 23 bp, synthetic construct
  misc_feature 1..23: note = spacer sequence for B-Gen.1 human albumin target 34
  source 1..23: mol_type = other DNA
aataatttttaaaatagtattct

SEQ ID NO: 35 - DNA, 23 bp, synthetic construct
  misc_feature 1..23: note = spacer sequence for B-Gen.1 human albumin target 35
  source 1..23: mol_type = other DNA
aatatttatagccttatattcaa

SEQ ID NO: 36 - DNA, 23 bp, synthetic construct
  misc_feature 1..23: note = spacer sequence for B-Gen.1 human albumin target 36
  source 1..23: mol_type = other DNA
ttaaatatttatagccttatatt

SEQ ID NO: 37 - DNA, 23 bp, synthetic construct
  misc_feature 1..23: note = spacer sequence for B-Gen.1 human albumin target 37
  source 1..23: mol_type = other DNA
ttaaaatagtattcttggtaatt

SEQ ID NO: 38 - DNA, 23 bp, synthetic construct
  misc_feature 1..23: note = spacer sequence for B-Gen.1 human albumin target 38
  source 1..23: mol_type = other DNA
taaaaattattaaatatttatag

SEQ ID NO: 39 - DNA, 23 bp, synthetic construct
  misc_feature 1..23: note = spacer sequence for B-Gen.1 human albumin target 39
  source 1..23: mol_type = other DNA
ttggtaattgaattattcttctg

SEQ ID NO: 40 - DNA, 23 bp, synthetic construct
  misc_feature 1..23: note = spacer sequence for B-Gen.1 human albumin target 40
  source 1..23: mol_type = other DNA
ccaagaatactattttaaaaatt

SEQ ID NO: 41 - DNA, 23 bp, synthetic construct
  misc_feature 1..23: note = spacer sequence for B-Gen.1 human albumin target 41
  source 1..23: mol_type = other DNA
aattattcttctgtttaaaggca

SEQ ID NO: 42 - DNA, 23 bp, synthetic construct
  misc_feature 1..23: note = spacer sequence for B-Gen.1 human albumin target 42
  source 1..23: mol_type = other DNA
aattaccaagaatactattttaa

SEQ ID NO: 43 - DNA, 23 bp, synthetic construct
  misc_feature 1..23: note = spacer sequence for B-Gen.1 human albumin target 43
  source 1..23: mol_type = other DNA
ttcttctgtttaaaggcagaaga

SEQ ID NO: 44 - DNA, 23 bp, synthetic construct
  misc_feature 1..23: note = spacer sequence for B-Gen.1 human albumin target 44
  source 1..23: mol_type = other DNA
ttctgtttaaaggcagaagaaat

SEQ ID NO: 45 - DNA, 23 bp, synthetic construct
  misc_feature 1..23: note = spacer sequence for B-Gen.1 human albumin target 45
  source 1..23: mol_type = other DNA
cttctgcctttaaacagaagaat

SEQ ID NO: 46 - DNA, 23 bp, synthetic construct
  misc_feature 1..23: note = spacer sequence for B-Gen.1 human albumin target 46
  source 1..23: mol_type = other DNA
tttcttctgcctttaaacagaag

SEQ ID NO: 47 - DNA, 23 bp, synthetic construct
  misc_feature 1..23: note = spacer sequence for B-Gen.1 human albumin target 47
  source 1..23: mol_type = other DNA
aacatcatcctgagtttttctgt

SEQ ID NO: 48 - DNA, 23 bp, synthetic construct
  misc_feature 1..23: note = spacer sequence for B-Gen.1 human albumin target 48
  source 1..23: mol_type = other DNA
ctacagaaaaactcaggatgatg

SEQ ID NO: 49 - DNA, 23 bp, synthetic construct
  misc_feature 1..23: note = spacer sequence for B-Gen.1 human albumin target 49
  source 1..23: mol_type = other DNA
ggctctgattcctacagaaaaac

SEQ ID NO: 50 - DNA, 23 bp, synthetic construct
  misc_feature 1..23: note = spacer sequence for B-Gen.1 human albumin target 50
  source 1..23: mol_type = other DNA
tgaaacaaatgcataatctaagt

SEQ ID NO: 51 - DNA, 23 bp, synthetic construct
  misc_feature 1..23: note = spacer sequence for B-Gen.1 human albumin target 51
  source 1..23: mol_type = other DNA
gtttcaaaatattgggctctgat

SEQ ID NO: 52 - DNA, 23 bp, synthetic construct
  misc_feature 1..23: note = spacer sequence for B-Gen.1 human albumin target 52
  source 1..23: mol_type = other DNA
tgcatttgtttcaaaatattggg

SEQ ID NO: 53 - DNA, 23 bp, synthetic construct
  misc_feature 1..23: note = spacer sequence for B-Gen.1 human albumin target 53
  source 1..23: mol_type = other DNA
ctttccatttgacttagattatg

SEQ ID NO: 54 - DNA, 23 bp, synthetic construct
  misc_feature 1..23: note = spacer sequence for B-Gen.1 human albumin target 54
  source 1..23: mol_type = other DNA
ttacttcttgttttcttcagtat

SEQ ID NO: 55 - DNA, 23 bp, synthetic construct
  misc_feature 1..23: note = spacer sequence for B-Gen.1 human albumin target 55
  source 1..23: mol_type = other DNA
cttcttgttttcttcagtattta

SEQ ID NO: 56 - DNA, 23 bp, synthetic construct
  misc_feature 1..23: note = spacer sequence for B-Gen.1 human albumin target 56
  source 1..23: mol_type = other DNA
aacaatccttttttttcttccct

SEQ ID NO: 57 - DNA, 23 bp, synthetic construct
  misc_feature 1..23: note = spacer sequence for B-Gen.1 human albumin target 57
  source 1..23: mol_type = other DNA
ttaaatactgaagaaaacaagaa

SEQ ID NO: 58 - DNA, 23 bp, synthetic construct
  misc_feature 1..23: note = spacer sequence for B-Gen.1 human albumin target 58
  source 1..23: mol_type = other DNA
aaacatcctaggtaaaaaaaaaa

SEQ ID NO: 59 - DNA, 23 bp, synthetic construct
  misc_feature 1..23: note = spacer sequence for B-Gen.1 human albumin target 59
  source 1..23: mol_type = other DNA
tattaataagataaccttgtaag

SEQ ID NO: 60 - DNA, 23 bp, synthetic construct
  misc_feature 1..23: note = spacer sequence for B-Gen.1 human albumin target 60
  source 1..23: mol_type = other DNA
aaacttagataatatctaatact

SEQ ID NO: 61 - DNA, 23 bp, synthetic construct
  misc_feature 1..23: note = spacer sequence for B-Gen.1 human albumin target 61
  source 1..23: mol_type = other DNA
gacttagattatgcatttgtttc

SEQ ID NO: 62 - RNA, 132 nt, synthetic construct
  misc_feature 1..132: note = gRNA sequence for B-GEn.1 human albumin target 1
  source 1..132: mol_type = other RNA
ctggatataataaagatgtttagctataggctaataagatagttgtgtcaagtgcttcggagacctaacacgtcatccagtcacaacggctatctatatttccactaacttctattgttcaacttttattct

SEQ ID NO: 63 - RNA, 132 nt, synthetic construct
  misc_feature 1..132: note = gRNA sequence for B-GEn.1 human albumin target 2
  source 1..132: mol_type = other RNA
ctggatataataaagatgtttagctataggctaataagatagttgtgtcaagtgcttcggagacctaacacgtcatccagtcacaacggctatctatatttccactaacttcaacttttattctattttccc

SEQ ID NO: 64 - RNA, 132 nt, synthetic construct
  misc_feature 1..132: note = gRNA sequence for B-GEn.1 human albumin target 3
  source 1..132: mol_type = other RNA
ctggatataataaagatgtttagctataggctaataagatagttgtgtcaagtgcttcggagacctaacacgtcatccagtcacaacggctatctatatttccactaactattttcccagtaaaataaagtt

SEQ ID NO: 65 - RNA, 132 nt, synthetic construct
  misc_feature 1..132: note = gRNA sequence for B-GEn.1 human albumin target 4
  source 1..132: mol_type = other RNA
ctggatataataaagatgtttagctataggctaataagatagttgtgtcaagtgcttcggagacctaacacgtcatccagtcacaacggctatctatatttccactaactcccagtaaaataaagttttagt

SEQ ID NO: 66 - RNA, 132 nt, synthetic construct
  misc_feature 1..132: note = gRNA sequence for B-GEn.1 human albumin target 5
  source 1..132: mol_type = other RNA
ctggatataataaagatgtttagctataggctaataagatagttgtgtcaagtgcttcggagacctaacacgtcatccagtcacaacggctatctatatttccactaactactgggaaaatagaataaaagt

SEQ ID NO: 67 - RNA, 132 nt, synthetic construct
  misc_feature 1..132: note = gRNA sequence for B-GEn.1 human albumin target 6
  source 1..132: mol_type = other RNA
ctggatataataaagatgtttagctataggctaataagatagttgtgtcaagtgcttcggagacctaacacgtcatccagtcacaacggctatctatatttccactaactttaaagatgcagagtttactaa

SEQ ID NO: 68 - RNA, 132 nt, synthetic construct
  misc_feature 1..132: note = gRNA sequence for B-GEn.1 human albumin target 7
  source 1..132: mol_type = other RNA
ctggatataataaagatgtttagctataggctaataagatagttgtgtcaagtgcttcggagacctaacacgtcatccagtcacaacggctatctatatttccactaacttttggcatttatttctaaaatg

SEQ ID NO: 69 - RNA, 132 nt, synthetic construct
  misc_feature 1..132: note = gRNA sequence for B-GEn.1 human albumin target 8
  source 1..132: mol_type = other RNA
ctggatataataaagatgtttagctataggctaataagatagttgtgtcaagtgcttcggagacctaacacgtcatccagtcacaacggctatctatatttccactaactggcatttatttctaaaatggca

SEQ ID NO: 70 - RNA, 132 nt, synthetic construct
  misc_feature 1..132: note = gRNA sequence for B-GEn.1 human albumin target 9
  source 1..132: mol_type = other RNA
ctggatataataaagatgtttagctataggctaataagatagttgtgtcaagtgcttcggagacctaacacgtcatccagtcacaacggctatctatatttccactaacatttctaaaatggcatagtattt

SEQ ID NO: 71 - RNA, 132 nt, synthetic construct
  misc_feature 1..132: note = gRNA sequence for B-GEn.1 human albumin target 10
  source 1..132: mol_type = other RNA
ctggatataataaagatgtttagctataggctaataagatagttgtgtcaagtgcttcggagacctaacacgtcatccagtcacaacggctatctatatttccactaacctaaaatggcatagtattttgta

SEQ ID NO: 72 - RNA, 132 nt, synthetic construct
  misc_feature 1..132: note = gRNA sequence for B-GEn.1 human albumin target 11
  source 1..132: mol_type = other RNA
ctggatataataaagatgtttagctataggctaataagatagttgtgtcaagtgcttcggagacctaacacgtcatccagtcacaacggctatctatatttccactaactagaaataaatgccaaaataatt

SEQ ID NO: 73 - RNA, 132 nt, synthetic construct
  misc_feature 1..132: note = gRNA sequence for B-GEn.1 human albumin target 12
  source 1..132: mol_type = other RNA
ctggatataataaagatgtttagctataggctaataagatagttgtgtcaagtgcttcggagacctaacacgtcatccagtcacaacggctatctatatttccactaactgtatttgtgaagtcttacaagg

SEQ ID NO: 74 - RNA, 132 nt, synthetic construct
  misc_feature 1..132: note = gRNA sequence for B-GEn.1 human albumin target 13
  source 1..132: mol_type = other RNA
ctggatataataaagatgtttagctataggctaataagatagttgtgtcaagtgcttcggagacctaacacgtcatccagtcacaacggctatctatatttccactaacgtgaagtcttacaaggttatctt

SEQ ID NO: 75 - RNA, 132 nt, synthetic construct
  misc_feature 1..132: note = gRNA sequence for B-GEn.1 human albumin target 14
  source 1..132: mol_type = other RNA
ctggatataataaagatgtttagctataggctaataagatagttgtgtcaagtgcttcggagacctaacacgtcatccagtcacaacggctatctatatttccactaacataaaattcaaacatcctaggta

SEQ ID NO: 76 - RNA, 132 nt, synthetic construct
  misc_feature 1..132: note = gRNA sequence for B-GEn.1 human albumin target 15
  source 1..132: mol_type = other RNA
ctggatataataaagatgtttagctataggctaataagatagttgtgtcaagtgcttcggagacctaacacgtcatccagtcacaacggctatctatatttccactaacataagataaccttgtaagacttc

SEQ ID NO: 77 - RNA, 132 nt, synthetic construct
  misc_feature 1..132: note = gRNA sequence for B-GEn.1 human albumin target 16
  source 1..132: mol_type = other RNA
ctggatataataaagatgtttagctataggctaataagatagttgtgtcaagtgcttcggagacctaacacgtcatccagtcacaacggctatctatatttccactaactgacctttttttttttttaccta

SEQ ID NO: 78 - RNA, 132 nt, synthetic construct
  misc_feature 1..132: note = gRNA sequence for B-GEn.1 human albumin target 17
  source 1..132: mol_type = other RNA
ctggatataataaagatgtttagctataggctaataagatagttgtgtcaagtgcttcggagacctaacacgtcatccagtcacaacggctatctatatttccactaactttagtgactgtaattttctttt

SEQ ID NO: 79 - RNA, 132 nt, synthetic construct
  misc_feature 1..132: note = gRNA sequence for B-GEn.1 human albumin target 18
  source 1..132: mol_type = other RNA
ctggatataataaagatgtttagctataggctaataagatagttgtgtcaagtgcttcggagacctaacacgtcatccagtcacaacggctatctatatttccactaaccagtcactaaacaattctgacct

SEQ ID NO: 80 - RNA, 132 nt, synthetic construct
  misc_feature 1..132: note = gRNA sequence for B-GEn.1 human albumin target 19
  source 1..132: mol_type = other RNA
ctggatataataaagatgtttagctataggctaataagatagttgtgtcaagtgcttcggagacctaacacgtcatccagtcacaacggctatctatatttccactaactcttttgcgcactaaggaaagtg

SEQ ID NO: 81 - RNA, 132 nt, synthetic construct
  misc_feature 1..132: note = gRNA sequence for B-GEn.1 human albumin target 20
  source 1..132: mol_type = other RNA
ctggatataataaagatgtttagctataggctaataagatagttgtgtcaagtgcttcggagacctaacacgtcatccagtcacaacggctatctatatttccactaactgtgaagtttcagtcactctaag

SEQ ID NO: 82 - RNA, 132 nt, synthetic construct
  misc_feature 1..132: note = gRNA sequence for B-GEn.1 human albumin target 21
  source 1..132: mol_type = other RNA
ctggatataataaagatgtttagctataggctaataagatagttgtgtcaagtgcttcggagacctaacacgtcatccagtcacaacggctatctatatttccactaacaattcataactatcccaaagacc

SEQ ID NO: 83 - RNA, 132 nt, synthetic construct
  misc_feature 1..132: note = gRNA sequence for B-GEn.1 human albumin target 22
  source 1..132: mol_type = other RNA
ctggatataataaagatgtttagctataggctaataagatagttgtgtcaagtgcttcggagacctaacacgtcatccagtcacaacggctatctatatttccactaacaatcttcaaccctattctgtgaa

SEQ ID NO: 84 - RNA, 132 nt, synthetic construct
  misc_feature 1..132: note = gRNA sequence for B-GEn.1 human albumin target 23
  source 1..132: mol_type = other RNA
ctggatataataaagatgtttagctataggctaataagatagttgtgtcaagtgcttcggagacctaacacgtcatccagtcacaacggctatctatatttccactaacataactatcccaaagacctatcc

SEQ ID NO: 85 - RNA, 132 nt, synthetic construct
  misc_feature 1..132: note = gRNA sequence for B-GEn.1 human albumin target 24
  source 1..132: mol_type = other RNA
ctggatataataaagatgtttagctataggctaataagatagttgtgtcaagtgcttcggagacctaacacgtcatccagtcacaacggctatctatatttccactaaccactatgctttatttaaaaacca

SEQ ID NO: 86 - RNA, 132 nt, synthetic construct
  misc_feature 1..132: note = gRNA sequence for B-GEn.1 human albumin target 25
  source 1..132: mol_type = other RNA
ctggatataataaagatgtttagctataggctaataagatagttgtgtcaagtgcttcggagacctaacacgtcatccagtcacaacggctatctatatttccactaacaaaaaccacaaaacctgtgctgt

SEQ ID NO: 87 - RNA, 132 nt, synthetic construct
  misc_feature 1..132: note = gRNA sequence for B-GEn.1 human albumin target 26
  source 1..132: mol_type = other RNA
ctggatataataaagatgtttagctataggctaataagatagttgtgtcaagtgcttcggagacctaacacgtcatccagtcacaacggctatctatatttccactaacatgagatcaacagcacaggtttt

SEQ ID NO: 88 - RNA, 132 nt, synthetic construct
  misc_feature 1..132: note = gRNA sequence for B-GEn.1 human albumin target 27
  source 1..132: mol_type = other RNA
ctggatataataaagatgtttagctataggctaataagatagttgtgtcaagtgcttcggagacctaacacgtcatccagtcacaacggctatctatatttccactaacatatttattttcattttagtctg

SEQ ID NO: 89 - RNA, 132 nt, synthetic construct
  misc_feature 1..132: note = gRNA sequence for B-GEn.1 human albumin target 28
  source 1..132: mol_type = other RNA
ctggatataataaagatgtttagctataggctaataagatagttgtgtcaagtgcttcggagacctaacacgtcatccagtcacaacggctatctatatttccactaacattttcattttagtctgtcttct

SEQ ID NO: 90 - RNA, 132 nt, synthetic construct
  misc_feature 1..132: note = gRNA sequence for B-GEn.1 human albumin target 29
  source 1..132: mol_type = other RNA
ctggatataataaagatgtttagctataggctaataagatagttgtgtcaagtgcttcggagacctaacacgtcatccagtcacaacggctatctatatttccactaactcattttagtctgtcttcttggt

SEQ ID NO: 91 - RNA, 132 nt, synthetic construct
  misc_feature 1..132: note = gRNA sequence for B-GEn.1 human albumin target 30
  source 1..132: mol_type = other RNA
ctggatataataaagatgtttagctataggctaataagatagttgtgtcaagtgcttcggagacctaacacgtcatccagtcacaacggctatctatatttccactaactagtctgtcttcttggttgctgt

SEQ ID NO: 92 - RNA, 132 nt, synthetic construct
  misc_feature 1..132: note = gRNA sequence for B-GEn.1 human albumin target 31
  source 1..132: mol_type = other RNA
ctggatataataaagatgtttagctataggctaataagatagttgtgtcaagtgcttcggagacctaacacgtcatccagtcacaacggctatctatatttccactaacgatattatctaagtttgaatata

SEQ ID NO: 93 - RNA, 132 nt, synthetic construct
  misc_feature 1..132: note = gRNA sequence for B-GEn.1 human albumin target 32
  source 1..132: mol_type = other RNA
ctggatataataaagatgtttagctataggctaataagatagttgtgtcaagtgcttcggagacctaacacgtcatccagtcacaacggctatctatatttccactaactctaagtttgaatataaggctat

SEQ ID NO: 94 - RNA, 132 nt, synthetic construct
  misc_feature 1..132: note = gRNA sequence for B-GEn.1 human albumin target 33
  source 1..132: mol_type = other RNA
ctggatataataaagatgtttagctataggctaataagatagttgtgtcaagtgcttcggagacctaacacgtcatccagtcacaacggctatctatatttccactaacatagccttatattcaaacttaga

SEQ ID NO: 95 - RNA, 132 nt, synthetic construct
  misc_feature 1..132: note = gRNA sequence for B-GEn.1 human albumin target 34
  source 1..132: mol_type = other RNA
ctggatataataaagatgtttagctataggctaataagatagttgtgtcaagtgcttcggagacctaacacgtcatccagtcacaacggctatctatatttccactaacaataatttttaaaatagtattct

SEQ ID NO: 96 - RNA, 132 nt, synthetic construct
  misc_feature 1..132: note = gRNA sequence for B-GEn.1 human albumin target 35
  source 1..132: mol_type = other RNA
ctggatataataaagatgtttagctataggctaataagatagttgtgtcaagtgcttcggagacctaacacgtcatccagtcacaacggctatctatatttccactaacaatatttatagccttatattcaa

SEQ ID NO: 97 - RNA, 132 nt, synthetic construct
  misc_feature 1..132: note = gRNA sequence for B-GEn.1 human albumin target 36
  source 1..132: mol_type = other RNA
ctggatataataaagatgtttagctataggctaataagatagttgtgtcaagtgcttcggagacctaacacgtcatccagtcacaacggctatctatatttccactaacttaaatatttatagccttatatt

SEQ ID NO: 98 - RNA, 132 nt, synthetic construct
  misc_feature 1..132: note = gRNA sequence for B-GEn.1 human albumin target 37
  source 1..132: mol_type = other RNA
ctggatataataaagatgtttagctataggctaataagatagttgtgtcaagtgcttcggagacctaacacgtcatccagtcacaacggctatctatatttccactaacttaaaatagtattcttggtaatt

SEQ ID NO: 99 - RNA, 132 nt, synthetic construct
  misc_feature 1..132: note = gRNA sequence for B-GEn.1 human albumin target 38
  source 1..132: mol_type = other RNA
ctggatataataaagatgtttagctataggctaataagatagttgtgtcaagtgcttcggagacctaacacgtcatccagtcacaacggctatctatatttccactaactaaaaattattaaatatttatag

SEQ ID NO: 100 - RNA, 132 nt, synthetic construct
  misc_feature 1..132: note = gRNA sequence for B-GEn.1 human albumin target 39
  source 1..132: mol_type = other RNA
ctggatataataaagatgtttagctataggctaataagatagttgtgtcaagtgcttcggagacctaacacgtcatccagtcacaacggctatctatatttccactaacttggtaattgaattattcttctg

SEQ ID NO: 101 - RNA, 132 nt, synthetic construct
  misc_feature 1..132: note = gRNA sequence for B-GEn.1 human albumin target 40
  source 1..132: mol_type = other RNA
ctggatataataaagatgtttagctataggctaataagatagttgtgtcaagtgcttcggagacctaacacgtcatccagtcacaacggctatctatatttccactaacccaagaatactattttaaaaatt

SEQ ID NO: 102 - RNA, 132 nt, synthetic construct
  misc_feature 1..132: note = gRNA sequence for B-GEn.1 human albumin target 41
  source 1..132: mol_type = other RNA
ctggatataataaagatgtttagctataggctaataagatagttgtgtcaagtgcttcggagacctaacacgtcatccagtcacaacggctatctatatttccactaacaattattcttctgtttaaaggca

SEQ ID NO: 103 - RNA, 132 nt, synthetic construct
  misc_feature 1..132: note = gRNA sequence for B-GEn.1 human albumin target 42
  source 1..132: mol_type = other RNA
ctggatataataaagatgtttagctataggctaataagatagttgtgtcaagtgcttcggagacctaacacgtcatccagtcacaacggctatctatatttccactaacaattaccaagaatactattttaa

SEQ ID NO: 104 - RNA, 132 nt, synthetic construct
  misc_feature 1..132: note = gRNA sequence for B-GEn.1 human albumin target 43
  source 1..132: mol_type = other RNA
ctggatataataaagatgtttagctataggctaataagatagttgtgtcaagtgcttcggagacctaacacgtcatccagtcacaacggctatctatatttccactaacttcttctgtttaaaggcagaaga

SEQ ID NO: 105 - RNA, 132 nt, synthetic construct
  misc_feature 1..132: note = gRNA sequence for B-GEn.1 human albumin target 44
  source 1..132: mol_type = other RNA
ctggatataataaagatgtttagctataggctaataagatagttgtgtcaagtgcttcggagacctaacacgtcatccagtcacaacggctatctatatttccactaacttctgtttaaaggcagaagaaat

SEQ ID NO: 106 - RNA, 132 nt, synthetic construct
  misc_feature 1..132: note = gRNA sequence for B-GEn.1 human albumin target 45
  source 1..132: mol_type = other RNA
ctggatataataaagatgtttagctataggctaataagatagttgtgtcaagtgcttcggagacctaacacgtcatccagtcacaacggctatctatatttccactaaccttctgcctttaaacagaagaat

SEQ ID NO: 107 - RNA, 132 nt, synthetic construct
  misc_feature 1..132: note = gRNA sequence for B-GEn.1 human albumin target 46
  source 1..132: mol_type = other RNA
ctggatataataaagatgtttagctataggctaataagatagttgtgtcaagtgcttcggagacctaacacgtcatccagtcacaacggctatctatatttccactaactttcttctgcctttaaacagaag

SEQ ID NO: 108 - RNA, 132 nt, synthetic construct
  misc_feature 1..132: note = gRNA sequence for B-GEn.1 human albumin target 47
  source 1..132: mol_type = other RNA
ctggatataataaagatgtttagctataggctaataagatagttgtgtcaagtgcttcggagacctaacacgtcatccagtcacaacggctatctatatttccactaacaacatcatcctgagtttttctgt

SEQ ID NO: 109 - RNA, 132 nt, synthetic construct
  misc_feature 1..132: note = gRNA sequence for B-GEn.1 human albumin target 48
  source 1..132: mol_type = other RNA
ctggatataataaagatgtttagctataggctaataagatagttgtgtcaagtgcttcggagacctaacacgtcatccagtcacaacggctatctatatttccactaacctacagaaaaactcaggatgatg

SEQ ID NO: 110 - RNA, 132 nt, synthetic construct
  misc_feature 1..132: note = gRNA sequence for B-GEn.1 human albumin target 49
  source 1..132: mol_type = other RNA
ctggatataataaagatgtttagctataggctaataagatagttgtgtcaagtgcttcggagacctaacacgtcatccagtcacaacggctatctatatttccactaacggctctgattcctacagaaaaac

SEQ ID NO: 111 - RNA, 132 nt, synthetic construct
  misc_feature 1..132: note = gRNA sequence for B-GEn.1 human albumin target 50
  source 1..132: mol_type = other RNA
ctggatataataaagatgtttagctataggctaataagatagttgtgtcaagtgcttcggagacctaacacgtcatccagtcacaacggctatctatatttccactaactgaaacaaatgcataatctaagt

SEQ ID NO: 112 - RNA, 132 nt, synthetic construct
  misc_feature 1..132: note = gRNA sequence for B-GEn.1 human albumin target 51
  source 1..132: mol_type = other RNA
ctggatataataaagatgtttagctataggctaataagatagttgtgtcaagtgcttcggagacctaacacgtcatccagtcacaacggctatctatatttccactaacgtttcaaaatattgggctctgat

SEQ ID NO: 113 - RNA, 132 nt, synthetic construct
  misc_feature 1..132: note = gRNA sequence for B-GEn.1 human albumin target 52
  source 1..132: mol_type = other RNA
ctggatataataaagatgtttagctataggctaataagatagttgtgtcaagtgcttcggagacctaacacgtcatccagtcacaacggctatctatatttccactaactgcatttgtttcaaaatattggg

SEQ ID NO: 114 - RNA, 132 nt, synthetic construct
  misc_feature 1..132: note = gRNA sequence for B-GEn.1 human albumin target 53
  source 1..132: mol_type = other RNA
ctggatataataaagatgtttagctataggctaataagatagttgtgtcaagtgcttcggagacctaacacgtcatccagtcacaacggctatctatatttccactaacctttccatttgacttagattatg

SEQ ID NO: 115 - RNA, 132 nt, synthetic construct
  misc_feature 1..132: note = gRNA sequence for B-GEn.1 human albumin target 54
  source 1..132: mol_type = other RNA
ctggatataataaagatgtttagctataggctaataagatagttgtgtcaagtgcttcggagacctaacacgtcatccagtcacaacggctatctatatttccactaacttacttcttgttttcttcagtat

SEQ ID NO: 116 - RNA, 132 nt, synthetic construct
  misc_feature 1..132: note = gRNA sequence for B-GEn.1 human albumin target 55
  source 1..132: mol_type = other RNA
ctggatataataaagatgtttagctataggctaataagatagttgtgtcaagtgcttcggagacctaacacgtcatccagtcacaacggctatctatatttccactaaccttcttgttttcttcagtattta

SEQ ID NO: 117 - RNA, 132 nt, synthetic construct
  misc_feature 1..132: note = gRNA sequence for B-GEn.1 human albumin target 56
  source 1..132: mol_type = other RNA
ctggatataataaagatgtttagctataggctaataagatagttgtgtcaagtgcttcggagacctaacacgtcatccagtcacaacggctatctatatttccactaacaacaatccttttttttcttccct

SEQ ID NO: 118 - RNA, 132 nt, synthetic construct
  misc_feature 1..132: note = gRNA sequence for B-GEn.1 human albumin target 57
  source 1..132: mol_type = other RNA
ctggatataataaagatgtttagctataggctaataagatagttgtgtcaagtgcttcggagacctaacacgtcatccagtcacaacggctatctatatttccactaacttaaatactgaagaaaacaagaa

SEQ ID NO: 119 - RNA, 132 nt, synthetic construct
  misc_feature 1..132: note = gRNA sequence for B-GEn.1 human albumin target 58
  source 1..132: mol_type = other RNA
ctggatataataaagatgtttagctataggctaataagatagttgtgtcaagtgcttcggagacctaacacgtcatccagtcacaacggctatctatatttccactaacaaacatcctaggtaaaaaaaaaa

SEQ ID NO: 120 - RNA, 132 nt, synthetic construct
  misc_feature 1..132: note = gRNA sequence for B-GEn.1 human albumin target 59
  source 1..132: mol_type = other RNA
ctggatataataaagatgtttagctataggctaataagatagttgtgtcaagtgcttcggagacctaacacgtcatccagtcacaacggctatctatatttccactaactattaataagataaccttgtaag

SEQ ID NO: 121 - RNA, 132 nt, synthetic construct
  misc_feature 1..132: note = gRNA sequence for B-GEn.1 human albumin target 60
  source 1..132: mol_type = other RNA
ctggatataataaagatgtttagctataggctaataagatagttgtgtcaagtgcttcggagacctaacacgtcatccagtcacaacggctatctatatttccactaacaaacttagataatatctaatact

SEQ ID NO: 122 - RNA, 132 nt, synthetic construct
  misc_feature 1..132: note = gRNA sequence for B-GEn.1 human albumin target 61
  source 1..132: mol_type = other RNA
ctggatataataaagatgtttagctataggctaataagatagttgtgtcaagtgcttcggagacctaacacgtcatccagtcacaacggctatctatatttccactaacgacttagattatgcatttgtttc

SEQ ID NO: 123 - DNA, 3364 bp, synthetic construct
  misc_feature 1..3364: note = plasmid including the sequence for B-Gen.1 human albumin target 1
  source 1..3364: mol_type = other DNA
gcacttctattgttcaacttttattctttttttgttttcaacaccggtaccgcgttacaatgataagtcgactgaataagtgaactcgagatcagcctcgactgtgccttctagttgccagccatctgttgtttgcccctcccccgtgccttccttgaccctggaaggtgccactcccactgtcctttcctaataaaatgaggaaattgcatccccacttcagaagttcctatactttctagtgaatgagtgagctaactcacattaattgcgttgcgctcactgcccgctttccagtcgggaaacctgtcgtgccagctgcattaatgaatcggccaacgcgcggggagaggcggtttgcgtattgggcgctcttgcgcttcctcgctcactgactcgctgcgctcggtcgttcggctgcggcgagcggtatcagctcactcaaaggcggtaatacggttatccacagaatcaggggataacgcaggaaagaacatgtgagcaaaaggccagcaaaaggccaggaaccgtaaaaaggccgcgttgctggcgtttttccataggctccgcccccctgacgagcatcacaaaaatcgacgctcaagtcagaggtggcgaaacccgacaggactataaagataccaggcgtttccccctggaagctccctcgtgcgctctcctgttccgaccctgccgcttaccggatacctgtccgcctttctcccttcgggaagcgtggcgctttctcatagctcacgctgtaggtatctcagttcggtgtaggtcgttcgctccaagctgggctgtgtgcacgaaccccccgttcagcccgaccgctgcgccttatccggtaactatcgtcttgagtccaacccggtaagacacgacttatcgccactggcagcagccactggtaacaggattagcagagcgaggtatgtaggcggtgctacagagttcttgaagtggtggcctaactacggctacactagaagaacagtatttggtatctgcgctctgctgaagccagttaccttcggaaaaagagttggtagctcttgatccggcaaacaaaccaccgctggtagcggtggtttttttgtttgcaagcagcagattacgcgcagaaaaaaaggatctcaagaagatcctttgatcttttctacggggtctgacgctcagtggaacgaaaactcacgttaagggattttggtcatgagattatcaaaaaggatcttcacctagatccttttaaattaaaaatgaagttttaaatcaatctaaagtatatatgagtaaacttggtctgacagttaccaatgcttaatcagtgaggcacctatctcagcgatctgtctatttcgttcatccatagttgcctgactccccgtcgtgtagataactacgatacgggagggcttaccatctggccccagtgctgcaatgataccgcgtgacccacgctcaccggctccagatttatcagcaataaaccagccagccggaagggccgagcgcagaagtggtcctgcaactttatccgcctccatccagtctattaattgttgccgggaagctagagtaagtagttcgccagttaatagtttgcgcaacgttgttgccattgctacaggcatcgtggtgtcacgctcgtcgtttggtatggcttcattcagctccggttcccaacgatcaaggcgagttacatgatcccccatgttgtgcaaaaaagcggttagctccttcggtcctccgatcgttgtcagaagtaagttggccgcagtgttatcactcatggttatggcagcactgcataattctcttactgtcatgccatccgtaagatgcttttctgtgactggtgagtactcaaccaagtcattctgagaatagtgtatgcggcgaccgagttgctcttgcccggcgtcaatacgggataataccgcgccacatagcagaactttaaaagtgctcatcattggaaaacgttcttcggggcgaaaactctcaaggatcttaccgctgttgagatccagttcgatgtaacccactcgtgcacccaactgatcttcagcatcttttactttcaccagcgtttctgggtgagcaaaaacaggaaggcaaaatgccgcaaaaaagggaataagggcgacacggaaatgttgaatactcatactcttcctttttcaatattattgaagcatttatcagggttattgtctcatgagcggatacatatttgaatgtatttagaaaaataaacaaataggggttccgcgcatatttccccgaaaagtgccacctgacgtcgacggatcgggagatctcccgatcccctatggtgcactctcagtacaatctgctctgatgccgcatagttaagccagtatctgctccctgcttgtgtgttggaggtcgctgagtagtgcgcgagcaaaatttaagctacaacaaggcaaggcttgaccgagcaaacaaactctttctgtgttgtaaaacgacggccagtcttaagctcgggccccctgggcggttctgataacgagtaatcgttaatccgcaaataacgtaaaaacccgcttcggcgggtttttttatggggggagtttagggaaagagcatttgtcagaatatttaagggcgcctgtcactttgcttgatatatgagaattatttaaccttataaatgagaaaaaagcaacgcactttaaataagatacgttgctttttcgattgatgaacacctataattaaactattcatctattatttatgattttttgtatatacaatatttctagtttgttaaagagaattaagaaaataaatctcgaaaataataaagggaaaatcagtttttgatatcaaaattatacatgtcaacgataatacaaaatataatacaaactataagatgttatcagtatttattatgcatttagaataaattttgtgtcgcccttattcgactcactatagaagttcctattctctagaaagtagaggaacttcacttcattttgctagcgtgtgagggcctatttcccatgattccttcatatttgcatatacgatacaaggctgttagagagataattggaattaatttgactgtaaacacaaagatattagtacaaaatacgtgacgtagaaagtaataatttcttgggtagtttgcagttttaaaattatgttttaaaatggactatcatatgcttaccgtaacttgaaagtatttcgatttcttggctttatatatcttgtggaaaggacgaaacaccgttagctataggctaataagatagttgtgtcaagtgcttcggagacctaacacgtctccagtcacaacggctaaaaatagcca

SEQ ID NO: 124 - DNA, 3364 bp, synthetic construct
  misc_feature 1..3364: note = plasmid including the sequence for B-Gen.1 human albumin target 2
  source 1..3364: mol_type = other DNA
gcacttcaacttttattctattttcccttttttgttttcaacaccggtaccgcgttacaatgataagtcgactgaataagtgaactcgagatcagcctcgactgtgccttctagttgccagccatctgttgtttgcccctcccccgtgccttccttgaccctggaaggtgccactcccactgtcctttcctaataaaatgaggaaattgcatccccacttcagaagttcctatactttctagtgaatgagtgagctaactcacattaattgcgttgcgctcactgcccgctttccagtcgggaaacctgtcgtgccagctgcattaatgaatcggccaacgcgcggggagaggcggtttgcgtattgggcgctcttgcgcttcctcgctcactgactcgctgcgctcggtcgttcggctgcggcgagcggtatcagctcactcaaaggcggtaatacggttatccacagaatcaggggataacgcaggaaagaacatgtgagcaaaaggccagcaaaaggccaggaaccgtaaaaaggccgcgttgctggcgtttttccataggctccgcccccctgacgagcatcacaaaaatcgacgctcaagtcagaggtggcgaaacccgacaggactataaagataccaggcgtttccccctggaagctccctcgtgcgctctcctgttccgaccctgccgcttaccggatacctgtccgcctttctcccttcgggaagcgtggcgctttctcatagctcacgctgtaggtatctcagttcggtgtaggtcgttcgctccaagctgggctgtgtgcacgaaccccccgttcagcccgaccgctgcgccttatccggtaactatcgtcttgagtccaacccggtaagacacgacttatcgccactggcagcagccactggtaacaggattagcagagcgaggtatgtaggcggtgctacagagttcttgaagtggtggcctaactacggctacactagaagaacagtatttggtatctgcgctctgctgaagccagttaccttcggaaaaagagttggtagctcttgatccggcaaacaaaccaccgctggtagcggtggtttttttgtttgcaagcagcagattacgcgcagaaaaaaaggatctcaagaagatcctttgatcttttctacggggtctgacgctcagtggaacgaaaactcacgttaagggattttggtcatgagattatcaaaaaggatcttcacctagatccttttaaattaaaaatgaagttttaaatcaatctaaagtatatatgagtaaacttggtctgacagttaccaatgcttaatcagtgaggcacctatctcagcgatctgtctatttcgttcatccatagttgcctgactccccgtcgtgtagataactacgatacgggagggcttaccatctggccccagtgctgcaatgataccgcgtgacccacgctcaccggctccagatttatcagcaataaaccagccagccggaagggccgagcgcagaagtggtcctgcaactttatccgcctccatccagtctattaattgttgccgggaagctagagtaagtagttcgccagttaatagtttgcgcaacgttgttgccattgctacaggcatcgtggtgtcacgctcgtcgtttggtatggcttcattcagctccggttcccaacgatcaaggcgagttacatgatcccccatgttgtgcaaaaaagcggttagctccttcggtcctccgatcgttgtcagaagtaagttggccgcagtgttatcactcatggttatggcagcactgcataattctcttactgtcatgccatccgtaagatgcttttctgtgactggtgagtactcaaccaagtcattctgagaatagtgtatgcggcgaccgagttgctcttgcccggcgtcaatacgggataataccgcgccacatagcagaactttaaaagtgctcatcattggaaaacgttcttcggggcgaaaactctcaaggatcttaccgctgttgagatccagttcgatgtaacccactcgtgcacccaactgatcttcagcatcttttactttcaccagcgtttctgggtgagcaaaaacaggaaggcaaaatgccgcaaaaaagggaataagggcgacacggaaatgttgaatactcatactcttcctttttcaatattattgaagcatttatcagggttattgtctcatgagcggatacatatttgaatgtatttagaaaaataaacaaataggggttccgcgcatatttccccgaaaagtgccacctgacgtcgacggatcgggagatctcccgatcccctatggtgcactctcagtacaatctgctctgatgccgcatagttaagccagtatctgctccctgcttgtgtgttggaggtcgctgagtagtgcgcgagcaaaatttaagctacaacaaggcaaggcttgaccgagcaaacaaactctttctgtgttgtaaaacgacggccagtcttaagctcgggccccctgggcggttctgataacgagtaatcgttaatccgcaaataacgtaaaaacccgcttcggcgggtttttttatggggggagtttagggaaagagcatttgtcagaatatttaagggcgcctgtcactttgcttgatatatgagaattatttaaccttataaatgagaaaaaagcaacgcactttaaataagatacgttgctttttcgattgatgaacacctataattaaactattcatctattatttatgattttttgtatatacaatatttctagtttgttaaagagaattaagaaaataaatctcgaaaataataaagggaaaatcagtttttgatatcaaaattatacatgtcaacgataatacaaaatataatacaaactataagatgttatcagtatttattatgcatttagaataaattttgtgtcgcccttattcgactcactatagaagttcctattctctagaaagtagaggaacttcacttcattttgctagcgtgtgagggcctatttcccatgattccttcatatttgcatatacgatacaaggctgttagagagataattggaattaatttgactgtaaacacaaagatattagtacaaaatacgtgacgtagaaagtaataatttcttgggtagtttgcagttttaaaattatgttttaaaatggactatcatatgcttaccgtaacttgaaagtatttcgatttcttggctttatatatcttgtggaaaggacgaaacaccgttagctataggctaataagatagttgtgtcaagtgcttcggagacctaacacgtctccagtcacaacggctaaaaatagcca

SEQ ID NO: 125 - DNA, 3364 bp, synthetic construct
  misc_feature 1..3364: note = plasmid including the sequence for B-Gen.1 human albumin target 3
  source 1..3364: mol_type = other DNA
gcactattttcccagtaaaataaagttttttttgttttcaacaccggtaccgcgttacaatgataagtcgactgaataagtgaactcgagatcagcctcgactgtgccttctagttgccagccatctgttgtttgcccctcccccgtgccttccttgaccctggaaggtgccactcccactgtcctttcctaataaaatgaggaaattgcatccccacttcagaagttcctatactttctagtgaatgagtgagctaactcacattaattgcgttgcgctcactgcccgctttccagtcgggaaacctgtcgtgccagctgcattaatgaatcggccaacgcgcggggagaggcggtttgcgtattgggcgctcttgcgcttcctcgctcactgactcgctgcgctcggtcgttcggctgcggcgagcggtatcagctcactcaaaggcggtaatacggttatccacagaatcaggggataacgcaggaaagaacatgtgagcaaaaggccagcaaaaggccaggaaccgtaaaaaggccgcgttgctggcgtttttccataggctccgcccccctgacgagcatcacaaaaatcgacgctcaagtcagaggtggcgaaacccgacaggactataaagataccaggcgtttccccctggaagctccctcgtgcgctctcctgttccgaccctgccgcttaccggatacctgtccgcctttctcccttcgggaagcgtggcgctttctcatagctcacgctgtaggtatctcagttcggtgtaggtcgttcgctccaagctgggctgtgtgcacgaaccccccgttcagcccgaccgctgcgccttatccggtaactatcgtcttgagtccaacccggtaagacacgacttatcgccactggcagcagccactggtaacaggattagcagagcgaggtatgtaggcggtgctacagagttcttgaagtggtggcctaactacggctacactagaagaacagtatttggtatctgcgctctgctgaagccagttaccttcggaaaaagagttggtagctcttgatccggcaaacaaaccaccgctggtagcggtggtttttttgtttgcaagcagcagattacgcgcagaaaaaaaggatctcaagaagatcctttgatcttttctacggggtctgacgctcagtggaacgaaaactcacgttaagggattttggtcatgagattatcaaaaaggatcttcacctagatccttttaaattaaaaatgaagttttaaatcaatctaaagtatatatgagtaaacttggtctgacagttaccaatgcttaatcagtgaggcacctatctcagcgatctgtctatttcgttcatccatagttgcctgactccccgtcgtgtagataactacgatacgggagggcttaccatctggccccagtgctgcaatgataccgcgtgacccacgctcaccggctccagatttatcagcaataaaccagccagccggaagggccgagcgcagaagtggtcctgcaactttatccgcctccatccagtctattaattgttgccgggaagctagagtaagtagttcgccagttaatagtttgcgcaacgttgttgccattgctacaggcatcgtggtgtcacgctcgtcgtttggtatggcttcattcagctccggttcccaacgatcaaggcgagttacatgatcccccatgttgtgcaaaaaagcggttagctccttcggtcctccgatcgttgtcagaagtaagttggccgcagtgttatcactcatggttatggcagcactgcataattctcttactgtcatgccatccgtaagatgcttttctgtgactggtgagtactcaaccaagtcattctgagaatagtgtatgcggcgaccgagttgctcttgcccggcgtcaatacgggataataccgcgccacatagcagaactttaaaagtgctcatcattggaaaacgttcttcggggcgaaaactctcaaggatcttaccgctgttgagatccagttcgatgtaacccactcgtgcacccaactgatcttcagcatcttttactttcaccagcgtttctgggtgagcaaaaacaggaaggcaaaatgccgcaaaaaagggaataagggcgacacggaaatgttgaatactcatactcttcctttttcaatattattgaagcatttatcagggttattgtctcatgagcggatacatatttgaatgtatttagaaaaataaacaaataggggttccgcgcatatttccccgaaaagtgccacctgacgtcgacggatcgggagatctcccgatcccctatggtgcactctcagtacaatctgctctgatgccgcatagttaagccagtatctgctccctgcttgtgtgttggaggtcgctgagtagtgcgcgagcaaaatttaagctacaacaaggcaaggcttgaccgagcaaacaaactctttctgtgttgtaaaacgacggccagtcttaagctcgggccccctgggcggttctgataacgagtaatcgttaatccgcaaataacgtaaaaacccgcttcggcgggtttttttatggggggagtttagggaaagagcatttgtcagaatatttaagggcgcctgtcactttgcttgatatatgagaattatttaaccttataaatgagaaaaaagcaacgcactttaaataagatacgttgctttttcgattgatgaacacctataattaaactattcatctattatttatgattttttgtatatacaatatttctagtttgttaaagagaattaagaaaataaatctcgaaaataataaagggaaaatcagtttttgatatcaaaattatacatgtcaacgataatacaaaatataatacaaactataagatgttatcagtatttattatgcatttagaataaattttgtgtcgcccttattcgactcactatagaagttcctattctctagaaagtagaggaacttcacttcattttgctagcgtgtgagggcctatttcccatgattccttcatatttgcatatacgatacaaggctgttagagagataattggaattaatttgactgtaaacacaaagatattagtacaaaatacgtgacgtagaaagtaataatttcttgggtagtttgcagttttaaaattatgttttaaaatggactatcatatgcttaccgtaacttgaaagtatttcgatttcttggctttatatatcttgtggaaaggacgaaacaccgttagctataggctaataagatagttgtgtcaagtgcttcggagacctaacacgtctccagtcacaacggctaaaaatagcca

SEQ ID NO: 126 - DNA, 3364 bp, synthetic construct
  misc_feature 1..3364: note = plasmid including the sequence for B-Gen.1 human albumin target 4
  source 1..3364: mol_type = other DNA
gcactcccagtaaaataaagttttagtttttttgttttcaacaccggtaccgcgttacaatgataagtcgactgaataagtgaactcgagatcagcctcgactgtgccttctagttgccagccatctgttgtttgcccctcccccgtgccttccttgaccctggaaggtgccactcccactgtcctttcctaataaaatgaggaaattgcatccccacttcagaagttcctatactttctagtgaatgagtgagctaactcacattaattgcgttgcgctcactgcccgctttccagtcgggaaacctgtcgtgccagctgcattaatgaatcggccaacgcgcggggagaggcggtttgcgtattgggcgctcttgcgcttcctcgctcactgactcgctgcgctcggtcgttcggctgcggcgagcggtatcagctcactcaaaggcggtaatacggttatccacagaatcaggggataacgcaggaaagaacatgtgagcaaaaggccagcaaaaggccaggaaccgtaaaaaggccgcgttgctggcgtttttccataggctccgcccccctgacgagcatcacaaaaatcgacgctcaagtcagaggtggcgaaacccgacaggactataaagataccaggcgtttccccctggaagctccctcgtgcgctctcctgttccgaccctgccgcttaccggatacctgtccgcctttctcccttcgggaagcgtggcgctttctcatagctcacgctgtaggtatctcagttcggtgtaggtcgttcgctccaagctgggctgtgtgcacgaaccccccgttcagcccgaccgctgcgccttatccggtaactatcgtcttgagtccaacccggtaagacacgacttatcgccactggcagcagccactggtaacaggattagcagagcgaggtatgtaggcggtgctacagagttcttgaagtggtggcctaactacggctacactagaagaacagtatttggtatctgcgctctgctgaagccagttaccttcggaaaaagagttggtagctcttgatccggcaaacaaaccaccgctggtagcggtggtttttttgtttgcaagcagcagattacgcgcagaaaaaaaggatctcaagaagatcctttgatcttttctacggggtctgacgctcagtggaacgaaaactcacgttaagggattttggtcatgagattatcaaaaaggatcttcacctagatccttttaaattaaaaatgaagttttaaatcaatctaaagtatatatgagtaaacttggtctgacagttaccaatgcttaatcagtgaggcacctatctcagcgatctgtctatttcgttcatccatagttgcctgactccccgtcgtgtagataactacgatacgggagggcttaccatctggccccagtgctgcaatgataccgcgtgacccacgctcaccggctccagatttatcagcaataaaccagccagccggaagggccgagcgcagaagtggtcctgcaactttatccgcctccatccagtctattaattgttgccgggaagctagagtaagtagttcgccagttaatagtttgcgcaacgttgttgccattgctacaggcatcgtggtgtcacgctcgtcgtttggtatggcttcattcagctccggttcccaacgatcaaggcgagttacatgatcccccatgttgtgcaaaaaagcggttagctccttcggtcctccgatcgttgtcagaagtaagttggccgcagtgttatcactcatggttatggcagcactgcataattctcttactgtcatgccatccgtaagatgcttttctgtgactggtgagtactcaaccaagtcattctgagaatagtgtatgcggcgaccgagttgctcttgcccggcgtcaatacgggataataccgcgccacatagcagaactttaaaagtgctcatcattggaaaacgttcttcggggcgaaaactctcaaggatcttaccgctgttgagatccagttcgatgtaacccactcgtgcacccaactgatcttcagcatcttttactttcaccagcgtttctgggtgagcaaaaacaggaaggcaaaatgccgcaaaaaagggaataagggcgacacggaaatgttgaatactcatactcttcctttttcaatattattgaagcatttatcagggttattgtctcatgagcggatacatatttgaatgtatttagaaaaataaacaaataggggttccgcgcatatttccccgaaaagtgccacctgacgtcgacggatcgggagatctcccgatcccctatggtgcactctcagtacaatctgctctgatgccgcatagttaagccagtatctgctccctgcttgtgtgttggaggtcgctgagtagtgcgcgagcaaaatttaagctacaacaaggcaaggcttgaccgagcaaacaaactctttctgtgttgtaaaacgacggccagtcttaagctcgggccccctgggcggttctgataacgagtaatcgttaatccgcaaataacgtaaaaacccgcttcggcgggtttttttatggggggagtttagggaaagagcatttgtcagaatatttaagggcgcctgtcactttgcttgatatatgagaattatttaaccttataaatgagaaaaaagcaacgcactttaaataagatacgttgctttttcgattgatgaacacctataattaaactattcatctattatttatgattttttgtatatacaatatttctagtttgttaaagagaattaagaaaataaatctcgaaaataataaagggaaaatcagtttttgatatcaaaattatacatgtcaacgataatacaaaatataatacaaactataagatgttatcagtatttattatgcatttagaataaattttgtgtcgcccttattcgactcactatagaagttcctattctctagaaagtagaggaacttcacttcattttgctagcgtgtgagggcctatttcccatgattccttcatatttgcatatacgatacaaggctgttagagagataattggaattaatttgactgtaaacacaaagatattagtacaaaatacgtgacgtagaaagtaataatttcttgggtagtttgcagttttaaaattatgttttaaaatggactatcatatgcttaccgtaacttgaaagtatttcgatttcttggctttatatatcttgtggaaaggacgaaacaccgttagctataggctaataagatagttgtgtcaagtgcttcggagacctaacacgtctccagtcacaacggctaaaaatagcca

SEQ ID NO: 127 - DNA, 3364 bp, synthetic construct
  misc_feature 1..3364: note = plasmid including the sequence for B-Gen.1 human albumin target 5
  source 1..3364: mol_type = other DNA
gcactactgggaaaatagaataaaagtttttttgttttcaacaccggtaccgcgttacaatgataagtcgactgaataagtgaactcgagatcagcctcgactgtgccttctagttgccagccatctgttgtttgcccctcccccgtgccttccttgaccctggaaggtgccactcccactgtcctttcctaataaaatgaggaaattgcatccccacttcagaagttcctatactttctagtgaatgagtgagctaactcacattaattgcgttgcgctcactgcccgctttccagtcgggaaacctgtcgtgccagctgcattaatgaatcggccaacgcgcggggagaggcggtttgcgtattgggcgctcttgcgcttcctcgctcactgactcgctgcgctcggtcgttcggctgcggcgagcggtatcagctcactcaaaggcggtaatacggttatccacagaatcaggggataacgcaggaaagaacatgtgagcaaaaggccagcaaaaggccaggaaccgtaaaaaggccgcgttgctggcgtttttccataggctccgcccccctgacgagcatcacaaaaatcgacgctcaagtcagaggtggcgaaacccgacaggactataaagataccaggcgtttccccctggaagctccctcgtgcgctctcctgttccgaccctgccgcttaccggatacctgtccgcctttctcccttcgggaagcgtggcgctttctcatagctcacgctgtaggtatctcagttcggtgtaggtcgttcgctccaagctgggctgtgtgcacgaaccccccgttcagcccgaccgctgcgccttatccggtaactatcgtcttgagtccaacccggtaagacacgacttatcgccactggcagcagccactggtaacaggattagcagagcgaggtatgtaggcggtgctacagagttcttgaagtggtggcctaactacggctacactagaagaacagtatttggtatctgcgctctgctgaagccagttaccttcggaaaaagagttggtagctcttgatccggcaaacaaaccaccgctggtagcggtggtttttttgtttgcaagcagcagattacgcgcagaaaaaaaggatctcaagaagatcctttgatcttttctacggggtctgacgctcagtggaacgaaaactcacgttaagggattttggtcatgagattatcaaaaaggatcttcacctagatccttttaaattaaaaatgaagttttaaatcaatctaaagtatatatgagtaaacttggtctgacagttaccaatgcttaatcagtgaggcacctatctcagcgatctgtctatttcgttcatccatagttgcctgactccccgtcgtgtagataactacgatacgggagggcttaccatctggccccagtgctgcaatgataccgcgtgacccacgctcaccggctccagatttatcagcaataaaccagccagccggaagggccgagcgcagaagtggtcctgcaactttatccgcctccatccagtctattaattgttgccgggaagctagagtaagtagttcgccagttaatagtttgcgcaacgttgttgccattgctacaggcatcgtggtgtcacgctcgtcgtttggtatggcttcattcagctccggttcccaacgatcaaggcgagttacatgatcccccatgttgtgcaaaaaagcggttagctccttcggtcctccgatcgttgtcagaagtaagttggccgcagtgttatcactcatggttatggcagcactgcataattctcttactgtcatgccatccgtaagatgcttttctgtgactggtgagtactcaaccaagtcattctgagaatagtgtatgcggcgaccgagttgctcttgcccggcgtcaatacgggataataccgcgccacatagcagaactttaaaagtgctcatcattggaaaacgttcttcggggcgaaaactctcaaggatcttaccgctgttgagatccagttcgatgtaacccactcgtgcacccaactgatcttcagcatcttttactttcaccagcgtttctgggtgagcaaaaacaggaaggcaaaatgccgcaaaaaagggaataagggcgacacggaaatgttgaatactcatactcttcctttttcaatattattgaagcatttatcagggttattgtctcatgagcggatacatatttgaatgtatttagaaaaataaacaaataggggttccgcgcatatttccccgaaaagtgccacctgacgtcgacggatcgggagatctcccgatcccctatggtgcactctcagtacaatctgctctgatgccgcatagttaagccagtatctgctccctgcttgtgtgttggaggtcgctgagtagtgcgcgagcaaaatttaagctacaacaaggcaaggcttgaccgagcaaacaaactctttctgtgttgtaaaacgacggccagtcttaagctcgggccccctgggcggttctgataacgagtaatcgttaatccgcaaataacgtaaaaacccgcttcggcgggtttttttatggggggagtttagggaaagagcatttgtcagaatatttaagggcgcctgtcactttgcttgatatatgagaattatttaaccttataaatgagaaaaaagcaacgcactttaaataagatacgttgctttttcgattgatgaacacctataattaaactattcatctattatttatgattttttgtatatacaatatttctagtttgttaaagagaattaagaaaataaatctcgaaaataataaagggaaaatcagtttttgatatcaaaattatacatgtcaacgataatacaaaatataatacaaactataagatgttatcagtatttattatgcatttagaataaattttgtgtcgcccttattcgactcactatagaagttcctattctctagaaagtagaggaacttcacttcattttgctagcgtgtgagggcctatttcccatgattccttcatatttgcatatacgatacaaggctgttagagagataattggaattaatttgactgtaaacacaaagatattagtacaaaatacgtgacgtagaaagtaataatttcttgggtagtttgcagttttaaaattatgttttaaaatggactatcatatgcttaccgtaacttgaaagtatttcgatttcttggctttatatatcttgtggaaaggacgaaacaccgttagctataggctaataagatagttgtgtcaagtgcttcggagacctaacacgtctccagtcacaacggctaaaaatagcca

SEQ ID NO: 128 - DNA, 3364 bp, synthetic construct
  misc_feature 1..3364: note = plasmid including the sequence for B-Gen.1 human albumin target 6
  source 1..3364: mol_type = other DNA
gcactttaaagatgcagagtttactaattttttgttttcaacaccggtaccgcgttacaatgataagtcgactgaataagtgaactcgagatcagcctcgactgtgccttctagttgccagccatctgttgtttgcccctcccccgtgccttccttgaccctggaaggtgccactcccactgtcctttcctaataaaatgaggaaattgcatccccacttcagaagttcctatactttctagtgaatgagtgagctaactcacattaattgcgttgcgctcactgcccgctttccagtcgggaaacctgtcgtgccagctgcattaatgaatcggccaacgcgcggggagaggcggtttgcgtattgggcgctcttgcgcttcctcgctcactgactcgctgcgctcggtcgttcggctgcggcgagcggtatcagctcactcaaaggcggtaatacggttatccacagaatcaggggataacgcaggaaagaacatgtgagcaaaaggccagcaaaaggccaggaaccgtaaaaaggccgcgttgctggcgtttttccataggctccgcccccctgacgagcatcacaaaaatcgacgctcaagtcagaggtggcgaaacccgacaggactataaagataccaggcgtttccccctggaagctccctcgtgcgctctcctgttccgaccctgccgcttaccggatacctgtccgcctttctcccttcgggaagcgtggcgctttctcatagctcacgctgtaggtatctcagttcggtgtaggtcgttcgctccaagctgggctgtgtgcacgaaccccccgttcagcccgaccgctgcgccttatccggtaactatcgtcttgagtccaacccggtaagacacgacttatcgccactggcagcagccactggtaacaggattagcagagcgaggtatgtaggcggtgctacagagttcttgaagtggtggcctaactacggctacactagaagaacagtatttggtatctgcgctctgctgaagccagttaccttcggaaaaagagttggtagctcttgatccggcaaacaaaccaccgctggtagcggtggtttttttgtttgcaagcagcagattacgcgcagaaaaaaaggatctcaagaagatcctttgatcttttctacggggtctgacgctcagtggaacgaaaactcacgttaagggattttggtcatgagattatcaaaaaggatcttcacctagatccttttaaattaaaaatgaagttttaaatcaatctaaagtatatatgagtaaacttggtctgacagttaccaatgcttaatcagtgaggcacctatctcagcgatctgtctatttcgttcatccatagttgcctgactccccgtcgtgtagataactacgatacgggagggcttaccatctggccccagtgctgcaatgataccgcgtgacccacgctcaccggctccagatttatcagcaataaaccagccagccggaagggccgagcgcagaagtggtcctgcaactttatccgcctccatccagtctattaattgttgccgggaagctagagtaagtagttcgccagttaatagtttgcgcaacgttgttgccattgctacaggcatcgtggtgtcacgctcgtcgtttggtatggcttcattcagctccggttcccaacgatcaaggcgagttacatgatcccccatgttgtgcaaaaaagcggttagctccttcggtcctccgatcgttgtcagaagtaagttggccgcagtgttatcactcatggttatggcagcactgcataattctcttactgtcatgccatccgtaagatgcttttctgtgactggtgagtactcaaccaagtcattctgagaatagtgtatgcggcgaccgagttgctcttgcccggcgtcaatacgggataataccgcgccacatagcagaactttaaaagtgctcatcattggaaaacgttcttcggggcgaaaactctcaaggatcttaccgctgttgagatccagttcgatgtaacccactcgtgcacccaactgatcttcagcatcttttactttcaccagcgtttctgggtgagcaaaaacaggaaggcaaaatgccgcaaaaaagggaataagggcgacacggaaatgttgaatactcatactcttcctttttcaatattattgaagcatttatcagggttattgtctcatgagcggatacatatttgaatgtatttagaaaaataaacaaataggggttccgcgcatatttccccgaaaagtgccacctgacgtcgacggatcgggagatctcccgatcccctatggtgcactctcagtacaatctgctctgatgccgcatagttaagccagtatctgctccctgcttgtgtgttggaggtcgctgagtagtgcgcgagcaaaatttaagctacaacaaggcaaggcttgaccgagcaaacaaactctttctgtgttgtaaaacgacggccagtcttaagctcgggccccctgggcggttctgataacgagtaatcgttaatccgcaaataacgtaaaaacccgcttcggcgggtttttttatggggggagtttagggaaagagcatttgtcagaatatttaagggcgcctgtcactttgcttgatatatgagaattatttaaccttataaatgagaaaaaagcaacgcactttaaataagatacgttgctttttcgattgatgaacacctataattaaactattcatctattatttatgattttttgtatatacaatatttctagtttgttaaagagaattaagaaaataaatctcgaaaataataaagggaaaatcagtttttgatatcaaaattatacatgtcaacgataatacaaaatataatacaaactataagatgttatcagtatttattatgcatttagaataaattttgtgtcgcccttattcgactcactatagaagttcctattctctagaaagtagaggaacttcacttcattttgctagcgtgtgagggcctatttcccatgattccttcatatttgcatatacgatacaaggctgttagagagataattggaattaatttgactgtaaacacaaagatattagtacaaaatacgtgacgtagaaagtaataatttcttgggtagtttgcagttttaaaattatgttttaaaatggactatcatatgcttaccgtaacttgaaagtatttcgatttcttggctttatatatcttgtggaaaggacgaaacaccgttagctataggctaataagatagttgtgtcaagtgcttcggagacctaacacgtctccagtcacaacggctaaaaatagcca

SEQ ID NO: 129 - DNA, 3364 bp, synthetic construct
  misc_feature 1..3364: note = plasmid including the sequence for B-Gen.1 human albumin target 7
  source 1..3364: mol_type = other DNA
gcacttttggcatttatttctaaaatgttttttgttttcaacaccggtaccgcgttacaatgataagtcgactgaataagtgaactcgagatcagcctcgactgtgccttctagttgccagccatctgttgtttgcccctcccccgtgccttccttgaccctggaaggtgccactcccactgtcctttcctaataaaatgaggaaattgcatccccacttcagaagttcctatactttctagtgaatgagtgagctaactcacattaattgcgttgcgctcactgcccgctttccagtcgggaaacctgtcgtgccagctgcattaatgaatcggccaacgcgcggggagaggcggtttgcgtattgggcgctcttgcgcttcctcgctcactgactcgctgcgctcggtcgttcggctgcggcgagcggtatcagctcactcaaaggcggtaatacggttatccacagaatcaggggataacgcaggaaagaacatgtgagcaaaaggccagcaaaaggccaggaaccgtaaaaaggccgcgttgctggcgtttttccataggctccgcccccctgacgagcatcacaaaaatcgacgctcaagtcagaggtggcgaaacccgacaggactataaagataccaggcgtttccccctggaagctccctcgtgcgctctcctgttccgaccctgccgcttaccggatacctgtccgcctttctcccttcgggaagcgtggcgctttctcatagctcacgctgtaggtatctcagttcggtgtaggtcgttcgctccaagctgggctgtgtgcacgaaccccccgttcagcccgaccgctgcgccttatccggtaactatcgtcttgagtccaacccggtaagacacgacttatcgccactggcagcagccactggtaacaggattagcagagcgaggtatgtaggcggtgctacagagttcttgaagtggtggcctaactacggctacactagaagaacagtatttggtatctgcgctctgctgaagccagttaccttcggaaaaagagttggtagctcttgatccggcaaacaaaccaccgctggtagcggtggtttttttgtttgcaagcagcagattacgcgcagaaaaaaaggatctcaagaagatcctttgatcttttctacggggtctgacgctcagtggaacgaaaactcacgttaagggattttggtcatgagattatcaaaaaggatcttcacctagatccttttaaattaaaaatgaagttttaaatcaatctaaagtatatatgagtaaacttggtctgacagttaccaatgcttaatcagtgaggcacctatctcagcgatctgtctatttcgttcatccatagttgcctgactccccgtcgtgtagataactacgatacgggagggcttaccatctggccccagtgctgcaatgataccgcgtgacccacgctcaccggctccagatttatcagcaataaaccagccagccggaagggccgagcgcagaagtggtcctgcaactttatccgcctccatccagtctattaattgttgccgggaagctagagtaagtagttcgccagttaatagtttgcgcaacgttgttgccattgctacaggcatcgtggtgtcacgctcgtcgtttggtatggcttcattcagctccggttcccaacgatcaaggcgagttacatgatcccccatgttgtgcaaaaaagcggttagctccttcggtcctccgatcgttgtcagaagtaagttggccgcagtgttatcactcatggttatggcagcactgcataattctcttactgtcatgccatccgtaagatgcttttctgtgactggtgagtactcaaccaagtcattctgagaatagtgtatgcggcgaccgagttgctcttgcccggcgtcaatacgggataataccgcgccacatagcagaactttaaaagtgctcatcattggaaaacgttcttcggggcgaaaactctcaaggatcttaccgctgttgagatccagttcgatgtaacccactcgtgcacccaactgatcttcagcatcttttactttcaccagcgtttctgggtgagcaaaaacaggaaggcaaaatgccgcaaaaaagggaataagggcgacacggaaatgttgaatactcatactcttcctttttcaatattattgaagcatttatcagggttattgtctcatgagcggatacatatttgaatgtatttagaaaaataaacaaataggggttccgcgcatatttccccgaaaagtgccacctgacgtcgacggatcgggagatctcccgatcccctatggtgcactctcagtacaatctgctctgatgccgcatagttaagccagtatctgctccctgcttgtgtgttggaggtcgctgagtagtgcgcgagcaaaatttaagctacaacaaggcaaggcttgaccgagcaaacaaactctttctgtgttgtaaaacgacggccagtcttaagctcgggccccctgggcggttctgataacgagtaatcgttaatccgcaaataacgtaaaaacccgcttcggcgggtttttttatggggggagtttagggaaagagcatttgtcagaatatttaagggcgcctgtcactttgcttgatatatgagaattatttaaccttataaatgagaaaaaagcaacgcactttaaataagatacgttgctttttcgattgatgaacacctataattaaactattcatctattatttatgattttttgtatatacaatatttctagtttgttaaagagaattaagaaaataaatctcgaaaataataaagggaaaatcagtttttgatatcaaaattatacatgtcaacgataatacaaaatataatacaaactataagatgttatcagtatttattatgcatttagaataaattttgtgtcgcccttattcgactcactatagaagttcctattctctagaaagtagaggaacttcacttcattttgctagcgtgtgagggcctatttcccatgattccttcatatttgcatatacgatacaaggctgttagagagataattggaattaatttgactgtaaacacaaagatattagtacaaaatacgtgacgtagaaagtaataatttcttgggtagtttgcagttttaaaattatgttttaaaatggactatcatatgcttaccgtaacttgaaagtatttcgatttcttggctttatatatcttgtggaaaggacgaaacaccgttagctataggctaataagatagttgtgtcaagtgcttcggagacctaacacgtctccagtcacaacggctaaaaatagcca

SEQ ID NO: 130 - DNA, 3364 bp, synthetic construct
  misc_feature 1..3364: note = plasmid including the sequence for B-Gen.1 human albumin target 8
  source 1..3364: mol_type = other DNA
gcactggcatttatttctaaaatggcattttttgttttcaacaccggtaccgcgttacaatgataagtcgactgaataagtgaactcgagatcagcctcgactgtgccttctagttgccagccatctgttgtttgcccctcccccgtgccttccttgaccctggaaggtgccactcccactgtcctttcctaataaaatgaggaaattgcatccccacttcagaagttcctatactttctagtgaatgagtgagctaactcacattaattgcgttgcgctcactgcccgctttccagtcgggaaacctgtcgtgccagctgcattaatgaatcggccaacgcgcggggagaggcggtttgcgtattgggcgctcttgcgcttcctcgctcactgactcgctgcgctcggtcgttcggctgcggcgagcggtatcagctcactcaaaggcggtaatacggttatccacagaatcaggggataacgcaggaaagaacatgtgagcaaaaggccagcaaaaggccaggaaccgtaaaaaggccgcgttgctggcgtttttccataggctccgcccccctgacgagcatcacaaaaatcgacgctcaagtcagaggtggcgaaacccgacaggactataaagataccaggcgtttccccctggaagctccctcgtgcgctctcctgttccgaccctgccgcttaccggatacctgtccgcctttctcccttcgggaagcgtggcgctttctcatagctcacgctgtaggtatctcagttcggtgtaggtcgttcgctccaagctgggctgtgtgcacgaaccccccgttcagcccgaccgctgcgccttatccggtaactatcgtcttgagtccaacccggtaagacacgacttatcgccactggcagcagccactggtaacaggattagcagagcgaggtatgtaggcggtgctacagagttcttgaagtggtggcctaactacggctacactagaagaacagtatttggtatctgcgctctgctgaagccagttaccttcggaaaaagagttggtagctcttgatccggcaaacaaaccaccgctggtagcggtggtttttttgtttgcaagcagcagattacgcgcagaaaaaaaggatctcaagaagatcctttgatcttttctacggggtctgacgctcagtggaacgaaaactcacgttaagggattttggtcatgagattatcaaaaaggatcttcacctagatccttttaaattaaaaatgaagttttaaatcaatctaaagtatatatgagtaaacttggtctgacagttaccaatgcttaatcagtgaggcacctatctcagcgatctgtctatttcgttcatccatagttgcctgactccccgtcgtgtagataactacgatacgggagggcttaccatctggccccagtgctgcaatgataccgcgtgacccacgctcaccggctccagatttatcagcaataaaccagccagccggaagggccgagcgcagaagtggtcctgcaactttatccgcctccatccagtctattaattgttgccgggaagctagagtaagtagttcgccagttaatagtttgcgcaacgttgttgccattgctacaggcatcgtggtgtcacgctcgtcgtttggtatggcttcattcagctccggttcccaacgatcaaggcgagttacatgatcccccatgttgtgcaaaaaagcggttagctccttcggtcctccgatcgttgtcagaagtaagttggccgcagtgttatcactcatggttatggcagcactgcataattctcttactgtcatgccatccgtaagatgcttttctgtgactggtgagtactcaaccaagtcattctgagaatagtgtatgcggcgaccgagttgctcttgcccggcgtcaatacgggataataccgcgccacatagcagaactttaaaagtgctcatcattggaaaacgttcttcggggcgaaaactctcaaggatcttaccgctgttgagatccagttcgatgtaacccactcgtgcacccaactgatcttcagcatcttttactttcaccagcgtttctgggtgagcaaaaacaggaaggcaaaatgccgcaaaaaagggaataagggcgacacggaaatgttgaatactcatactcttcctttttcaatattattgaagcatttatcagggttattgtctcatgagcggatacatatttgaatgtatttagaaaaataaacaaataggggttccgcgcatatttccccgaaaagtgccacctgacgtcgacggatcgggagatctcccgatcccctatggtgcactctcagtacaatctgctctgatgccgcatagttaagccagtatctgctccctgcttgtgtgttggaggtcgctgagtagtgcgcgagcaaaatttaagctacaacaaggcaaggcttgaccgagcaaacaaactctttctgtgttgtaaaacgacggccagtcttaagctcgggccccctgggcggttctgataacgagtaatcgttaatccgcaaataacgtaaaaacccgcttcggcgggtttttttatggggggagtttagggaaagagcatttgtcagaatatttaagggcgcctgtcactttgcttgatatatgagaattatttaaccttataaatgagaaaaaagcaacgcactttaaataagatacgttgctttttcgattgatgaacacctataattaaactattcatctattatttatgattttttgtatatacaatatttctagtttgttaaagagaattaagaaaataaatctcgaaaataataaagggaaaatcagtttttgatatcaaaattatacatgtcaacgataatacaaaatataatacaaactataagatgttatcagtatttattatgcatttagaataaattttgtgtcgcccttattcgactcactatagaagttcctattctctagaaagtagaggaacttcacttcattttgctagcgtgtgagggcctatttcccatgattccttcatatttgcatatacgatacaaggctgttagagagataattggaattaatttgactgtaaacacaaagatattagtacaaaatacgtgacgtagaaagtaataatttcttgggtagtttgcagttttaaaattatgttttaaaatggactatcatatgcttaccgtaacttgaaagtatttcgatttcttggctttatatatcttgtggaaaggacgaaacaccgttagctataggctaataagatagttgtgtcaagtgcttcggagacctaacacgtctccagtcacaacggctaaaaatagcca

SEQ ID NO: 131 - DNA, 3364 bp, synthetic construct
  misc_feature 1..3364: note = plasmid including the sequence for B-Gen.1 human albumin target 9
  source 1..3364: mol_type = other DNA
gcacatttctaaaatggcatagtatttttttttgttttcaacaccggtaccgcgttacaatgataagtcgactgaataagtgaactcgagatcagcctcgactgtgccttctagttgccagccatctgttgtttgcccctcccccgtgccttccttgaccctggaaggtgccactcccactgtcctttcctaataaaatgaggaaattgcatccccacttcagaagttcctatactttctagtgaatgagtgagctaactcacattaattgcgttgcgctcactgcccgctttccagtcgggaaacctgtcgtgccagctgcattaatgaatcggccaacgcgcggggagaggcggtttgcgtattgggcgctcttgcgcttcctcgctcactgactcgctgcgctcggtcgttcggctgcggcgagcggtatcagctcactcaaaggcggtaatacggttatccacagaatcaggggataacgcaggaaagaacatgtgagcaaaaggccagcaaaaggccaggaaccgtaaaaaggccgcgttgctggcgtttttccataggctccgcccccctgacgagcatcacaaaaatcgacgctcaagtcagaggtggcgaaacccgacaggactataaagataccaggcgtttccccctggaagctccctcgtgcgctctcctgttccgaccctgccgcttaccggatacctgtccgcctttctcccttcgggaagcgtggcgctttctcatagctcacgctgtaggtatctcagttcggtgtaggtcgttcgctccaagctgggctgtgtgcacgaaccccccgttcagcccgaccgctgcgccttatccggtaactatcgtcttgagtccaacccggtaagacacgacttatcgccactggcagcagccactggtaacaggattagcagagcgaggtatgtaggcggtgctacagagttcttgaagtggtggcctaactacggctacactagaagaacagtatttggtatctgcgctctgctgaagccagttaccttcggaaaaagagttggtagctcttgatccggcaaacaaaccaccgctggtagcggtggtttttttgtttgcaagcagcagattacgcgcagaaaaaaaggatctcaagaagatcctttgatcttttctacggggtctgacgctcagtggaacgaaaactcacgttaagggattttggtcatgagattatcaaaaaggatcttcacctagatccttttaaattaaaaatgaagttttaaatcaatctaaagtatatatgagtaaacttggtctgacagttaccaatgcttaatcagtgaggcacctatctcagcgatctgtctatttcgttcatccatagttgcctgactccccgtcgtgtagataactacgatacgggagggcttaccatctggccccagtgctgcaatgataccgcgtgacccacgctcaccggctccagatttatcagcaataaaccagccagccggaagggccgagcgcagaagtggtcctgcaactttatccgcctccatccagtctattaattgttgccgggaagctagagtaagtagttcgccagttaatagtttgcgcaacgttgttgccattgctacaggcatcgtggtgtcacgctcgtcgtttggtatggcttcattcagctccggttcccaacgatcaaggcgagttacatgatcccccatgttgtgcaaaaaagcggttagctccttcggtcctccgatcgttgtcagaagtaagttggccgcagtgttatcactcatggttatggcagcactgcataattctcttactgtcatgccatccgtaagatgcttttctgtgactggtgagtactcaaccaagtcattctgagaatagtgtatgcggcgaccgagttgctcttgcccggcgtcaatacgggataataccgcgccacatagcagaactttaaaagtgctcatcattggaaaacgttcttcggggcgaaaactctcaaggatcttaccgctgttgagatccagttcgatgtaacccactcgtgcacccaactgatcttcagcatcttttactttcaccagcgtttctgggtgagcaaaaacaggaaggcaaaatgccgcaaaaaagggaataagggcgacacggaaatgttgaatactcatactcttcctttttcaatattattgaagcatttatcagggttattgtctcatgagcggatacatatttgaatgtatttagaaaaataaacaaataggggttccgcgcatatttccccgaaaagtgccacctgacgtcgacggatcgggagatctcccgatcccctatggtgcactctcagtacaatctgctctgatgccgcatagttaagccagtatctgctccctgcttgtgtgttggaggtcgctgagtagtgcgcgagcaaaatttaagctacaacaaggcaaggcttgaccgagcaaacaaactctttctgtgttgtaaaacgacggccagtcttaagctcgggccccctgggcggttctgataacgagtaatcgttaatccgcaaataacgtaaaaacccgcttcggcgggtttttttatggggggagtttagggaaagagcatttgtcagaatatttaagggcgcctgtcactttgcttgatatatgagaattatttaaccttataaatgagaaaaaagcaacgcactttaaataagatacgttgctttttcgattgatgaacacctataattaaactattcatctattatttatgattttttgtatatacaatatttctagtttgttaaagagaattaagaaaataaatctcgaaaataataaagggaaaatcagtttttgatatcaaaattatacatgtcaacgataatacaaaatataatacaaactataagatgttatcagtatttattatgcatttagaataaattttgtgtcgcccttattcgactcactatagaagttcctattctctagaaagtagaggaacttcacttcattttgctagcgtgtgagggcctatttcccatgattccttcatatttgcatatacgatacaaggctgttagagagataattggaattaatttgactgtaaacacaaagatattagtacaaaatacgtgacgtagaaagtaataatttcttgggtagtttgcagttttaaaattatgttttaaaatggactatcatatgcttaccgtaacttgaaagtatttcgatttcttggctttatatatcttgtggaaaggacgaaacaccgttagctataggctaataagatagttgtgtcaagtgcttcggagacctaacacgtctccagtcacaacggctaaaaatagcca

SEQ ID NO: 132 - DNA, 3364 bp, synthetic construct
  misc_feature 1..3364: note = plasmid including the sequence for B-Gen.1 human albumin target 10
  source 1..3364: mol_type = other DNA
gcacctaaaatggcatagtattttgtattttttgttttcaacaccggtaccgcgttacaatgataagtcgactgaataagtgaactcgagatcagcctcgactgtgccttctagttgccagccatctgttgtttgcccctcccccgtgccttccttgaccctggaaggtgccactcccactgtcctttcctaataaaatgaggaaattgcatccccacttcagaagttcctatactttctagtgaatgagtgagctaactcacattaattgcgttgcgctcactgcccgctttccagtcgggaaacctgtcgtgccagctgcattaatgaatcggccaacgcgcggggagaggcggtttgcgtattgggcgctcttgcgcttcctcgctcactgactcgctgcgctcggtcgttcggctgcggcgagcggtatcagctcactcaaaggcggtaatacggttatccacagaatcaggggataacgcaggaaagaacatgtgagcaaaaggccagcaaaaggccaggaaccgtaaaaaggccgcgttgctggcgtttttccataggctccgcccccctgacgagcatcacaaaaatcgacgctcaagtcagaggtggcgaaacccgacaggactataaagataccaggcgtttccccctggaagctccctcgtgcgctctcctgttccgaccctgccgcttaccggatacctgtccgcctttctcccttcgggaagcgtggcgctttctcatagctcacgctgtaggtatctcagttcggtgtaggtcgttcgctccaagctgggctgtgtgcacgaaccccccgttcagcccgaccgctgcgccttatccggtaactatcgtcttgagtccaacccggtaagacacgacttatcgccactggcagcagccactggtaacaggattagcagagcgaggtatgtaggcggtgctacagagttcttgaagtggtggcctaactacggctacactagaagaacagtatttggtatctgcgctctgctgaagccagttaccttcggaaaaagagttggtagctcttgatccggcaaacaaaccaccgctggtagcggtggtttttttgtttgcaagcagcagattacgcgcagaaaaaaaggatctcaagaagatcctttgatcttttctacggggtctgacgctcagtggaacgaaaactcacgttaagggattttggtcatgagattatcaaaaaggatcttcacctagatccttttaaattaaaaatgaagttttaaatcaatctaaagtatatatgagtaaacttggtctgacagttaccaatgcttaatcagtgaggcacctatctcagcgatctgtctatttcgttcatccatagttgcctgactccccgtcgtgtagataactacgatacgggagggcttaccatctggccccagtgctgcaatgataccgcgtgacccacgctcaccggctccagatttatcagcaataaaccagccagccggaagggccgagcgcagaagtggtcctgcaactttatccgcctccatccagtctattaattgttgccgggaagctagagtaagtagttcgccagttaatagtttgcgcaacgttgttgccattgctacaggcatcgtggtgtcacgctcgtcgtttggtatggcttcattcagctccggttcccaacgatcaaggcgagttacatgatcccccatgttgtgcaaaaaagcggttagctccttcggtcctccgatcgttgtcagaagtaagttggccgcagtgttatcactcatggttatggcagcactgcataattctcttactgtcatgccatccgtaagatgcttttctgtgactggtgagtactcaaccaagtcattctgagaatagtgtatgcggcgaccgagttgctcttgcccggcgtcaatacgggataataccgcgccacatagcagaactttaaaagtgctcatcattggaaaacgttcttcggggcgaaaactctcaaggatcttaccgctgttgagatccagttcgatgtaacccactcgtgcacccaactgatcttcagcatcttttactttcaccagcgtttctgggtgagcaaaaacaggaaggcaaaatgccgcaaaaaagggaataagggcgacacggaaatgttgaatactcatactcttcctttttcaatattattgaagcatttatcagggttattgtctcatgagcggatacatatttgaatgtatttagaaaaataaacaaataggggttccgcgcatatttccccgaaaagtgccacctgacgtcgacggatcgggagatctcccgatcccctatggtgcactctcagtacaatctgctctgatgccgcatagttaagccagtatctgctccctgcttgtgtgttggaggtcgctgagtagtgcgcgagcaaaatttaagctacaacaaggcaaggcttgaccgagcaaacaaactctttctgtgttgtaaaacgacggccagtcttaagctcgggccccctgggcggttctgataacgagtaatcgttaatccgcaaataacgtaaaaacccgcttcggcgggtttttttatggggggagtttagggaaagagcatttgtcagaatatttaagggcgcctgtcactttgcttgatatatgagaattatttaaccttataaatgagaaaaaagcaacgcactttaaataagatacgttgctttttcgattgatgaacacctataattaaactattcatctattatttatgattttttgtatatacaatatttctagtttgttaaagagaattaagaaaataaatctcgaaaataataaagggaaaatcagtttttgatatcaaaattatacatgtcaacgataatacaaaatataatacaaactataagatgttatcagtatttattatgcatttagaataaattttgtgtcgcccttattcgactcactatagaagttcctattctctagaaagtagaggaacttcacttcattttgctagcgtgtgagggcctatttcccatgattccttcatatttgcatatacgatacaaggctgttagagagataattggaattaatttgactgtaaacacaaagatattagtacaaaatacgtgacgtagaaagtaataatttcttgggtagtttgcagttttaaaattatgttttaaaatggactatcatatgcttaccgtaacttgaaagtatttcgatttcttggctttatatatcttgtggaaaggacgaaacaccgttagctataggctaataagatagttgtgtcaagtgcttcggagacctaacacgtctccagtcacaacggctaaaaatagcca

SEQ ID NO: 133 - DNA, 3364 bp, synthetic construct
  misc_feature 1..3364: note = plasmid including the sequence for B-Gen.1 human albumin target 11
  source 1..3364: mol_type = other DNA
gcactagaaataaatgccaaaataattttttttgttttcaacaccggtaccgcgttacaatgataagtcgactgaataagtgaactcgagatcagcctcgactgtgccttctagttgccagccatctgttgtttgcccctcccccgtgccttccttgaccctggaaggtgccactcccactgtcctttcctaataaaatgaggaaattgcatccccacttcagaagttcctatactttctagtgaatgagtgagctaactcacattaattgcgttgcgctcactgcccgctttccagtcgggaaacctgtcgtgccagctgcattaatgaatcggccaacgcgcggggagaggcggtttgcgtattgggcgctcttgcgcttcctcgctcactgactcgctgcgctcggtcgttcggctgcggcgagcggtatcagctcactcaaaggcggtaatacggttatccacagaatcaggggataacgcaggaaagaacatgtgagcaaaaggccagcaaaaggccaggaaccgtaaaaaggccgcgttgctggcgtttttccataggctccgcccccctgacgagcatcacaaaaatcgacgctcaagtcagaggtggcgaaacccgacaggactataaagataccaggcgtttccccctggaagctccctcgtgcgctctcctgttccgaccctgccgcttaccggatacctgtccgcctttctcccttcgggaagcgtggcgctttctcatagctcacgctgtaggtatctcagttcggtgtaggtcgttcgctccaagctgggctgtgtgcacgaaccccccgttcagcccgaccgctgcgccttatccggtaactatcgtcttgagtccaacccggtaagacacgacttatcgccactggcagcagccactggtaacaggattagcagagcgaggtatgtaggcggtgctacagagttcttgaagtggtggcctaactacggctacactagaagaacagtatttggtatctgcgctctgctgaagccagttaccttcggaaaaagagttggtagctcttgatccggcaaacaaaccaccgctggtagcggtggtttttttgtttgcaagcagcagattacgcgcagaaaaaaaggatctcaagaagatcctttgatcttttctacggggtctgacgctcagtggaacgaaaactcacgttaagggattttggtcatgagattatcaaaaaggatcttcacctagatccttttaaattaaaaatgaagttttaaatcaatctaaagtatatatgagtaaacttggtctgacagttaccaatgcttaatcagtgaggcacctatctcagcgatctgtctatttcgttcatccatagttgcctgactccccgtcgtgtagataactacgatacgggagggcttaccatctggccccagtgctgcaatgataccgcgtgacccacgctcaccggctccagatttatcagcaataaaccagccagccggaagggccgagcgcagaagtggtcctgcaactttatccgcctccatccagtctattaattgttgccgggaagctagagtaagtagttcgccagttaatagtttgcgcaacgttgttgccattgctacaggcatcgtggtgtcacgctcgtcgtttggtatggcttcattcagctccggttcccaacgatcaaggcgagttacatgatcccccatgttgtgcaaaaaagcggttagctccttcggtcctccgatcgttgtcagaagtaagttggccgcagtgttatcactcatggttatggcagcactgcataattctcttactgtcatgccatccgtaagatgcttttctgtgactggtgagtactcaaccaagtcattctgagaatagtgtatgcggcgaccgagttgctcttgcccggcgtcaatacgggataataccgcgccacatagcagaactttaaaagtgctcatcattggaaaacgttcttcggggcgaaaactctcaaggatcttaccgctgttgagatccagttcgatgtaacccactcgtgcacccaactgatcttcagcatcttttactttcaccagcgtttctgggtgagcaaaaacaggaaggcaaaatgccgcaaaaaagggaataagggcgacacggaaatgttgaatactcatactcttcctttttcaatattattgaagcatttatcagggttattgtctcatgagcggatacatatttgaatgtatttagaaaaataaacaaataggggttccgcgcatatttccccgaaaagtgccacctgacgtcgacggatcgggagatctcccgatcccctatggtgcactctcagtacaatctgctctgatgccgcatagttaagccagtatctgctccctgcttgtgtgttggaggtcgctgagtagtgcgcgagcaaaatttaagctacaacaaggcaaggcttgaccgagcaaacaaactctttctgtgttgtaaaacgacggccagtcttaagctcgggccccctgggcggttctgataacgagtaatcgttaatccgcaaataacgtaaaaacccgcttcggcgggtttttttatggggggagtttagggaaagagcatttgtcagaatatttaagggcgcctgtcactttgcttgatatatgagaattatttaaccttataaatgagaaaaaagcaacgcactttaaataagatacgttgctttttcgattgatgaacacctataattaaactattcatctattatttatgattttttgtatatacaatatttctagtttgttaaagagaattaagaaaataaatctcgaaaataataaagggaaaatcagtttttgatatcaaaattatacatgtcaacgataatacaaaatataatacaaactataagatgttatcagtatttattatgcatttagaataaattttgtgtcgcccttattcgactcactatagaagttcctattctctagaaagtagaggaacttcacttcattttgctagcgtgtgagggcctatttcccatgattccttcatatttgcatatacgatacaaggctgttagagagataattggaattaatttgactgtaaacacaaagatattagtacaaaatacgtgacgtagaaagtaataatttcttgggtagtttgcagttttaaaattatgttttaaaatggactatcatatgcttaccgtaacttgaaagtatttcgatttcttggctttatatatcttgtggaaaggacgaaacaccgttagctataggctaataagatagttgtgtcaagtgcttcggagacctaacacgtctccagtcacaacggctaaaaatagcca

SEQ ID NO: 134 - DNA, 3364 bp, synthetic construct
  misc_feature 1..3364: note = plasmid including the sequence for B-Gen.1 human albumin target 12
  source 1..3364: mol_type = other DNA
gcactgtatttgtgaagtcttacaaggttttttgttttcaacaccggtaccgcgttacaatgataagtcgactgaataagtgaactcgagatcagcctcgactgtgccttctagttgccagccatctgttgtttgcccctcccccgtgccttccttgaccctggaaggtgccactcccactgtcctttcctaataaaatgaggaaattgcatccccacttcagaagttcctatactttctagtgaatgagtgagctaactcacattaattgcgttgcgctcactgcccgctttccagtcgggaaacctgtcgtgccagctgcattaatgaatcggccaacgcgcggggagaggcggtttgcgtattgggcgctcttgcgcttcctcgctcactgactcgctgcgctcggtcgttcggctgcggcgagcggtatcagctcactcaaaggcggtaatacggttatccacagaatcaggggataacgcaggaaagaacatgtgagcaaaaggccagcaaaaggccaggaaccgtaaaaaggccgcgttgctggcgtttttccataggctccgcccccctgacgagcatcacaaaaatcgacgctcaagtcagaggtggcgaaacccgacaggactataaagataccaggcgtttccccctggaagctccctcgtgcgctctcctgttccgaccctgccgcttaccggatacctgtccgcctttctcccttcgggaagcgtggcgctttctcatagctcacgctgtaggtatctcagttcggtgtaggtcgttcgctccaagctgggctgtgtgcacgaaccccccgttcagcccgaccgctgcgccttatccggtaactatcgtcttgagtccaacccggtaagacacgacttatcgccactggcagcagccactggtaacaggattagcagagcgaggtatgtaggcggtgctacagagttcttgaagtggtggcctaactacggctacactagaagaacagtatttggtatctgcgctctgctgaagccagttaccttcggaaaaagagttggtagctcttgatccggcaaacaaaccaccgctggtagcggtggtttttttgtttgcaagcagcagattacgcgcagaaaaaaaggatctcaagaagatcctttgatcttttctacggggtctgacgctcagtggaacgaaaactcacgttaagggattttggtcatgagattatcaaaaaggatcttcacctagatccttttaaattaaaaatgaagttttaaatcaatctaaagtatatatgagtaaacttggtctgacagttaccaatgcttaatcagtgaggcacctatctcagcgatctgtctatttcgttcatccatagttgcctgactccccgtcgtgtagataactacgatacgggagggcttaccatctggccccagtgctgcaatgataccgcgtgacccacgctcaccggctccagatttatcagcaataaaccagccagccggaagggccgagcgcagaagtggtcctgcaactttatccgcctccatccagtctattaattgttgccgggaagctagagtaagtagttcgccagttaatagtttgcgcaacgttgttgccattgctacaggcatcgtggtgtcacgctcgtcgtttggtatggcttcattcagctccggttcccaacgatcaaggcgagttacatgatcccccatgttgtgcaaaaaagcggttagctccttcggtcctccgatcgttgtcagaagtaagttggccgcagtgttatcactcatggttatggcagcactgcataattctcttactgtcatgccatccgtaagatgcttttctgtgactggtgagtactcaaccaagtcattctgagaatagtgtatgcggcgaccgagttgctcttgcccggcgtcaatacgggataataccgcgccacatagcagaactttaaaagtgctcatcattggaaaacgttcttcggggcgaaaactctcaaggatcttaccgctgttgagatccagttcgatgtaacccactcgtgcacccaactgatcttcagcatcttttactttcaccagcgtttctgggtgagcaaaaacaggaaggcaaaatgccgcaaaaaagggaataagggcgacacggaaatgttgaatactcatactcttcctttttcaatattattgaagcatttatcagggttattgtctcatgagcggatacatatttgaatgtatttagaaaaataaacaaataggggttccgcgcatatttccccgaaaagtgccacctgacgtcgacggatcgggagatctcccgatcccctatggtgcactctcagtacaatctgctctgatgccgcatagttaagccagtatctgctccctgcttgtgtgttggaggtcgctgagtagtgcgcgagcaaaatttaagctacaacaaggcaaggcttgaccgagcaaacaaactctttctgtgttgtaaaacgacggccagtcttaagctcgggccccctgggcggttctgataacgagtaatcgttaatccgcaaataacgtaaaaacccgcttcggcgggtttttttatggggggagtttagggaaagagcatttgtcagaatatttaagggcgcctgtcactttgcttgatatatgagaattatttaaccttataaatgagaaaaaagcaacgcactttaaataagatacgttgctttttcgattgatgaacacctataattaaactattcatctattatttatgattttttgtatatacaatatttctagtttgttaaagagaattaagaaaataaatctcgaaaataataaagggaaaatcagtttttgatatcaaaattatacatgtcaacgataatacaaaatataatacaaactataagatgttatcagtatttattatgcatttagaataaattttgtgtcgcccttattcgactcactatagaagttcctattctctagaaagtagaggaacttcacttcattttgctagcgtgtgagggcctatttcccatgattccttcatatttgcatatacgatacaaggctgttagagagataattggaattaatttgactgtaaacacaaagatattagtacaaaatacgtgacgtagaaagtaataatttcttgggtagtttgcagttttaaaattatgttttaaaatggactatcatatgcttaccgtaacttgaaagtatttcgatttcttggctttatatatcttgtggaaaggacgaaacaccgttagctataggctaataagatagttgtgtcaagtgcttcggagacctaacacgtctccagtcacaacggctaaaaatagcca

SEQ ID NO: 135 - DNA, 3364 bp, synthetic construct
  misc_feature 1..3364: note = plasmid including the sequence for B-Gen.1 human albumin target 13
  source 1..3364: mol_type = other DNA
gcacgtgaagtcttacaaggttatcttttttttgttttcaacaccggtaccgcgttacaatgataagtcgactgaataagtgaactcgagatcagcctcgactgtgccttctagttgccagccatctgttgtttgcccctcccccgtgccttccttgaccctggaaggtgccactcccactgtcctttcctaataaaatgaggaaattgcatccccacttcagaagttcctatactttctagtgaatgagtgagctaactcacattaattgcgttgcgctcactgcccgctttccagtcgggaaacctgtcgtgccagctgcattaatgaatcggccaacgcgcggggagaggcggtttgcgtattgggcgctcttgcgcttcctcgctcactgactcgctgcgctcggtcgttcggctgcggcgagcggtatcagctcactcaaaggcggtaatacggttatccacagaatcaggggataacgcaggaaagaacatgtgagcaaaaggccagcaaaaggccaggaaccgtaaaaaggccgcgttgctggcgtttttccataggctccgcccccctgacgagcatcacaaaaatcgacgctcaagtcagaggtggcgaaacccgacaggactataaagataccaggcgtttccccctggaagctccctcgtgcgctctcctgttccgaccctgccgcttaccggatacctgtccgcctttctcccttcgggaagcgtggcgctttctcatagctcacgctgtaggtatctcagttcggtgtaggtcgttcgctccaagctgggctgtgtgcacgaaccccccgttcagcccgaccgctgcgccttatccggtaactatcgtcttgagtccaacccggtaagacacgacttatcgccactggcagcagccactggtaacaggattagcagagcgaggtatgtaggcggtgctacagagttcttgaagtggtggcctaactacggctacactagaagaacagtatttggtatctgcgctctgctgaagccagttaccttcggaaaaagagttggtagctcttgatccggcaaacaaaccaccgctggtagcggtggtttttttgtttgcaagcagcagattacgcgcagaaaaaaaggatctcaagaagatcctttgatcttttctacggggtctgacgctcagtggaacgaaaactcacgttaagggattttggtcatgagattatcaaaaaggatcttcacctagatccttttaaattaaaaatgaagttttaaatcaatctaaagtatatatgagtaaacttggtctgacagttaccaatgcttaatcagtgaggcacctatctcagcgatctgtctatttcgttcatccatagttgcctgactccccgtcgtgtagataactacgatacgggagggcttaccatctggccccagtgctgcaatgataccgcgtgacccacgctcaccggctccagatttatcagcaataaaccagccagccggaagggccgagcgcagaagtggtcctgcaactttatccgcctccatccagtctattaattgttgccgggaagctagagtaagtagttcgccagttaatagtttgcgcaacgttgttgccattgctacaggcatcgtggtgtcacgctcgtcgtttggtatggcttcattcagctccggttcccaacgatcaaggcgagttacatgatcccccatgttgtgcaaaaaagcggttagctccttcggtcctccgatcgttgtcagaagtaagttggccgcagtgttatcactcatggttatggcagcactgcataattctcttactgtcatgccatccgtaagatgcttttctgtgactggtgagtactcaaccaagtcattctgagaatagtgtatgcggcgaccgagttgctcttgcccggcgtcaatacgggataataccgcgccacatagcagaactttaaaagtgctcatcattggaaaacgttcttcggggcgaaaactctcaaggatcttaccgctgttgagatccagttcgatgtaacccactcgtgcacccaactgatcttcagcatcttttactttcaccagcgtttctgggtgagcaaaaacaggaaggcaaaatgccgcaaaaaagggaataagggcgacacggaaatgttgaatactcatactcttcctttttcaatattattgaagcatttatcagggttattgtctcatgagcggatacatatttgaatgtatttagaaaaataaacaaataggggttccgcgcatatttccccgaaaagtgccacctgacgtcgacggatcgggagatctcccgatcccctatggtgcactctcagtacaatctgctctgatgccgcatagttaagccagtatctgctccctgcttgtgtgttggaggtcgctgagtagtgcgcgagcaaaatttaagctacaacaaggcaaggcttgaccgagcaaacaaactctttctgtgttgtaaaacgacggccagtcttaagctcgggccccctgggcggttctgataacgagtaatcgttaatccgcaaataacgtaaaaacccgcttcggcgggtttttttatggggggagtttagggaaagagcatttgtcagaatatttaagggcgcctgtcactttgcttgatatatgagaattatttaaccttataaatgagaaaaaagcaacgcactttaaataagatacgttgctttttcgattgatgaacacctataattaaactattcatctattatttatgattttttgtatatacaatatttctagtttgttaaagagaattaagaaaataaatctcgaaaataataaagggaaaatcagtttttgatatcaaaattatacatgtcaacgataatacaaaatataatacaaactataagatgttatcagtatttattatgcatttagaataaattttgtgtcgcccttattcgactcactatagaagttcctattctctagaaagtagaggaacttcacttcattttgctagcgtgtgagggcctatttcccatgattccttcatatttgcatatacgatacaaggctgttagagagataattggaattaatttgactgtaaacacaaagatattagtacaaaatacgtgacgtagaaagtaataatttcttgggtagtttgcagttttaaaattatgttttaaaatggactatcatatgcttaccgtaacttgaaagtatttcgatttcttggctttatatatcttgtggaaaggacgaaacaccgttagctataggctaataagatagttgtgtcaagtgcttcggagacctaacacgtctccagtcacaacggctaaaaatagcca

SEQ ID NO: 136 - DNA, 3364 bp, synthetic construct
  misc_feature 1..3364: note = plasmid including the sequence for B-Gen.1 human albumin target 14
  source 1..3364: mol_type = other DNA
gcacataaaattcaaacatcctaggtattttttgttttcaacaccggtaccgcgttacaatgataagtcgactgaataagtgaactcgagatcagcctcgactgtgccttctagttgccagccatctgttgtttgcccctcccccgtgccttccttgaccctggaaggtgccactcccactgtcctttcctaataaaatgaggaaattgcatccccacttcagaagttcctatactttctagtgaatgagtgagctaactcacattaattgcgttgcgctcactgcccgctttccagtcgggaaacctgtcgtgccagctgcattaatgaatcggccaacgcgcggggagaggcggtttgcgtattgggcgctcttgcgcttcctcgctcactgactcgctgcgctcggtcgttcggctgcggcgagcggtatcagctcactcaaaggcggtaatacggttatccacagaatcaggggataacgcaggaaagaacatgtgagcaaaaggccagcaaaaggccaggaaccgtaaaaaggccgcgttgctggcgtttttccataggctccgcccccctgacgagcatcacaaaaatcgacgctcaagtcagaggtggcgaaacccgacaggactataaagataccaggcgtttccccctggaagctccctcgtgcgctctcctgttccgaccctgccgcttaccggatacctgtccgcctttctcccttcgggaagcgtggcgctttctcatagctcacgctgtaggtatctcagttcggtgtaggtcgttcgctccaagctgggctgtgtgcacgaaccccccgttcagcccgaccgctgcgccttatccggtaactatcgtcttgagtccaacccggtaagacacgacttatcgccactggcagcagccactggtaacaggattagcagagcgaggtatgtaggcggtgctacagagttcttgaagtggtggcctaactacggctacactagaagaacagtatttggtatctgcgctctgctgaagccagttaccttcggaaaaagagttggtagctcttgatccggcaaacaaaccaccgctggtagcggtggtttttttgtttgcaagcagcagattacgcgcagaaaaaaaggatctcaagaagatcctttgatcttttctacggggtctgacgctcagtggaacgaaaactcacgttaagggattttggtcatgagattatcaaaaaggatcttcacctagatccttttaaattaaaaatgaagttttaaatcaatctaaagtatatatgagtaaacttggtctgacagttaccaatgcttaatcagtgaggcacctatctcagcgatctgtctatttcgttcatccatagttgcctgactccccgtcgtgtagataactacgatacgggagggcttaccatctggccccagtgctgcaatgataccgcgtgacccacgctcaccggctccagatttatcagcaataaaccagccagccggaagggccgagcgcagaagtggtcctgcaactttatccgcctccatccagtctattaattgttgccgggaagctagagtaagtagttcgccagttaatagtttgcgcaacgttgttgccattgctacaggcatcgtggtgtcacgctcgtcgtttggtatggcttcattcagctccggttcccaacgatcaaggcgagttacatgatcccccatgttgtgcaaaaaagcggttagctccttcggtcctccgatcgttgtcagaagtaagttggccgcagtgttatcactcatggttatggcagcactgcataattctcttactgtcatgccatccgtaagatgcttttctgtgactggtgagtactcaaccaagtcattctgagaatagtgtatgcggcgaccgagttgctcttgcccggcgtcaatacgggataataccgcgccacatagcagaactttaaaagtgctcatcattggaaaacgttcttcggggcgaaaactctcaaggatcttaccgctgttgagatccagttcgatgtaacccactcgtgcacccaactgatcttcagcatcttttactttcaccagcgtttctgggtgagcaaaaacaggaaggcaaaatgccgcaaaaaagggaataagggcgacacggaaatgttgaatactcatactcttcctttttcaatattattgaagcatttatcagggttattgtctcatgagcggatacatatttgaatgtatttagaaaaataaacaaataggggttccgcgcatatttccccgaaaagtgccacctgacgtcgacggatcgggagatctcccgatcccctatggtgcactctcagtacaatctgctctgatgccgcatagttaagccagtatctgctccctgcttgtgtgttggaggtcgctgagtagtgcgcgagcaaaatttaagctacaacaaggcaaggcttgaccgagcaaacaaactctttctgtgttgtaaaacgacggccagtcttaagctcgggccccctgggcggttctgataacgagtaatcgttaatccgcaaataacgtaaaaacccgcttcggcgggtttttttatggggggagtttagggaaagagcatttgtcagaatatttaagggcgcctgtcactttgcttgatatatgagaattatttaaccttataaatgagaaaaaagcaacgcactttaaataagatacgttgctttttcgattgatgaacacctataattaaactattcatctattatttatgattttttgtatatacaatatttctagtttgttaaagagaattaagaaaataaatctcgaaaataataaagggaaaatcagtttttgatatcaaaattatacatgtcaacgataatacaaaatataatacaaactataagatgttatcagtatttattatgcatttagaataaattttgtgtcgcccttattcgactcactatagaagttcctattctctagaaagtagaggaacttcacttcattttgctagcgtgtgagggcctatttcccatgattccttcatatttgcatatacgatacaaggctgttagagagataattggaattaatttgactgtaaacacaaagatattagtacaaaatacgtgacgtagaaagtaataatttcttgggtagtttgcagttttaaaattatgttttaaaatggactatcatatgcttaccgtaacttgaaagtatttcgatttcttggctttatatatcttgtggaaaggacgaaacaccgttagctataggctaataagatagttgtgtcaagtgcttcggagacctaacacgtctccagtcacaacggctaaaaatagcca

SEQ ID NO: 137 - DNA, 3364 bp, synthetic construct
  misc_feature 1..3364: note = plasmid including the sequence for B-Gen.1 human albumin target 15
  source 1..3364: mol_type = other DNA
gcacataagataaccttgtaagacttcttttttgttttcaacaccggtaccgcgttacaatgataagtcgactgaataagtgaactcgagatcagcctcgactgtgccttctagttgccagccatctgttgtttgcccctcccccgtgccttccttgaccctggaaggtgccactcccactgtcctttcctaataaaatgaggaaattgcatccccacttcagaagttcctatactttctagtgaatgagtgagctaactcacattaattgcgttgcgctcactgcccgctttccagtcgggaaacctgtcgtgccagctgcattaatgaatcggccaacgcgcggggagaggcggtttgcgtattgggcgctcttgcgcttcctcgctcactgactcgctgcgctcggtcgttcggctgcggcgagcggtatcagctcactcaaaggcggtaatacggttatccacagaatcaggggataacgcaggaaagaacatgtgagcaaaaggccagcaaaaggccaggaaccgtaaaaaggccgcgttgctggcgtttttccataggctccgcccccctgacgagcatcacaaaaatcgacgctcaagtcagaggtggcgaaacccgacaggactataaagataccaggcgtttccccctggaagctccctcgtgcgctctcctgttccgaccctgccgcttaccggatacctgtccgcctttctcccttcgggaagcgtggcgctttctcatagctcacgctgtaggtatctcagttcggtgtaggtcgttcgctccaagctgggctgtgtgcacgaaccccccgttcagcccgaccgctgcgccttatccggtaactatcgtcttgagtccaacccggtaagacacgacttatcgccactggcagcagccactggtaacaggattagcagagcgaggtatgtaggcggtgctacagagttcttgaagtggtggcctaactacggctacactagaagaacagtatttggtatctgcgctctgctgaagccagttaccttcggaaaaagagttggtagctcttgatccggcaaacaaaccaccgctggtagcggtggtttttttgtttgcaagcagcagattacgcgcagaaaaaaaggatctcaagaagatcctttgatcttttctacggggtctgacgctcagtggaacgaaaactcacgttaagggattttggtcatgagattatcaaaaaggatcttcacctagatccttttaaattaaaaatgaagttttaaatcaatctaaagtatatatgagtaaacttggtctgacagttaccaatgcttaatcagtgaggcacctatctcagcgatctgtctatttcgttcatccatagttgcctgactccccgtcgtgtagataactacgatacgggagggcttaccatctggccccagtgctgcaatgataccgcgtgacccacgctcaccggctccagatttatcagcaataaaccagccagccggaagggccgagcgcagaagtggtcctgcaactttatccgcctccatccagtctattaattgttgccgggaagctagagtaagtagttcgccagttaatagtttgcgcaacgttgttgccattgctacaggcatcgtggtgtcacgctcgtcgtttggtatggcttcattcagctccggttcccaacgatcaaggcgagttacatgatcccccatgttgtgcaaaaaagcggttagctccttcggtcctccgatcgttgtcagaagtaagttggccgcagtgttatcactcatggttatggcagcactgcataattctcttactgtcatgccatccgtaagatgcttttctgtgactggtgagtactcaaccaagtcattctgagaatagtgtatgcggcgaccgagttgctcttgcccggcgtcaatacgggataataccgcgccacatagcagaactttaaaagtgctcatcattggaaaacgttcttcggggcgaaaactctcaaggatcttaccgctgttgagatccagttcgatgtaacccactcgtgcacccaactgatcttcagcatcttttactttcaccagcgtttctgggtgagcaaaaacaggaaggcaaaatgccgcaaaaaagggaataagggcgacacggaaatgttgaatactcatactcttcctttttcaatattattgaagcatttatcagggttattgtctcatgagcggatacatatttgaatgtatttagaaaaataaacaaataggggttccgcgcatatttccccgaaaagtgccacctgacgtcgacggatcgggagatctcccgatcccctatggtgcactctcagtacaatctgctctgatgccgcatagttaagccagtatctgctccctgcttgtgtgttggaggtcgctgagtagtgcgcgagcaaaatttaagctacaacaaggcaaggcttgaccgagcaaacaaactctttctgtgttgtaaaacgacggccagtcttaagctcgggccccctgggcggttctgataacgagtaatcgttaatccgcaaataacgtaaaaacccgcttcggcgggtttttttatggggggagtttagggaaagagcatttgtcagaatatttaagggcgcctgtcactttgcttgatatatgagaattatttaaccttataaatgagaaaaaagcaacgcactttaaataagatacgttgctttttcgattgatgaacacctataattaaactattcatctattatttatgattttttgtatatacaatatttctagtttgttaaagagaattaagaaaataaatctcgaaaataataaagggaaaatcagtttttgatatcaaaattatacatgtcaacgataatacaaaatataatacaaactataagatgttatcagtatttattatgcatttagaataaattttgtgtcgcccttattcgactcactatagaagttcctattctctagaaagtagaggaacttcacttcattttgctagcgtgtgagggcctatttcccatgattccttcatatttgcatatacgatacaaggctgttagagagataattggaattaatttgactgtaaacacaaagatattagtacaaaatacgtgacgtagaaagtaataatttcttgggtagtttgcagttttaaaattatgttttaaaatggactatcatatgcttaccgtaacttgaaagtatttcgatttcttggctttatatatcttgtggaaaggacgaaacaccgttagctataggctaataagatagttgtgtcaagtgcttcggagacctaacacgtctccagtcacaacggctaaaaatagcca

SEQ ID NO: 138 - DNA, 3364 bp, synthetic construct
  misc_feature 1..3364: note = plasmid including the sequence for B-Gen.1 human albumin target 16
  source 1..3364: mol_type = other DNA
gcactgacctttttttttttttacctattttttgttttcaacaccggtaccgcgttacaatgataagtcgactgaataagtgaactcgagatcagcctcgactgtgccttctagttgccagccatctgttgtttgcccctcccccgtgccttccttgaccctggaaggtgccactcccactgtcctttcctaataaaatgaggaaattgcatccccacttcagaagttcctatactttctagtgaatgagtgagctaactcacattaattgcgttgcgctcactgcccgctttccagtcgggaaacctgtcgtgccagctgcattaatgaatcggccaacgcgcggggagaggcggtttgcgtattgggcgctcttgcgcttcctcgctcactgactcgctgcgctcggtcgttcggctgcggcgagcggtatcagctcactcaaaggcggtaatacggttatccacagaatcaggggataacgcaggaaagaacatgtgagcaaaaggccagcaaaaggccaggaaccgtaaaaaggccgcgttgctggcgtttttccataggctccgcccccctgacgagcatcacaaaaatcgacgctcaagtcagaggtggcgaaacccgacaggactataaagataccaggcgtttccccctggaagctccctcgtgcgctctcctgttccgaccctgccgcttaccggatacctgtccgcctttctcccttcgggaagcgtggcgctttctcatagctcacgctgtaggtatctcagttcggtgtaggtcgttcgctccaagctgggctgtgtgcacgaaccccccgttcagcccgaccgctgcgccttatccggtaactatcgtcttgagtccaacccggtaagacacgacttatcgccactggcagcagccactggtaacaggattagcagagcgaggtatgtaggcggtgctacagagttcttgaagtggtggcctaactacggctacactagaagaacagtatttggtatctgcgctctgctgaagccagttaccttcggaaaaagagttggtagctcttgatccggcaaacaaaccaccgctggtagcggtggtttttttgtttgcaagcagcagattacgcgcagaaaaaaaggatctcaagaagatcctttgatcttttctacggggtctgacgctcagtggaacgaaaactcacgttaagggattttggtcatgagattatcaaaaaggatcttcacctagatccttttaaattaaaaatgaagttttaaatcaatctaaagtatatatgagtaaacttggtctgacagttaccaatgcttaatcagtgaggcacctatctcagcgatctgtctatttcgttcatccatagttgcctgactccccgtcgtgtagataactacgatacgggagggcttaccatctggccccagtgctgcaatgataccgcgtgacccacgctcaccggctccagatttatcagcaataaaccagccagccggaagggccgagcgcagaagtggtcctgcaactttatccgcctccatccagtctattaattgttgccgggaagctagagtaagtagttcgccagttaatagtttgcgcaacgttgttgccattgctacaggcatcgtggtgtcacgctcgtcgtttggtatggcttcattcagctccggttcccaacgatcaaggcgagttacatgatcccccatgttgtgcaaaaaagcggttagctccttcggtcctccgatcgttgtcagaagtaagttggccgcagtgttatcactcatggttatggcagcactgcataattctcttactgtcatgccatccgtaagatgcttttctgtgactggtgagtactcaaccaagtcattctgagaatagtgtatgcggcgaccgagttgctcttgcccggcgtcaatacgggataataccgcgccacatagcagaactttaaaagtgctcatcattggaaaacgttcttcggggcgaaaactctcaaggatcttaccgctgttgagatccagttcgatgtaacccactcgtgcacccaactgatcttcagcatcttttactttcaccagcgtttctgggtgagcaaaaacaggaaggcaaaatgccgcaaaaaagggaataagggcgacacggaaatgttgaatactcatactcttcctttttcaatattattgaagcatttatcagggttattgtctcatgagcggatacatatttgaatgtatttagaaaaataaacaaataggggttccgcgcatatttccccgaaaagtgccacctgacgtcgacggatcgggagatctcccgatcccctatggtgcactctcagtacaatctgctctgatgccgcatagttaagccagtatctgctccctgcttgtgtgttggaggtcgctgagtagtgcgcgagcaaaatttaagctacaacaaggcaaggcttgaccgagcaaacaaactctttctgtgttgtaaaacgacggccagtcttaagctcgggccccctgggcggttctgataacgagtaatcgttaatccgcaaataacgtaaaaacccgcttcggcgggtttttttatggggggagtttagggaaagagcatttgtcagaatatttaagggcgcctgtcactttgcttgatatatgagaattatttaaccttataaatgagaaaaaagcaacgcactttaaataagatacgttgctttttcgattgatgaacacctataattaaactattcatctattatttatgattttttgtatatacaatatttctagtttgttaaagagaattaagaaaataaatctcgaaaataataaagggaaaatcagtttttgatatcaaaattatacatgtcaacgataatacaaaatataatacaaactataagatgttatcagtatttattatgcatttagaataaattttgtgtcgcccttattcgactcactatagaagttcctattctctagaaagtagaggaacttcacttcattttgctagcgtgtgagggcctatttcccatgattccttcatatttgcatatacgatacaaggctgttagagagataattggaattaatttgactgtaaacacaaagatattagtacaaaatacgtgacgtagaaagtaataatttcttgggtagtttgcagttttaaaattatgttttaaaatggactatcatatgcttaccgtaacttgaaagtatttcgatttcttggctttatatatcttgtggaaaggacgaaacaccgttagctataggctaataagatagttgtgtcaagtgcttcggagacctaacacgtctccagtcacaacggctaaaaatagcca

SEQ ID NO: 139 - DNA, 3364 bp, synthetic construct
  misc_feature 1..3364: note = plasmid including the sequence for B-Gen.1 human albumin target 17
  source 1..3364: mol_type = other DNA
gcactttagtgactgtaattttcttttttttttgttttcaacaccggtaccgcgttacaatgataagtcgactgaataagtgaactcgagatcagcctcgactgtgccttctagttgccagccatctgttgtttgcccctcccccgtgccttccttgaccctggaaggtgccactcccactgtcctttcctaataaaatgaggaaattgcatccccacttcagaagttcctatactttctagtgaatgagtgagctaactcacattaattgcgttgcgctcactgcccgctttccagtcgggaaacctgtcgtgccagctgcattaatgaatcggccaacgcgcggggagaggcggtttgcgtattgggcgctcttgcgcttcctcgctcactgactcgctgcgctcggtcgttcggctgcggcgagcggtatcagctcactcaaaggcggtaatacggttatccacagaatcaggggataacgcaggaaagaacatgtgagcaaaaggccagcaaaaggccaggaaccgtaaaaaggccgcgttgctggcgtttttccataggctccgcccccctgacgagcatcacaaaaatcgacgctcaagtcagaggtggcgaaacccgacaggactataaagataccaggcgtttccccctggaagctccctcgtgcgctctcctgttccgaccctgccgcttaccggatacctgtccgcctttctcccttcgggaagcgtggcgctttctcatagctcacgctgtaggtatctcagttcggtgtaggtcgttcgctccaagctgggctgtgtgcacgaaccccccgttcagcccgaccgctgcgccttatccggtaactatcgtcttgagtccaacccggtaagacacgacttatcgccactggcagcagccactggtaacaggattagcagagcgaggtatgtaggcggtgctacagagttcttgaagtggtggcctaactacggctacactagaagaacagtatttggtatctgcgctctgctgaagccagttaccttcggaaaaagagttggtagctcttgatccggcaaacaaaccaccgctggtagcggtggtttttttgtttgcaagcagcagattacgcgcagaaaaaaaggatctcaagaagatcctttgatcttttctacggggtctgacgctcagtggaacgaaaactcacgttaagggattttggtcatgagattatcaaaaaggatcttcacctagatccttttaaattaaaaatgaagttttaaatcaatctaaagtatatatgagtaaacttggtctgacagttaccaatgcttaatcagtgaggcacctatctcagcgatctgtctatttcgttcatccatagttgcctgactccccgtcgtgtagataactacgatacgggagggcttaccatctggccccagtgctgcaatgataccgcgtgacccacgctcaccggctccagatttatcagcaataaaccagccagccggaagggccgagcgcagaagtggtcctgcaactttatccgcctccatccagtctattaattgttgccgggaagctagagtaagtagttcgccagttaatagtttgcgcaacgttgttgccattgctacaggcatcgtggtgtcacgctcgtcgtttggtatggcttcattcagctccggttcccaacgatcaaggcgagttacatgatcccccatgttgtgcaaaaaagcggttagctccttcggtcctccgatcgttgtcagaagtaagttggccgcagtgttatcactcatggttatggcagcactgcataattctcttactgtcatgccatccgtaagatgcttttctgtgactggtgagtactcaaccaagtcattctgagaatagtgtatgcggcgaccgagttgctcttgcccggcgtcaatacgggataataccgcgccacatagcagaactttaaaagtgctcatcattggaaaacgttcttcggggcgaaaactctcaaggatcttaccgctgttgagatccagttcgatgtaacccactcgtgcacccaactgatcttcagcatcttttactttcaccagcgtttctgggtgagcaaaaacaggaaggcaaaatgccgcaaaaaagggaataagggcgacacggaaatgttgaatactcatactcttcctttttcaatattattgaagcatttatcagggttattgtctcatgagcggatacatatttgaatgtatttagaaaaataaacaaataggggttccgcgcatatttccccgaaaagtgccacctgacgtcgacggatcgggagatctcccgatcccctatggtgcactctcagtacaatctgctctgatgccgcatagttaagccagtatctgctccctgcttgtgtgttggaggtcgctgagtagtgcgcgagcaaaatttaagctacaacaaggcaaggcttgaccgagcaaacaaactctttctgtgttgtaaaacgacggccagtcttaagctcgggccccctgggcggttctgataacgagtaatcgttaatccgcaaataacgtaaaaacccgcttcggcgggtttttttatggggggagtttagggaaagagcatttgtcagaatatttaagggcgcctgtcactttgcttgatatatgagaattatttaaccttataaatgagaaaaaagcaacgcactttaaataagatacgttgctttttcgattgatgaacacctataattaaactattcatctattatttatgattttttgtatatacaatatttctagtttgttaaagagaattaagaaaataaatctcgaaaataataaagggaaaatcagtttttgatatcaaaattatacatgtcaacgataatacaaaatataatacaaactataagatgttatcagtatttattatgcatttagaataaattttgtgtcgcccttattcgactcactatagaagttcctattctctagaaagtagaggaacttcacttcattttgctagcgtgtgagggcctatttcccatgattccttcatatttgcatatacgatacaaggctgttagagagataattggaattaatttgactgtaaacacaaagatattagtacaaaatacgtgacgtagaaagtaataatttcttgggtagtttgcagttttaaaattatgttttaaaatggactatcatatgcttaccgtaacttgaaagtatttcgatttcttggctttatatatcttgtggaaaggacgaaacaccgttagctataggctaataagatagttgtgtcaagtgcttcggagacctaacacgtctccagtcacaacggctaaaaatagcca

SEQ ID NO: 140 - DNA, 3364 bp, synthetic construct
  misc_feature 1..3364: note = plasmid including the sequence for B-Gen.1 human albumin target 18
  source 1..3364: mol_type = other DNA
gcaccagtcactaaacaattctgacctttttttgttttcaacaccggtaccgcgttacaatgataagtcgactgaataagtgaactcgagatcagcctcgactgtgccttctagttgccagccatctgttgtttgcccctcccccgtgccttccttgaccctggaaggtgccactcccactgtcctttcctaataaaatgaggaaattgcatccccacttcagaagttcctatactttctagtgaatgagtgagctaactcacattaattgcgttgcgctcactgcccgctttccagtcgggaaacctgtcgtgccagctgcattaatgaatcggccaacgcgcggggagaggcggtttgcgtattgggcgctcttgcgcttcctcgctcactgactcgctgcgctcggtcgttcggctgcggcgagcggtatcagctcactcaaaggcggtaatacggttatccacagaatcaggggataacgcaggaaagaacatgtgagcaaaaggccagcaaaaggccaggaaccgtaaaaaggccgcgttgctggcgtttttccataggctccgcccccctgacgagcatcacaaaaatcgacgctcaagtcagaggtggcgaaacccgacaggactataaagataccaggcgtttccccctggaagctccctcgtgcgctctcctgttccgaccctgccgcttaccggatacctgtccgcctttctcccttcgggaagcgtggcgctttctcatagctcacgctgtaggtatctcagttcggtgtaggtcgttcgctccaagctgggctgtgtgcacgaaccccccgttcagcccgaccgctgcgccttatccggtaactatcgtcttgagtccaacccggtaagacacgacttatcgccactggcagcagccactggtaacaggattagcagagcgaggtatgtaggcggtgctacagagttcttgaagtggtggcctaactacggctacactagaagaacagtatttggtatctgcgctctgctgaagccagttaccttcggaaaaagagttggtagctcttgatccggcaaacaaaccaccgctggtagcggtggtttttttgtttgcaagcagcagattacgcgcagaaaaaaaggatctcaagaagatcctttgatcttttctacggggtctgacgctcagtggaacgaaaactcacgttaagggattttggtcatgagattatcaaaaaggatcttcacctagatccttttaaattaaaaatgaagttttaaatcaatctaaagtatatatgagtaaacttggtctgacagttaccaatgcttaatcagtgaggcacctatctcagcgatctgtctatttcgttcatccatagttgcctgactccccgtcgtgtagataactacgatacgggagggcttaccatctggccccagtgctgcaatgataccgcgtgacccacgctcaccggctccagatttatcagcaataaaccagccagccggaagggccgagcgcagaagtggtcctgcaactttatccgcctccatccagtctattaattgttgccgggaagctagagtaagtagttcgccagttaatagtttgcgcaacgttgttgccattgctacaggcatcgtggtgtcacgctcgtcgtttggtatggcttcattcagctccggttcccaacgatcaaggcgagttacatgatcccccatgttgtgcaaaaaagcggttagctccttcggtcctccgatcgttgtcagaagtaagttggccgcagtgttatcactcatggttatggcagcactgcataattctcttactgtcatgccatccgtaagatgcttttctgtgactggtgagtactcaaccaagtcattctgagaatagtgtatgcggcgaccgagttgctcttgcccggcgtcaatacgggataataccgcgccacatagcagaactttaaaagtgctcatcattggaaaacgttcttcggggcgaaaactctcaaggatcttaccgctgttgagatccagttcgatgtaacccactcgtgcacccaactgatcttcagcatcttttactttcaccagcgtttctgggtgagcaaaaacaggaaggcaaaatgccgcaaaaaagggaataagggcgacacggaaatgttgaatactcatactcttcctttttcaatattattgaagcatttatcagggttattgtctcatgagcggatacatatttgaatgtatttagaaaaataaacaaataggggttccgcgcatatttccccgaaaagtgccacctgacgtcgacggatcgggagatctcccgatcccctatggtgcactctcagtacaatctgctctgatgccgcatagttaagccagtatctgctccctgcttgtgtgttggaggtcgctgagtagtgcgcgagcaaaatttaagctacaacaaggcaaggcttgaccgagcaaacaaactctttctgtgttgtaaaacgacggccagtcttaagctcgggccccctgggcggttctgataacgagtaatcgttaatccgcaaataacgtaaaaacccgcttcggcgggtttttttatggggggagtttagggaaagagcatttgtcagaatatttaagggcgcctgtcactttgcttgatatatgagaattatttaaccttataaatgagaaaaaagcaacgcactttaaataagatacgttgctttttcgattgatgaacacctataattaaactattcatctattatttatgattttttgtatatacaatatttctagtttgttaaagagaattaagaaaataaatctcgaaaataataaagggaaaatcagtttttgatatcaaaattatacatgtcaacgataatacaaaatataatacaaactataagatgttatcagtatttattatgcatttagaataaattttgtgtcgcccttattcgactcactatagaagttcctattctctagaaagtagaggaacttcacttcattttgctagcgtgtgagggcctatttcccatgattccttcatatttgcatatacgatacaaggctgttagagagataattggaattaatttgactgtaaacacaaagatattagtacaaaatacgtgacgtagaaagtaataatttcttgggtagtttgcagttttaaaattatgttttaaaatggactatcatatgcttaccgtaacttgaaagtatttcgatttcttggctttatatatcttgtggaaaggacgaaacaccgttagctataggctaataagatagttgtgtcaagtgcttcggagacctaacacgtctccagtcacaacggctaaaaatagcca

SEQ ID NO: 141 - DNA, 3364 bp, synthetic construct
  misc_feature 1..3364: note = plasmid including the sequence for B-Gen.1 human albumin target 19
  source 1..3364: mol_type = other DNA
gcactcttttgcgcactaaggaaagtgttttttgttttcaacaccggtaccgcgttacaatgataagtcgactgaataagtgaactcgagatcagcctcgactgtgccttctagttgccagccatctgttgtttgcccctcccccgtgccttccttgaccctggaaggtgccactcccactgtcctttcctaataaaatgaggaaattgcatccccacttcagaagttcctatactttctagtgaatgagtgagctaactcacattaattgcgttgcgctcactgcccgctttccagtcgggaaacctgtcgtgccagctgcattaatgaatcggccaacgcgcggggagaggcggtttgcgtattgggcgctcttgcgcttcctcgctcactgactcgctgcgctcggtcgttcggctgcggcgagcggtatcagctcactcaaaggcggtaatacggttatccacagaatcaggggataacgcaggaaagaacatgtgagcaaaaggccagcaaaaggccaggaaccgtaaaaaggccgcgttgctggcgtttttccataggctccgcccccctgacgagcatcacaaaaatcgacgctcaagtcagaggtggcgaaacccgacaggactataaagataccaggcgtttccccctggaagctccctcgtgcgctctcctgttccgaccctgccgcttaccggatacctgtccgcctttctcccttcgggaagcgtggcgctttctcatagctcacgctgtaggtatctcagttcggtgtaggtcgttcgctccaagctgggctgtgtgcacgaaccccccgttcagcccgaccgctgcgccttatccggtaactatcgtcttgagtccaacccggtaagacacgacttatcgccactggcagcagccactggtaacaggattagcagagcgaggtatgtaggcggtgctacagagttcttgaagtggtggcctaactacggctacactagaagaacagtatttggtatctgcgctctgctgaagccagttaccttcggaaaaagagttggtagctcttgatccggcaaacaaaccaccgctggtagcggtggtttttttgtttgcaagcagcagattacgcgcagaaaaaaaggatctcaagaagatcctttgatcttttctacggggtctgacgctcagtggaacgaaaactcacgttaagggattttggtcatgagattatcaaaaaggatcttcacctagatccttttaaattaaaaatgaagttttaaatcaatctaaagtatatatgagtaaacttggtctgacagttaccaatgcttaatcagtgaggcacctatctcagcgatctgtctatttcgttcatccatagttgcctgactccccgtcgtgtagataactacgatacgggagggcttaccatctggccccagtgctgcaatgataccgcgtgacccacgctcaccggctccagatttatcagcaataaaccagccagccggaagggccgagcgcagaagtggtcctgcaactttatccgcctccatccagtctattaattgttgccgggaagctagagtaagtagttcgccagttaatagtttgcgcaacgttgttgccattgctacaggcatcgtggtgtcacgctcgtcgtttggtatggcttcattcagctccggttcccaacgatcaaggcgagttacatgatcccccatgttgtgcaaaaaagcggttagctccttcggtcctccgatcgttgtcagaagtaagttggccgcagtgttatcactcatggttatggcagcactgcataattctcttactgtcatgccatccgtaagatgcttttctgtgactggtgagtactcaaccaagtcattctgagaatagtgtatgcggcgaccgagttgctcttgcccggcgtcaatacgggataataccgcgccacatagcagaactttaaaagtgctcatcattggaaaacgttcttcggggcgaaaactctcaaggatcttaccgctgttgagatccagttcgatgtaacccactcgtgcacccaactgatcttcagcatcttttactttcaccagcgtttctgggtgagcaaaaacaggaaggcaaaatgccgcaaaaaagggaataagggcgacacggaaatgttgaatactcatactcttcctttttcaatattattgaagcatttatcagggttattgtctcatgagcggatacatatttgaatgtatttagaaaaataaacaaataggggttccgcgcatatttccccgaaaagtgccacctgacgtcgacggatcgggagatctcccgatcccctatggtgcactctcagtacaatctgctctgatgccgcatagttaagccagtatctgctccctgcttgtgtgttggaggtcgctgagtagtgcgcgagcaaaatttaagctacaacaaggcaaggcttgaccgagcaaacaaactctttctgtgttgtaaaacgacggccagtcttaagctcgggccccctgggcggttctgataacgagtaatcgttaatccgcaaataacgtaaaaacccgcttcggcgggtttttttatggggggagtttagggaaagagcatttgtcagaatatttaagggcgcctgtcactttgcttgatatatgagaattatttaaccttataaatgagaaaaaagcaacgcactttaaataagatacgttgctttttcgattgatgaacacctataattaaactattcatctattatttatgattttttgtatatacaatatttctagtttgttaaagagaattaagaaaataaatctcgaaaataataaagggaaaatcagtttttgatatcaaaattatacatgtcaacgataatacaaaatataatacaaactataagatgttatcagtatttattatgcatttagaataaattttgtgtcgcccttattcgactcactatagaagttcctattctctagaaagtagaggaacttcacttcattttgctagcgtgtgagggcctatttcccatgattccttcatatttgcatatacgatacaaggctgttagagagataattggaattaatttgactgtaaacacaaagatattagtacaaaatacgtgacgtagaaagtaataatttcttgggtagtttgcagttttaaaattatgttttaaaatggactatcatatgcttaccgtaacttgaaagtatttcgatttcttggctttatatatcttgtggaaaggacgaaacaccgttagctataggctaataagatagttgtgtcaagtgcttcggagacctaacacgtctccagtcacaacggctaaaaatagcca

SEQ ID NO: 142 - DNA, 3364 bp, synthetic construct
  misc_feature 1..3364: note = plasmid including the sequence for B-Gen.1 human albumin target 20
  source 1..3364: mol_type = other DNA
gcactgtgaagtttcagtcactctaagttttttgttttcaacaccggtaccgcgttacaatgataagtcgactgaataagtgaactcgagatcagcctcgactgtgccttctagttgccagccatctgttgtttgcccctcccccgtgccttccttgaccctggaaggtgccactcccactgtcctttcctaataaaatgaggaaattgcatccccacttcagaagttcctatactttctagtgaatgagtgagctaactcacattaattgcgttgcgctcactgcccgctttccagtcgggaaacctgtcgtgccagctgcattaatgaatcggccaacgcgcggggagaggcggtttgcgtattgggcgctcttgcgcttcctcgctcactgactcgctgcgctcggtcgttcggctgcggcgagcggtatcagctcactcaaaggcggtaatacggttatccacagaatcaggggataacgcaggaaagaacatgtgagcaaaaggccagcaaaaggccaggaaccgtaaaaaggccgcgttgctggcgtttttccataggctccgcccccctgacgagcatcacaaaaatcgacgctcaagtcagaggtggcgaaacccgacaggactataaagataccaggcgtttccccctggaagctccctcgtgcgctctcctgttccgaccctgccgcttaccggatacctgtccgcctttctcccttcgggaagcgtggcgctttctcatagctcacgctgtaggtatctcagttcggtgtaggtcgttcgctccaagctgggctgtgtgcacgaaccccccgttcagcccgaccgctgcgccttatccggtaactatcgtcttgagtccaacccggtaagacacgacttatcgccactggcagcagccactggtaacaggattagcagagcgaggtatgtaggcggtgctacagagttcttgaagtggtggcctaactacggctacactagaagaacagtatttggtatctgcgctctgctgaagccagttaccttcggaaaaagagttggtagctcttgatccggcaaacaaaccaccgctggtagcggtggtttttttgtttgcaagcagcagattacgcgcagaaaaaaaggatctcaagaagatcctttgatcttttctacggggtctgacgctcagtggaacgaaaactcacgttaagggattttggtcatgagattatcaaaaaggatcttcacctagatccttttaaattaaaaatgaagttttaaatcaatctaaagtatatatgagtaaacttggtctgacagttaccaatgcttaatcagtgaggcacctatctcagcgatctgtctatttcgttcatccatagttgcctgactccccgtcgtgtagataactacgatacgggagggcttaccatctggccccagtgctgcaatgataccgcgtgacccacgctcaccggctccagatttatcagcaataaaccagccagccggaagggccgagcgcagaagtggtcctgcaactttatccgcctccatccagtctattaattgttgccgggaagctagagtaagtagttcgccagttaatagtttgcgcaacgttgttgccattgctacaggcatcgtggtgtcacgctcgtcgtttggtatggcttcattcagctccggttcccaacgatcaaggcgagttacatgatcccccatgttgtgcaaaaaagcggttagctccttcggtcctccgatcgttgtcagaagtaagttggccgcagtgttatcactcatggttatggcagcactgcataattctcttactgtcatgccatccgtaagatgcttttctgtgactggtgagtactcaaccaagtcattctgagaatagtgtatgcggcgaccgagttgctcttgcccggcgtcaatacgggataataccgcgccacatagcagaactttaaaagtgctcatcattggaaaacgttcttcggggcgaaaactctcaaggatcttaccgctgttgagatccagttcgatgtaacccactcgtgcacccaactgatcttcagcatcttttactttcaccagcgtttctgggtgagcaaaaacaggaaggcaaaatgccgcaaaaaagggaataagggcgacacggaaatgttgaatactcatactcttcctttttcaatattattgaagcatttatcagggttattgtctcatgagcggatacatatttgaatgtatttagaaaaataaacaaataggggttccgcgcatatttccccgaaaagtgccacctgacgtcgacggatcgggagatctcccgatcccctatggtgcactctcagtacaatctgctctgatgccgcatagttaagccagtatctgctccctgcttgtgtgttggaggtcgctgagtagtgcgcgagcaaaatttaagctacaacaaggcaaggcttgaccgagcaaacaaactctttctgtgttgtaaaacgacggccagtcttaagctcgggccccctgggcggttctgataacgagtaatcgttaatccgcaaataacgtaaaaacccgcttcggcgggtttttttatggggggagtttagggaaagagcatttgtcagaatatttaagggcgcctgtcactttgcttgatatatgagaattatttaaccttataaatgagaaaaaagcaacgcactttaaataagatacgttgctttttcgattgatgaacacctataattaaactattcatctattatttatgattttttgtatatacaatatttctagtttgttaaagagaattaagaaaataaatctcgaaaataataaagggaaaatcagtttttgatatcaaaattatacatgtcaacgataatacaaaatataatacaaactataagatgttatcagtatttattatgcatttagaataaattttgtgtcgcccttattcgactcactatagaagttcctattctctagaaagtagaggaacttcacttcattttgctagcgtgtgagggcctatttcccatgattccttcatatttgcatatacgatacaaggctgttagagagataattggaattaatttgactgtaaacacaaagatattagtacaaaatacgtgacgtagaaagtaataatttcttgggtagtttgcagttttaaaattatgttttaaaatggactatcatatgcttaccgtaacttgaaagtatttcgatttcttggctttatatatcttgtggaaaggacgaaacaccgttagctataggctaataagatagttgtgtcaagtgcttcggagacctaacacgtctccagtcacaacggctaaaaatagcca

SEQ ID NO: 143 - DNA, 3364 bp, synthetic construct
  misc_feature 1..3364: note = plasmid including the sequence for B-Gen.1 human albumin target 21
  source 1..3364: mol_type = other DNA
gcacaattcataactatcccaaagaccttttttgttttcaacaccggtaccgcgttacaatgataagtcgactgaataagtgaactcgagatcagcctcgactgtgccttctagttgccagccatctgttgtttgcccctcccccgtgccttccttgaccctggaaggtgccactcccactgtcctttcctaataaaatgaggaaattgcatccccacttcagaagttcctatactttctagtgaatgagtgagctaactcacattaattgcgttgcgctcactgcccgctttccagtcgggaaacctgtcgtgccagctgcattaatgaatcggccaacgcgcggggagaggcggtttgcgtattgggcgctcttgcgcttcctcgctcactgactcgctgcgctcggtcgttcggctgcggcgagcggtatcagctcactcaaaggcggtaatacggttatccacagaatcaggggataacgcaggaaagaacatgtgagcaaaaggccagcaaaaggccaggaaccgtaaaaaggccgcgttgctggcgtttttccataggctccgcccccctgacgagcatcacaaaaatcgacgctcaagtcagaggtggcgaaacccgacaggactataaagataccaggcgtttccccctggaagctccctcgtgcgctctcctgttccgaccctgccgcttaccggatacctgtccgcctttctcccttcgggaagcgtggcgctttctcatagctcacgctgtaggtatctcagttcggtgtaggtcgttcgctccaagctgggctgtgtgcacgaaccccccgttcagcccgaccgctgcgccttatccggtaactatcgtcttgagtccaacccggtaagacacgacttatcgccactggcagcagccactggtaacaggattagcagagcgaggtatgtaggcggtgctacagagttcttgaagtggtggcctaactacggctacactagaagaacagtatttggtatctgcgctctgctgaagccagttaccttcggaaaaagagttggtagctcttgatccggcaaacaaaccaccgctggtagcggtggtttttttgtttgcaagcagcagattacgcgcagaaaaaaaggatctcaagaagatcctttgatcttttctacggggtctgacgctcagtggaacgaaaactcacgttaagggattttggtcatgagattatcaaaaaggatcttcacctagatccttttaaattaaaaatgaagttttaaatcaatctaaagtatatatgagtaaacttggtctgacagttaccaatgcttaatcagtgaggcacctatctcagcgatctgtctatttcgttcatccatagttgcctgactccccgtcgtgtagataactacgatacgggagggcttaccatctggccccagtgctgcaatgataccgcgtgacccacgctcaccggctccagatttatcagcaataaaccagccagccggaagggccgagcgcagaagtggtcctgcaactttatccgcctccatccagtctattaattgttgccgggaagctagagtaagtagttcgccagttaatagtttgcgcaacgttgttgccattgctacaggcatcgtggtgtcacgctcgtcgtttggtatggcttcattcagctccggttcccaacgatcaaggcgagttacatgatcccccatgttgtgcaaaaaagcggttagctccttcggtcctccgatcgttgtcagaagtaagttggccgcagtgttatcactcatggttatggcagcactgcataattctcttactgtcatgccatccgtaagatgcttttctgtgactggtgagtactcaaccaagtcattctgagaatagtgtatgcggcgaccgagttgctcttgcccggcgtcaatacgggataataccgcgccacatagcagaactttaaaagtgctcatcattggaaaacgttcttcggggcgaaaactctcaaggatcttaccgctgttgagatccagttcgatgtaacccactcgtgcacccaactgatcttcagcatcttttactttcaccagcgtttctgggtgagcaaaaacaggaaggcaaaatgccgcaaaaaagggaataagggcgacacggaaatgttgaatactcatactcttcctttttcaatattattgaagcatttatcagggttattgtctcatgagcggatacatatttgaatgtatttagaaaaataaacaaataggggttccgcgcatatttccccgaaaagtgccacctgacgtcgacggatcgggagatctcccgatcccctatggtgcactctcagtacaatctgctctgatgccgcatagttaagccagtatctgctccctgcttgtgtgttggaggtcgctgagtagtgcgcgagcaaaatttaagctacaacaaggcaaggcttgaccgagcaaacaaactctttctgtgttgtaaaacgacggccagtcttaagctcgggccccctgggcggttctgataacgagtaatcgttaatccgcaaataacgtaaaaacccgcttcggcgggtttttttatggggggagtttagggaaagagcatttgtcagaatatttaagggcgcctgtcactttgcttgatatatgagaattatttaaccttataaatgagaaaaaagcaacgcactttaaataagatacgttgctttttcgattgatgaacacctataattaaactattcatctattatttatgattttttgtatatacaatatttctagtttgttaaagagaattaagaaaataaatctcgaaaataataaagggaaaatcagtttttgatatcaaaattatacatgtcaacgataatacaaaatataatacaaactataagatgttatcagtatttattatgcatttagaataaattttgtgtcgcccttattcgactcactatagaagttcctattctctagaaagtagaggaacttcacttcattttgctagcgtgtgagggcctatttcccatgattccttcatatttgcatatacgatacaaggctgttagagagataattggaattaatttgactgtaaacacaaagatattagtacaaaatacgtgacgtagaaagtaataatttcttgggtagtttgcagttttaaaattatgttttaaaatggactatcatatgcttaccgtaacttgaaagtatttcgatttcttggctttatatatcttgtggaaaggacgaaacaccgttagctataggctaataagatagttgtgtcaagtgcttcggagacctaacacgtctccagtcacaacggctaaaaatagcca

SEQ ID NO: 144 - DNA, 3364 bp, synthetic construct
  misc_feature 1..3364: note = plasmid including the sequence for B-Gen.1 human albumin target 22
  source 1..3364: mol_type = other DNA
gcacaatcttcaaccctattctgtgaattttttgttttcaacaccggtaccgcgttacaatgataagtcgactgaataagtgaactcgagatcagcctcgactgtgccttctagttgccagccatctgttgtttgcccctcccccgtgccttccttgaccctggaaggtgccactcccactgtcctttcctaataaaatgaggaaattgcatccccacttcagaagttcctatactttctagtgaatgagtgagctaactcacattaattgcgttgcgctcactgcccgctttccagtcgggaaacctgtcgtgccagctgcattaatgaatcggccaacgcgcggggagaggcggtttgcgtattgggcgctcttgcgcttcctcgctcactgactcgctgcgctcggtcgttcggctgcggcgagcggtatcagctcactcaaaggcggtaatacggttatccacagaatcaggggataacgcaggaaagaacatgtgagcaaaaggccagcaaaaggccaggaaccgtaaaaaggccgcgttgctggcgtttttccataggctccgcccccctgacgagcatcacaaaaatcgacgctcaagtcagaggtggcgaaacccgacaggactataaagataccaggcgtttccccctggaagctccctcgtgcgctctcctgttccgaccctgccgcttaccggatacctgtccgcctttctcccttcgggaagcgtggcgctttctcatagctcacgctgtaggtatctcagttcggtgtaggtcgttcgctccaagctgggctgtgtgcacgaaccccccgttcagcccgaccgctgcgccttatccggtaactatcgtcttgagtccaacccggtaagacacgacttatcgccactggcagcagccactggtaacaggattagcagagcgaggtatgtaggcggtgctacagagttcttgaagtggtggcctaactacggctacactagaagaacagtatttggtatctgcgctctgctgaagccagttaccttcggaaaaagagttggtagctcttgatccggcaaacaaaccaccgctggtagcggtggtttttttgtttgcaagcagcagattacgcgcagaaaaaaaggatctcaagaagatcctttgatcttttctacggggtctgacgctcagtggaacgaaaactcacgttaagggattttggtcatgagattatcaaaaaggatcttcacctagatccttttaaattaaaaatgaagttttaaatcaatctaaagtatatatgagtaaacttggtctgacagttaccaatgcttaatcagtgaggcacctatctcagcgatctgtctatttcgttcatccatagttgcctgactccccgtcgtgtagataactacgatacgggagggcttaccatctggccccagtgctgcaatgataccgcgtgacccacgctcaccggctccagatttatcagcaataaaccagccagccggaagggccgagcgcagaagtggtcctgcaactttatccgcctccatccagtctattaattgttgccgggaagctagagtaagtagttcgccagttaatagtttgcgcaacgttgttgccattgctacaggcatcgtggtgtcacgctcgtcgtttggtatggcttcattcagctccggttcccaacgatcaaggcgagttacatgatcccccatgttgtgcaaaaaagcggttagctccttcggtcctccgatcgttgtcagaagtaagttggccgcagtgttatcactcatggttatggcagcactgcataattctcttactgtcatgccatccgtaagatgcttttctgtgactggtgagtactcaaccaagtcattctgagaatagtgtatgcggcgaccgagttgctcttgcccggcgtcaatacgggataataccgcgccacatagcagaactttaaaagtgctcatcattggaaaacgttcttcggggcgaaaactctcaaggatcttaccgctgttgagatccagttcgatgtaacccactcgtgcacccaactgatcttcagcatcttttactttcaccagcgtttctgggtgagcaaaaacaggaaggcaaaatgccgcaaaaaagggaataagggcgacacggaaatgttgaatactcatactcttcctttttcaatattattgaagcatttatcagggttattgtctcatgagcggatacatatttgaatgtatttagaaaaataaacaaataggggttccgcgcatatttccccgaaaagtgccacctgacgtcgacggatcgggagatctcccgatcccctatggtgcactctcagtacaatctgctctgatgccgcatagttaagccagtatctgctccctgcttgtgtgttggaggtcgctgagtagtgcgcgagcaaaatttaagctacaacaaggcaaggcttgaccgagcaaacaaactctttctgtgttgtaaaacgacggccagtcttaagctcgggccccctgggcggttctgataacgagtaatcgttaatccgcaaataacgtaaaaacccgcttcggcgggtttttttatggggggagtttagggaaagagcatttgtcagaatatttaagggcgcctgtcactttgcttgatatatgagaattatttaaccttataaatgagaaaaaagcaacgcactttaaataagatacgttgctttttcgattgatgaacacctataattaaactattcatctattatttatgattttttgtatatacaatatttctagtttgttaaagagaattaagaaaataaatctcgaaaataataaagggaaaatcagtttttgatatcaaaattatacatgtcaacgataatacaaaatataatacaaactataagatgttatcagtatttattatgcatttagaataaattttgtgtcgcccttattcgactcactatagaagttcctattctctagaaagtagaggaacttcacttcattttgctagcgtgtgagggcctatttcccatgattccttcatatttgcatatacgatacaaggctgttagagagataattggaattaatttgactgtaaacacaaagatattagtacaaaatacgtgacgtagaaagtaataatttcttgggtagtttgcagttttaaaattatgttttaaaatggactatcatatgcttaccgtaacttgaaagtatttcgatttcttggctttatatatcttgtggaaaggacgaaacaccgttagctataggctaataagatagttgtgtcaagtgcttcggagacctaacacgtctccagtcacaacggctaaaaatagcca

SEQ ID NO: 145 - DNA, 3364 bp, synthetic construct
  misc_feature 1..3364: note = plasmid including the sequence for B-Gen.1 human albumin target 23
  source 1..3364: mol_type = other DNA
gcacataactatcccaaagacctatccttttttgttttcaacaccggtaccgcgttacaatgataagtcgactgaataagtgaactcgagatcagcctcgactgtgccttctagttgccagccatctgttgtttgcccctcccccgtgccttccttgaccctggaaggtgccactcccactgtcctttcctaataaaatgaggaaattgcatccccacttcagaagttcctatactttctagtgaatgagtgagctaactcacattaattgcgttgcgctcactgcccgctttccagtcgggaaacctgtcgtgccagctgcattaatgaatcggccaacgcgcggggagaggcggtttgcgtattgggcgctcttgcgcttcctcgctcactgactcgctgcgctcggtcgttcggctgcggcgagcggtatcagctcactcaaaggcggtaatacggttatccacagaatcaggggataacgcaggaaagaacatgtgagcaaaaggccagcaaaaggccaggaaccgtaaaaaggccgcgttgctggcgtttttccataggctccgcccccctgacgagcatcacaaaaatcgacgctcaagtcagaggtggcgaaacccgacaggactataaagataccaggcgtttccccctggaagctccctcgtgcgctctcctgttccgaccctgccgcttaccggatacctgtccgcctttctcccttcgggaagcgtggcgctttctcatagctcacgctgtaggtatctcagttcggtgtaggtcgttcgctccaagctgggctgtgtgcacgaaccccccgttcagcccgaccgctgcgccttatccggtaactatcgtcttgagtccaacccggtaagacacgacttatcgccactggcagcagccactggtaacaggattagcagagcgaggtatgtaggcggtgctacagagttcttgaagtggtggcctaactacggctacactagaagaacagtatttggtatctgcgctctgctgaagccagttaccttcggaaaaagagttggtagctcttgatccggcaaacaaaccaccgctggtagcggtggtttttttgtttgcaagcagcagattacgcgcagaaaaaaaggatctcaagaagatcctttgatcttttctacggggtctgacgctcagtggaacgaaaactcacgttaagggattttggtcatgagattatcaaaaaggatcttcacctagatccttttaaattaaaaatgaagttttaaatcaatctaaagtatatatgagtaaacttggtctgacagttaccaatgcttaatcagtgaggcacctatctcagcgatctgtctatttcgttcatccatagttgcctgactccccgtcgtgtagataactacgatacgggagggcttaccatctggccccagtgctgcaatgataccgcgtgacccacgctcaccggctccagatttatcagcaataaaccagccagccggaagggccgagcgcagaagtggtcctgcaactttatccgcctccatccagtctattaattgttgccgggaagctagagtaagtagttcgccagttaatagtttgcgcaacgttgttgccattgctacaggcatcgtggtgtcacgctcgtcgtttggtatggcttcattcagctccggttcccaacgatcaaggcgagttacatgatcccccatgttgtgcaaaaaagcggttagctccttcggtcctccgatcgttgtcagaagtaagttggccgcagtgttatcactcatggttatggcagcactgcataattctcttactgtcatgccatccgtaagatgcttttctgtgactggtgagtactcaaccaagtcattctgagaatagtgtatgcggcgaccgagttgctcttgcccggcgtcaatacgggataataccgcgccacatagcagaactttaaaagtgctcatcattggaaaacgttcttcggggcgaaaactctcaaggatcttaccgctgttgagatccagttcgatgtaacccactcgtgcacccaactgatcttcagcatcttttactttcaccagcgtttctgggtgagcaaaaacaggaaggcaaaatgccgcaaaaaagggaataagggcgacacggaaatgttgaatactcatactcttcctttttcaatattattgaagcatttatcagggttattgtctcatgagcggatacatatttgaatgtatttagaaaaataaacaaataggggttccgcgcatatttccccgaaaagtgccacctgacgtcgacggatcgggagatctcccgatcccctatggtgcactctcagtacaatctgctctgatgccgcatagttaagccagtatctgctccctgcttgtgtgttggaggtcgctgagtagtgcgcgagcaaaatttaagctacaacaaggcaaggcttgaccgagcaaacaaactctttctgtgttgtaaaacgacggccagtcttaagctcgggccccctgggcggttctgataacgagtaatcgttaatccgcaaataacgtaaaaacccgcttcggcgggtttttttatggggggagtttagggaaagagcatttgtcagaatatttaagggcgcctgtcactttgcttgatatatgagaattatttaaccttataaatgagaaaaaagcaacgcactttaaataagatacgttgctttttcgattgatgaacacctataattaaactattcatctattatttatgattttttgtatatacaatatttctagtttgttaaagagaattaagaaaataaatctcgaaaataataaagggaaaatcagtttttgatatcaaaattatacatgtcaacgataatacaaaatataatacaaactataagatgttatcagtatttattatgcatttagaataaattttgtgtcgcccttattcgactcactatagaagttcctattctctagaaagtagaggaacttcacttcattttgctagcgtgtgagggcctatttcccatgattccttcatatttgcatatacgatacaaggctgttagagagataattggaattaatttgactgtaaacacaaagatattagtacaaaatacgtgacgtagaaagtaataatttcttgggtagtttgcagttttaaaattatgttttaaaatggactatcatatgcttaccgtaacttgaaagtatttcgatttcttggctttatatatcttgtggaaaggacgaaacaccgttagctataggctaataagatagttgtgtcaagtgcttcggagacctaacacgtctccagtcacaacggctaaaaatagcca

SEQ ID NO: 146 - DNA, 3364 bp, synthetic construct
  misc_feature 1..3364: note = plasmid including the sequence for B-Gen.1 human albumin target 24
  source 1..3364: mol_type = other DNA
gcaccactatgctttatttaaaaaccattttttgttttcaacaccggtaccgcgttacaatgataagtcgactgaataagtgaactcgagatcagcctcgactgtgccttctagttgccagccatctgttgtttgcccctcccccgtgccttccttgaccctggaaggtgccactcccactgtcctttcctaataaaatgaggaaattgcatccccacttcagaagttcctatactttctagtgaatgagtgagctaactcacattaattgcgttgcgctcactgcccgctttccagtcgggaaacctgtcgtgccagctgcattaatgaatcggccaacgcgcggggagaggcggtttgcgtattgggcgctcttgcgcttcctcgctcactgactcgctgcgctcggtcgttcggctgcggcgagcggtatcagctcactcaaaggcggtaatacggttatccacagaatcaggggataacgcaggaaagaacatgtgagcaaaaggccagcaaaaggccaggaaccgtaaaaaggccgcgttgctggcgtttttccataggctccgcccccctgacgagcatcacaaaaatcgacgctcaagtcagaggtggcgaaacccgacaggactataaagataccaggcgtttccccctggaagctccctcgtgcgctctcctgttccgaccctgccgcttaccggatacctgtccgcctttctcccttcgggaagcgtggcgctttctcatagctcacgctgtaggtatctcagttcggtgtaggtcgttcgctccaagctgggctgtgtgcacgaaccccccgttcagcccgaccgctgcgccttatccggtaactatcgtcttgagtccaacccggtaagacacgacttatcgccactggcagcagccactggtaacaggattagcagagcgaggtatgtaggcggtgctacagagttcttgaagtggtggcctaactacggctacactagaagaacagtatttggtatctgcgctctgctgaagccagttaccttcggaaaaagagttggtagctcttgatccggcaaacaaaccaccgctggtagcggtggtttttttgtttgcaagcagcagattacgcgcagaaaaaaaggatctcaagaagatcctttgatcttttctacggggtctgacgctcagtggaacgaaaactcacgttaagggattttggtcatgagattatcaaaaaggatcttcacctagatccttttaaattaaaaatgaagttttaaatcaatctaaagtatatatgagtaaacttggtctgacagttaccaatgcttaatcagtgaggcacctatctcagcgatctgtctatttcgttcatccatagttgcctgactccccgtcgtgtagataactacgatacgggagggcttaccatctggccccagtgctgcaatgataccgcgtgacccacgctcaccggctccagatttatcagcaataaaccagccagccggaagggccgagcgcagaagtggtcctgcaactttatccgcctccatccagtctattaattgttgccgggaagctagagtaagtagttcgccagttaatagtttgcgcaacgttgttgccattgctacaggcatcgtggtgtcacgctcgtcgtttggtatggcttcattcagctccggttcccaacgatcaaggcgagttacatgatcccccatgttgtgcaaaaaagcggttagctccttcggtcctccgatcgttgtcagaagtaagttggccgcagtgttatcactcatggttatggcagcactgcataattctcttactgtcatgccatccgtaagatgcttttctgtgactggtgagtactcaaccaagtcattctgagaatagtgtatgcggcgaccgagttgctcttgcccggcgtcaatacgggataataccgcgccacatagcagaactttaaaagtgctcatcattggaaaacgttcttcggggcgaaaactctcaaggatcttaccgctgttgagatccagttcgatgtaacccactcgtgcacccaactgatcttcagcatcttttactttcaccagcgtttctgggtgagcaaaaacaggaaggcaaaatgccgcaaaaaagggaataagggcgacacggaaatgttgaatactcatactcttcctttttcaatattattgaagcatttatcagggttattgtctcatgagcggatacatatttgaatgtatttagaaaaataaacaaataggggttccgcgcatatttccccgaaaagtgccacctgacgtcgacggatcgggagatctcccgatcccctatggtgcactctcagtacaatctgctctgatgccgcatagttaagccagtatctgctccctgcttgtgtgttggaggtcgctgagtagtgcgcgagcaaaatttaagctacaacaaggcaaggcttgaccgagcaaacaaactctttctgtgttgtaaaacgacggccagtcttaagctcgggccccctgggcggttctgataacgagtaatcgttaatccgcaaataacgtaaaaacccgcttcggcgggtttttttatggggggagtttagggaaagagcatttgtcagaatatttaagggcgcctgtcactttgcttgatatatgagaattatttaaccttataaatgagaaaaaagcaacgcactttaaataagatacgttgctttttcgattgatgaacacctataattaaactattcatctattatttatgattttttgtatatacaatatttctagtttgttaaagagaattaagaaaataaatctcgaaaataataaagggaaaatcagtttttgatatcaaaattatacatgtcaacgataatacaaaatataatacaaactataagatgttatcagtatttattatgcatttagaataaattttgtgtcgcccttattcgactcactatagaagttcctattctctagaaagtagaggaacttcacttcattttgctagcgtgtgagggcctatttcccatgattccttcatatttgcatatacgatacaaggctgttagagagataattggaattaatttgactgtaaacacaaagatattagtacaaaatacgtgacgtagaaagtaataatttcttgggtagtttgcagttttaaaattatgttttaaaatggactatcatatgcttaccgtaacttgaaagtatttcgatttcttggctttatatatcttgtggaaaggacgaaacaccgttagctataggctaataagatagttgtgtcaagtgcttcggagacctaacacgtctccagtcacaacggctaaaaatagcca

SEQ ID NO: 147 - DNA, 3364 bp, synthetic construct
  misc_feature 1..3364: note = plasmid including the sequence for B-Gen.1 human albumin target 25
  source 1..3364: mol_type = other DNA
gcacaaaaaccacaaaacctgtgctgtttttttgttttcaacaccggtaccgcgttacaatgataagtcgactgaataagtgaactcgagatcagcctcgactgtgccttctagttgccagccatctgttgtttgcccctcccccgtgccttccttgaccctggaaggtgccactcccactgtcctttcctaataaaatgaggaaattgcatccccacttcagaagttcctatactttctagtgaatgagtgagctaactcacattaattgcgttgcgctcactgcccgctttccagtcgggaaacctgtcgtgccagctgcattaatgaatcggccaacgcgcggggagaggcggtttgcgtattgggcgctcttgcgcttcctcgctcactgactcgctgcgctcggtcgttcggctgcggcgagcggtatcagctcactcaaaggcggtaatacggttatccacagaatcaggggataacgcaggaaagaacatgtgagcaaaaggccagcaaaaggccaggaaccgtaaaaaggccgcgttgctggcgtttttccataggctccgcccccctgacgagcatcacaaaaatcgacgctcaagtcagaggtggcgaaacccgacaggactataaagataccaggcgtttccccctggaagctccctcgtgcgctctcctgttccgaccctgccgcttaccggatacctgtccgcctttctcccttcgggaagcgtggcgctttctcatagctcacgctgtaggtatctcagttcggtgtaggtcgttcgctccaagctgggctgtgtgcacgaaccccccgttcagcccgaccgctgcgccttatccggtaactatcgtcttgagtccaacccggtaagacacgacttatcgccactggcagcagccactggtaacaggattagcagagcgaggtatgtaggcggtgctacagagttcttgaagtggtggcctaactacggctacactagaagaacagtatttggtatctgcgctctgctgaagccagttaccttcggaaaaagagttggtagctcttgatccggcaaacaaaccaccgctggtagcggtggtttttttgtttgcaagcagcagattacgcgcagaaaaaaaggatctcaagaagatcctttgatcttttctacggggtctgacgctcagtggaacgaaaactcacgttaagggattttggtcatgagattatcaaaaaggatcttcacctagatccttttaaattaaaaatgaagttttaaatcaatctaaagtatatatgagtaaacttggtctgacagttaccaatgcttaatcagtgaggcacctatctcagcgatctgtctatttcgttcatccatagttgcctgactccccgtcgtgtagataactacgatacgggagggcttaccatctggccccagtgctgcaatgataccgcgtgacccacgctcaccggctccagatttatcagcaataaaccagccagccggaagggccgagcgcagaagtggtcctgcaactttatccgcctccatccagtctattaattgttgccgggaagctagagtaagtagttcgccagttaatagtttgcgcaacgttgttgccattgctacaggcatcgtggtgtcacgctcgtcgtttggtatggcttcattcagctccggttcccaacgatcaaggcgagttacatgatcccccatgttgtgcaaaaaagcggttagctccttcggtcctccgatcgttgtcagaagtaagttggccgcagtgttatcactcatggttatggcagcactgcataattctcttactgtcatgccatccgtaagatgcttttctgtgactggtgagtactcaaccaagtcattctgagaatagtgtatgcggcgaccgagttgctcttgcccggcgtcaatacgggataataccgcgccacatagcagaactttaaaagtgctcatcattggaaaacgttcttcggggcgaaaactctcaaggatcttaccgctgttgagatccagttcgatgtaacccactcgtgcacccaactgatcttcagcatcttttactttcaccagcgtttctgggtgagcaaaaacaggaaggcaaaatgccgcaaaaaagggaataagggcgacacggaaatgttgaatactcatactcttcctttttcaatattattgaagcatttatcagggttattgtctcatgagcggatacatatttgaatgtatttagaaaaataaacaaataggggttccgcgcatatttccccgaaaagtgccacctgacgtcgacggatcgggagatctcccgatcccctatggtgcactctcagtacaatctgctctgatgccgcatagttaagccagtatctgctccctgcttgtgtgttggaggtcgctgagtagtgcgcgagcaaaatttaagctacaacaaggcaaggcttgaccgagcaaacaaactctttctgtgttgtaaaacgacggccagtcttaagctcgggccccctgggcggttctgataacgagtaatcgttaatccgcaaataacgtaaaaacccgcttcggcgggtttttttatggggggagtttagggaaagagcatttgtcagaatatttaagggcgcctgtcactttgcttgatatatgagaattatttaaccttataaatgagaaaaaagcaacgcactttaaataagatacgttgctttttcgattgatgaacacctataattaaactattcatctattatttatgattttttgtatatacaatatttctagtttgttaaagagaattaagaaaataaatctcgaaaataataaagggaaaatcagtttttgatatcaaaattatacatgtcaacgataatacaaaatataatacaaactataagatgttatcagtatttattatgcatttagaataaattttgtgtcgcccttattcgactcactatagaagttcctattctctagaaagtagaggaacttcacttcattttgctagcgtgtgagggcctatttcccatgattccttcatatttgcatatacgatacaaggctgttagagagataattggaattaatttgactgtaaacacaaagatattagtacaaaatacgtgacgtagaaagtaataatttcttgggtagtttgcagttttaaaattatgttttaaaatggactatcatatgcttaccgtaacttgaaagtatttcgatttcttggctttatatatcttgtggaaaggacgaaacaccgttagctataggctaataagatagttgtgtcaagtgcttcggagacctaacacgtctccagtcacaacggctaaaaatagcca

SEQ ID NO: 148 - DNA, 3364 bp, synthetic construct
  misc_feature 1..3364: note = plasmid including the sequence for B-Gen.1 human albumin target 26
  source 1..3364: mol_type = other DNA
gcacatgagatcaacagcacaggttttttttttgttttcaacaccggtaccgcgttacaatgataagtcgactgaataagtgaactcgagatcagcctcgactgtgccttctagttgccagccatctgttgtttgcccctcccccgtgccttccttgaccctggaaggtgccactcccactgtcctttcctaataaaatgaggaaattgcatccccacttcagaagttcctatactttctagtgaatgagtgagctaactcacattaattgcgttgcgctcactgcccgctttccagtcgggaaacctgtcgtgccagctgcattaatgaatcggccaacgcgcggggagaggcggtttgcgtattgggcgctcttgcgcttcctcgctcactgactcgctgcgctcggtcgttcggctgcggcgagcggtatcagctcactcaaaggcggtaatacggttatccacagaatcaggggataacgcaggaaagaacatgtgagcaaaaggccagcaaaaggccaggaaccgtaaaaaggccgcgttgctggcgtttttccataggctccgcccccctgacgagcatcacaaaaatcgacgctcaagtcagaggtggcgaaacccgacaggactataaagataccaggcgtttccccctggaagctccctcgtgcgctctcctgttccgaccctgccgcttaccggatacctgtccgcctttctcccttcgggaagcgtggcgctttctcatagctcacgctgtaggtatctcagttcggtgtaggtcgttcgctccaagctgggctgtgtgcacgaaccccccgttcagcccgaccgctgcgccttatccggtaactatcgtcttgagtccaacccggtaagacacgacttatcgccactggcagcagccactggtaacaggattagcagagcgaggtatgtaggcggtgctacagagttcttgaagtggtggcctaactacggctacactagaagaacagtatttggtatctgcgctctgctgaagccagttaccttcggaaaaagagttggtagctcttgatccggcaaacaaaccaccgctggtagcggtggtttttttgtttgcaagcagcagattacgcgcagaaaaaaaggatctcaagaagatcctttgatcttttctacggggtctgacgctcagtggaacgaaaactcacgttaagggattttggtcatgagattatcaaaaaggatcttcacctagatccttttaaattaaaaatgaagttttaaatcaatctaaagtatatatgagtaaacttggtctgacagttaccaatgcttaatcagtgaggcacctatctcagcgatctgtctatttcgttcatccatagttgcctgactccccgtcgtgtagataactacgatacgggagggcttaccatctggccccagtgctgcaatgataccgcgtgacccacgctcaccggctccagatttatcagcaataaaccagccagccggaagggccgagcgcagaagtggtcctgcaactttatccgcctccatccagtctattaattgttgccgggaagctagagtaagtagttcgccagttaatagtttgcgcaacgttgttgccattgctacaggcatcgtggtgtcacgctcgtcgtttggtatggcttcattcagctccggttcccaacgatcaaggcgagttacatgatcccccatgttgtgcaaaaaagcggttagctccttcggtcctccgatcgttgtcagaagtaagttggccgcagtgttatcactcatggttatggcagcactgcataattctcttactgtcatgccatccgtaagatgcttttctgtgactggtgagtactcaaccaagtcattctgagaatagtgtatgcggcgaccgagttgctcttgcccggcgtcaatacgggataataccgcgccacatagcagaactttaaaagtgctcatcattggaaaacgttcttcggggcgaaaactctcaaggatcttaccgctgttgagatccagttcgatgtaacccactcgtgcacccaactgatcttcagcatcttttactttcaccagcgtttctgggtgagcaaaaacaggaaggcaaaatgccgcaaaaaagggaataagggcgacacggaaatgttgaatactcatactcttcctttttcaatattattgaagcatttatcagggttattgtctcatgagcggatacatatttgaatgtatttagaaaaataaacaaataggggttccgcgcatatttccccgaaaagtgccacctgacgtcgacggatcgggagatctcccgatcccctatggtgcactctcagtacaatctgctctgatgccgcatagttaagccagtatctgctccctgcttgtgtgttggaggtcgctgagtagtgcgcgagcaaaatttaagctacaacaaggcaaggcttgaccgagcaaacaaactctttctgtgttgtaaaacgacggccagtcttaagctcgggccccctgggcggttctgataacgagtaatcgttaatccgcaaataacgtaaaaacccgcttcggcgggtttttttatggggggagtttagggaaagagcatttgtcagaatatttaagggcgcctgtcactttgcttgatatatgagaattatttaaccttataaatgagaaaaaagcaacgcactttaaataagatacgttgctttttcgattgatgaacacctataattaaactattcatctattatttatgattttttgtatatacaatatttctagtttgttaaagagaattaagaaaataaatctcgaaaataataaagggaaaatcagtttttgatatcaaaattatacatgtcaacgataatacaaaatataatacaaactataagatgttatcagtatttattatgcatttagaataaattttgtgtcgcccttattcgactcactatagaagttcctattctctagaaagtagaggaacttcacttcattttgctagcgtgtgagggcctatttcccatgattccttcatatttgcatatacgatacaaggctgttagagagataattggaattaatttgactgtaaacacaaagatattagtacaaaatacgtgacgtagaaagtaataatttcttgggtagtttgcagttttaaaattatgttttaaaatggactatcatatgcttaccgtaacttgaaagtatttcgatttcttggctttatatatcttgtggaaaggacgaaacaccgttagctataggctaataagatagttgtgtcaagtgcttcggagacctaacacgtctccagtcacaacggctaaaaatagcca

SEQ ID NO: 149 - DNA, 3364 bp, synthetic construct
  misc_feature 1..3364: note = plasmid including the sequence for B-Gen.1 human albumin target 27
  source 1..3364: mol_type = other DNA
gcacatatttattttcattttagtctgttttttgttttcaacaccggtaccgcgttacaatgataagtcgactgaataagtgaactcgagatcagcctcgactgtgccttctagttgccagccatctgttgtttgcccctcccccgtgccttccttgaccctggaaggtgccactcccactgtcctttcctaataaaatgaggaaattgcatccccacttcagaagttcctatactttctagtgaatgagtgagctaactcacattaattgcgttgcgctcactgcccgctttccagtcgggaaacctgtcgtgccagctgcattaatgaatcggccaacgcgcggggagaggcggtttgcgtattgggcgctcttgcgcttcctcgctcactgactcgctgcgctcggtcgttcggctgcggcgagcggtatcagctcactcaaaggcggtaatacggttatccacagaatcaggggataacgcaggaaagaacatgtgagcaaaaggccagcaaaaggccaggaaccgtaaaaaggccgcgttgctggcgtttttccataggctccgcccccctgacgagcatcacaaaaatcgacgctcaagtcagaggtggcgaaacccgacaggactataaagataccaggcgtttccccctggaagctccctcgtgcgctctcctgttccgaccctgccgcttaccggatacctgtccgcctttctcccttcgggaagcgtggcgctttctcatagctcacgctgtaggtatctcagttcggtgtaggtcgttcgctccaagctgggctgtgtgcacgaaccccccgttcagcccgaccgctgcgccttatccggtaactatcgtcttgagtccaacccggtaagacacgacttatcgccactggcagcagccactggtaacaggattagcagagcgaggtatgtaggcggtgctacagagttcttgaagtggtggcctaactacggctacactagaagaacagtatttggtatctgcgctctgctgaagccagttaccttcggaaaaagagttggtagctcttgatccggcaaacaaaccaccgctggtagcggtggtttttttgtttgcaagcagcagattacgcgcagaaaaaaaggatctcaagaagatcctttgatcttttctacggggtctgacgctcagtggaacgaaaactcacgttaagggattttggtcatgagattatcaaaaaggatcttcacctagatccttttaaattaaaaatgaagttttaaatcaatctaaagtatatatgagtaaacttggtctgacagttaccaatgcttaatcagtgaggcacctatctcagcgatctgtctatttcgttcatccatagttgcctgactccccgtcgtgtagataactacgatacgggagggcttaccatctggccccagtgctgcaatgataccgcgtgacccacgctcaccggctccagatttatcagcaataaaccagccagccggaagggccgagcgcagaagtggtcctgcaactttatccgcctccatccagtctattaattgttgccgggaagctagagtaagtagttcgccagttaatagtttgcgcaacgttgttgccattgctacaggcatcgtggtgtcacgctcgtcgtttggtatggcttcattcagctccggttcccaacgatcaaggcgagttacatgatcccccatgttgtgcaaaaaagcggttagctccttcggtcctccgatcgttgtcagaagtaagttggccgcagtgttatcactcatggttatggcagcactgcataattctcttactgtcatgccatccgtaagatgcttttctgtgactggtgagtactcaaccaagtcattctgagaatagtgtatgcggcgaccgagttgctcttgcccggcgtcaatacgggataataccgcgccacatagcagaactttaaaagtgctcatcattggaaaacgttcttcggggcgaaaactctcaaggatcttaccgctgttgagatccagttcgatgtaacccactcgtgcacccaactgatcttcagcatcttttactttcaccagcgtttctgggtgagcaaaaacaggaaggcaaaatgccgcaaaaaagggaataagggcgacacggaaatgttgaatactcatactcttcctttttcaatattattgaagcatttatcagggttattgtctcatgagcggatacatatttgaatgtatttagaaaaataaacaaataggggttccgcgcatatttccccgaaaagtgccacctgacgtcgacggatcgggagatctcccgatcccctatggtgcactctcagtacaatctgctctgatgccgcatagttaagccagtatctgctccctgcttgtgtgttggaggtcgctgagtagtgcgcgagcaaaatttaagctacaacaaggcaaggcttgaccgagcaaacaaactctttctgtgttgtaaaacgacggccagtcttaagctcgggccccctgggcggttctgataacgagtaatcgttaatccgcaaataacgtaaaaacccgcttcggcgggtttttttatggggggagtttagggaaagagcatttgtcagaatatttaagggcgcctgtcactttgcttgatatatgagaattatttaaccttataaatgagaaaaaagcaacgcactttaaataagatacgttgctttttcgattgatgaacacctataattaaactattcatctattatttatgattttttgtatatacaatatttctagtttgttaaagagaattaagaaaataaatctcgaaaataataaagggaaaatcagtttttgatatcaaaattatacatgtcaacgataatacaaaatataatacaaactataagatgttatcagtatttattatgcatttagaataaattttgtgtcgcccttattcgactcactatagaagttcctattctctagaaagtagaggaacttcacttcattttgctagcgtgtgagggcctatttcccatgattccttcatatttgcatatacgatacaaggctgttagagagataattggaattaatttgactgtaaacacaaagatattagtacaaaatacgtgacgtagaaagtaataatttcttgggtagtttgcagttttaaaattatgttttaaaatggactatcatatgcttaccgtaacttgaaagtatttcgatttcttggctttatatatcttgtggaaaggacgaaacaccgttagctataggctaataagatagttgtgtcaagtgcttcggagacctaacacgtctccagtcacaacggctaaaaatagcca

SEQ ID NO: 150 - DNA, 3364 bp, synthetic construct
  misc_feature 1..3364: note = plasmid including the sequence for B-Gen.1 human albumin target 28
  source 1..3364: mol_type = other DNA
gcacattttcattttagtctgtcttctttttttgttttcaacaccggtaccgcgttacaatgataagtcgactgaataagtgaactcgagatcagcctcgactgtgccttctagttgccagccatctgttgtttgcccctcccccgtgccttccttgaccctggaaggtgccactcccactgtcctttcctaataaaatgaggaaattgcatccccacttcagaagttcctatactttctagtgaatgagtgagctaactcacattaattgcgttgcgctcactgcccgctttccagtcgggaaacctgtcgtgccagctgcattaatgaatcggccaacgcgcggggagaggcggtttgcgtattgggcgctcttgcgcttcctcgctcactgactcgctgcgctcggtcgttcggctgcggcgagcggtatcagctcactcaaaggcggtaatacggttatccacagaatcaggggataacgcaggaaagaacatgtgagcaaaaggccagcaaaaggccaggaaccgtaaaaaggccgcgttgctggcgtttttccataggctccgcccccctgacgagcatcacaaaaatcgacgctcaagtcagaggtggcgaaacccgacaggactataaagataccaggcgtttccccctggaagctccctcgtgcgctctcctgttccgaccctgccgcttaccggatacctgtccgcctttctcccttcgggaagcgtggcgctttctcatagctcacgctgtaggtatctcagttcggtgtaggtcgttcgctccaagctgggctgtgtgcacgaaccccccgttcagcccgaccgctgcgccttatccggtaactatcgtcttgagtccaacccggtaagacacgacttatcgccactggcagcagccactggtaacaggattagcagagcgaggtatgtaggcggtgctacagagttcttgaagtggtggcctaactacggctacactagaagaacagtatttggtatctgcgctctgctgaagccagttaccttcggaaaaagagttggtagctcttgatccggcaaacaaaccaccgctggtagcggtggtttttttgtttgcaagcagcagattacgcgcagaaaaaaaggatctcaagaagatcctttgatcttttctacggggtctgacgctcagtggaacgaaaactcacgttaagggattttggtcatgagattatcaaaaaggatcttcacctagatccttttaaattaaaaatgaagttttaaatcaatctaaagtatatatgagtaaacttggtctgacagttaccaatgcttaatcagtgaggcacctatctcagcgatctgtctatttcgttcatccatagttgcctgactccccgtcgtgtagataactacgatacgggagggcttaccatctggccccagtgctgcaatgataccgcgtgacccacgctcaccggctccagatttatcagcaataaaccagccagccggaagggccgagcgcagaagtggtcctgcaactttatccgcctccatccagtctattaattgttgccgggaagctagagtaagtagttcgccagttaatagtttgcgcaacgttgttgccattgctacaggcatcgtggtgtcacgctcgtcgtttggtatggcttcattcagctccggttcccaacgatcaaggcgagttacatgatcccccatgttgtgcaaaaaagcggttagctccttcggtcctccgatcgttgtcagaagtaagttggccgcagtgttatcactcatggttatggcagcactgcataattctcttactgtcatgccatccgtaagatgcttttctgtgactggtgagtactcaaccaagtcattctgagaatagtgtatgcggcgaccgagttgctcttgcccggcgtcaatacgggataataccgcgccacatagcagaactttaaaagtgctcatcattggaaaacgttcttcggggcgaaaactctcaaggatcttaccgctgttgagatccagttcgatgtaacccactcgtgcacccaactgatcttcagcatcttttactttcaccagcgtttctgggtgagcaaaaacaggaaggcaaaatgccgcaaaaaagggaataagggcgacacggaaatgttgaatactcatactcttcctttttcaatattattgaagcatttatcagggttattgtctcatgagcggatacatatttgaatgtatttagaaaaataaacaaataggggttccgcgcatatttccccgaaaagtgccacctgacgtcgacggatcgggagatctcccgatcccctatggtgcactctcagtacaatctgctctgatgccgcatagttaagccagtatctgctccctgcttgtgtgttggaggtcgctgagtagtgcgcgagcaaaatttaagctacaacaaggcaaggcttgaccgagcaaacaaactctttctgtgttgtaaaacgacggccagtcttaagctcgggccccctgggcggttctgataacgagtaatcgttaatccgcaaataacgtaaaaacccgcttcggcgggtttttttatggggggagtttagggaaagagcatttgtcagaatatttaagggcgcctgtcactttgcttgatatatgagaattatttaaccttataaatgagaaaaaagcaacgcactttaaataagatacgttgctttttcgattgatgaacacctataattaaactattcatctattatttatgattttttgtatatacaatatttctagtttgttaaagagaattaagaaaataaatctcgaaaataataaagggaaaatcagtttttgatatcaaaattatacatgtcaacgataatacaaaatataatacaaactataagatgttatcagtatttattatgcatttagaataaattttgtgtcgcccttattcgactcactatagaagttcctattctctagaaagtagaggaacttcacttcattttgctagcgtgtgagggcctatttcccatgattccttcatatttgcatatacgatacaaggctgttagagagataattggaattaatttgactgtaaacacaaagatattagtacaaaatacgtgacgtagaaagtaataatttcttgggtagtttgcagttttaaaattatgttttaaaatggactatcatatgcttaccgtaacttgaaagtatttcgatttcttggctttatatatcttgtggaaaggacgaaacaccgttagctataggctaataagatagttgtgtcaagtgcttcggagacctaacacgtctccagtcacaacggctaaaaatagcca

SEQ ID NO: 151 - DNA, 3364 bp, synthetic construct
  misc_feature 1..3364: note = plasmid including the sequence for B-Gen.1 human albumin target 29
  source 1..3364: mol_type = other DNA
gcactcattttagtctgtcttcttggtttttttgttttcaacaccggtaccgcgttacaatgataagtcgactgaataagtgaactcgagatcagcctcgactgtgccttctagttgccagccatctgttgtttgcccctcccccgtgccttccttgaccctggaaggtgccactcccactgtcctttcctaataaaatgaggaaattgcatccccacttcagaagttcctatactttctagtgaatgagtgagctaactcacattaattgcgttgcgctcactgcccgctttccagtcgggaaacctgtcgtgccagctgcattaatgaatcggccaacgcgcggggagaggcggtttgcgtattgggcgctcttgcgcttcctcgctcactgactcgctgcgctcggtcgttcggctgcggcgagcggtatcagctcactcaaaggcggtaatacggttatccacagaatcaggggataacgcaggaaagaacatgtgagcaaaaggccagcaaaaggccaggaaccgtaaaaaggccgcgttgctggcgtttttccataggctccgcccccctgacgagcatcacaaaaatcgacgctcaagtcagaggtggcgaaacccgacaggactataaagataccaggcgtttccccctggaagctccctcgtgcgctctcctgttccgaccctgccgcttaccggatacctgtccgcctttctcccttcgggaagcgtggcgctttctcatagctcacgctgtaggtatctcagttcggtgtaggtcgttcgctccaagctgggctgtgtgcacgaaccccccgttcagcccgaccgctgcgccttatccggtaactatcgtcttgagtccaacccggtaagacacgacttatcgccactggcagcagccactggtaacaggattagcagagcgaggtatgtaggcggtgctacagagttcttgaagtggtggcctaactacggctacactagaagaacagtatttggtatctgcgctctgctgaagccagttaccttcggaaaaagagttggtagctcttgatccggcaaacaaaccaccgctggtagcggtggtttttttgtttgcaagcagcagattacgcgcagaaaaaaaggatctcaagaagatcctttgatcttttctacggggtctgacgctcagtggaacgaaaactcacgttaagggattttggtcatgagattatcaaaaaggatcttcacctagatccttttaaattaaaaatgaagttttaaatcaatctaaagtatatatgagtaaacttggtctgacagttaccaatgcttaatcagtgaggcacctatctcagcgatctgtctatttcgttcatccatagttgcctgactccccgtcgtgtagataactacgatacgggagggcttaccatctggccccagtgctgcaatgataccgcgtgacccacgctcaccggctccagatttatcagcaataaaccagccagccggaagggccgagcgcagaagtggtcctgcaactttatccgcctccatccagtctattaattgttgccgggaagctagagtaagtagttcgccagttaatagtttgcgcaacgttgttgccattgctacaggcatcgtggtgtcacgctcgtcgtttggtatggcttcattcagctccggttcccaacgatcaaggcgagttacatgatcccccatgttgtgcaaaaaagcggttagctccttcggtcctccgatcgttgtcagaagtaagttggccgcagtgttatcactcatggttatggcagcactgcataattctcttactgtcatgccatccgtaagatgcttttctgtgactggtgagtactcaaccaagtcattctgagaatagtgtatgcggcgaccgagttgctcttgcccggcgtcaatacgggataataccgcgccacatagcagaactttaaaagtgctcatcattggaaaacgttcttcggggcgaaaactctcaaggatcttaccgctgttgagatccagttcgatgtaacccactcgtgcacccaactgatcttcagcatcttttactttcaccagcgtttctgggtgagcaaaaacaggaaggcaaaatgccgcaaaaaagggaataagggcgacacggaaatgttgaatactcatactcttcctttttcaatattattgaagcatttatcagggttattgtctcatgagcggatacatatttgaatgtatttagaaaaataaacaaataggggttccgcgcatatttccccgaaaagtgccacctgacgtcgacggatcgggagatctcccgatcccctatggtgcactctcagtacaatctgctctgatgccgcatagttaagccagtatctgctccctgcttgtgtgttggaggtcgctgagtagtgcgcgagcaaaatttaagctacaacaaggcaaggcttgaccgagcaaacaaactctttctgtgttgtaaaacgacggccagtcttaagctcgggccccctgggcggttctgataacgagtaatcgttaatccgcaaataacgtaaaaacccgcttcggcgggtttttttatggggggagtttagggaaagagcatttgtcagaatatttaagggcgcctgtcactttgcttgatatatgagaattatttaaccttataaatgagaaaaaagcaacgcactttaaataagatacgttgctttttcgattgatgaacacctataattaaactattcatctattatttatgattttttgtatatacaatatttctagtttgttaaagagaattaagaaaataaatctcgaaaataataaagggaaaatcagtttttgatatcaaaattatacatgtcaacgataatacaaaatataatacaaactataagatgttatcagtatttattatgcatttagaataaattttgtgtcgcccttattcgactcactatagaagttcctattctctagaaagtagaggaacttcacttcattttgctagcgtgtgagggcctatttcccatgattccttcatatttgcatatacgatacaaggctgttagagagataattggaattaatttgactgtaaacacaaagatattagtacaaaatacgtgacgtagaaagtaataatttcttgggtagtttgcagttttaaaattatgttttaaaatggactatcatatgcttaccgtaacttgaaagtatttcgatttcttggctttatatatcttgtggaaaggacgaaacaccgttagctataggctaataagatagttgtgtcaagtgcttcggagacctaacacgtctccagtcacaacggctaaaaatagcca

SEQ ID NO: 152 - DNA, 3364 bp, synthetic construct
  misc_feature 1..3364: note = plasmid including the sequence for B-Gen.1 human albumin target 30
  source 1..3364: mol_type = other DNA
gcactagtctgtcttcttggttgctgtttttttgttttcaacaccggtaccgcgttacaatgataagtcgactgaataagtgaactcgagatcagcctcgactgtgccttctagttgccagccatctgttgtttgcccctcccccgtgccttccttgaccctggaaggtgccactcccactgtcctttcctaataaaatgaggaaattgcatccccacttcagaagttcctatactttctagtgaatgagtgagctaactcacattaattgcgttgcgctcactgcccgctttccagtcgggaaacctgtcgtgccagctgcattaatgaatcggccaacgcgcggggagaggcggtttgcgtattgggcgctcttgcgcttcctcgctcactgactcgctgcgctcggtcgttcggctgcggcgagcggtatcagctcactcaaaggcggtaatacggttatccacagaatcaggggataacgcaggaaagaacatgtgagcaaaaggccagcaaaaggccaggaaccgtaaaaaggccgcgttgctggcgtttttccataggctccgcccccctgacgagcatcacaaaaatcgacgctcaagtcagaggtggcgaaacccgacaggactataaagataccaggcgtttccccctggaagctccctcgtgcgctctcctgttccgaccctgccgcttaccggatacctgtccgcctttctcccttcgggaagcgtggcgctttctcatagctcacgctgtaggtatctcagttcggtgtaggtcgttcgctccaagctgggctgtgtgcacgaaccccccgttcagcccgaccgctgcgccttatccggtaactatcgtcttgagtccaacccggtaagacacgacttatcgccactggcagcagccactggtaacaggattagcagagcgaggtatgtaggcggtgctacagagttcttgaagtggtggcctaactacggctacactagaagaacagtatttggtatctgcgctctgctgaagccagttaccttcggaaaaagagttggtagctcttgatccggcaaacaaaccaccgctggtagcggtggtttttttgtttgcaagcagcagattacgcgcagaaaaaaaggatctcaagaagatcctttgatcttttctacggggtctgacgctcagtggaacgaaaactcacgttaagggattttggtcatgagattatcaaaaaggatcttcacctagatccttttaaattaaaaatgaagttttaaatcaatctaaagtatatatgagtaaacttggtctgacagttaccaatgcttaatcagtgaggcacctatctcagcgatctgtctatttcgttcatccatagttgcctgactccccgtcgtgtagataactacgatacgggagggcttaccatctggccccagtgctgcaatgataccgcgtgacccacgctcaccggctccagatttatcagcaataaaccagccagccggaagggccgagcgcagaagtggtcctgcaactttatccgcctccatccagtctattaattgttgccgggaagctagagtaagtagttcgccagttaatagtttgcgcaacgttgttgccattgctacaggcatcgtggtgtcacgctcgtcgtttggtatggcttcattcagctccggttcccaacgatcaaggcgagttacatgatcccccatgttgtgcaaaaaagcggttagctccttcggtcctccgatcgttgtcagaagtaagttggccgcagtgttatcactcatggttatggcagcactgcataattctcttactgtcatgccatccgtaagatgcttttctgtgactggtgagtactcaaccaagtcattctgagaatagtgtatgcggcgaccgagttgctcttgcccggcgtcaatacgggataataccgcgccacatagcagaactttaaaagtgctcatcattggaaaacgttcttcggggcgaaaactctcaaggatcttaccgctgttgagatccagttcgatgtaacccactcgtgcacccaactgatcttcagcatcttttactttcaccagcgtttctgggtgagcaaaaacaggaaggcaaaatgccgcaaaaaagggaataagggcgacacggaaatgttgaatactcatactcttcctttttcaatattattgaagcatttatcagggttattgtctcatgagcggatacatatttgaatgtatttagaaaaataaacaaataggggttccgcgcatatttccccgaaaagtgccacctgacgtcgacggatcgggagatctcccgatcccctatggtgcactctcagtacaatctgctctgatgccgcatagttaagccagtatctgctccctgcttgtgtgttggaggtcgctgagtagtgcgcgagcaaaatttaagctacaacaaggcaaggcttgaccgagcaaacaaactctttctgtgttgtaaaacgacggccagtcttaagctcgggccccctgggcggttctgataacgagtaatcgttaatccgcaaataacgtaaaaacccgcttcggcgggtttttttatggggggagtttagggaaagagcatttgtcagaatatttaagggcgcctgtcactttgcttgatatatgagaattatttaaccttataaatgagaaaaaagcaacgcactttaaataagatacgttgctttttcgattgatgaacacctataattaaactattcatctattatttatgattttttgtatatacaatatttctagtttgttaaagagaattaagaaaataaatctcgaaaataataaagggaaaatcagtttttgatatcaaaattatacatgtcaacgataatacaaaatataatacaaactataagatgttatcagtatttattatgcatttagaataaattttgtgtcgcccttattcgactcactatagaagttcctattctctagaaagtagaggaacttcacttcattttgctagcgtgtgagggcctatttcccatgattccttcatatttgcatatacgatacaaggctgttagagagataattggaattaatttgactgtaaacacaaagatattagtacaaaatacgtgacgtagaaagtaataatttcttgggtagtttgcagttttaaaattatgttttaaaatggactatcatatgcttaccgtaacttgaaagtatttcgatttcttggctttatatatcttgtggaaaggacgaaacaccgttagctataggctaataagatagttgtgtcaagtgcttcggagacctaacacgtctccagtcacaacggctaaaaatagcca

SEQ ID NO: 153 - DNA, 3364 bp, synthetic construct
  misc_feature 1..3364: note = plasmid including the sequence for B-Gen.1 human albumin target 31
  source 1..3364: mol_type = other DNA
gcacgatattatctaagtttgaatatattttttgttttcaacaccggtaccgcgttacaatgataagtcgactgaataagtgaactcgagatcagcctcgactgtgccttctagttgccagccatctgttgtttgcccctcccccgtgccttccttgaccctggaaggtgccactcccactgtcctttcctaataaaatgaggaaattgcatccccacttcagaagttcctatactttctagtgaatgagtgagctaactcacattaattgcgttgcgctcactgcccgctttccagtcgggaaacctgtcgtgccagctgcattaatgaatcggccaacgcgcggggagaggcggtttgcgtattgggcgctcttgcgcttcctcgctcactgactcgctgcgctcggtcgttcggctgcggcgagcggtatcagctcactcaaaggcggtaatacggttatccacagaatcaggggataacgcaggaaagaacatgtgagcaaaaggccagcaaaaggccaggaaccgtaaaaaggccgcgttgctggcgtttttccataggctccgcccccctgacgagcatcacaaaaatcgacgctcaagtcagaggtggcgaaacccgacaggactataaagataccaggcgtttccccctggaagctccctcgtgcgctctcctgttccgaccctgccgcttaccggatacctgtccgcctttctcccttcgggaagcgtggcgctttctcatagctcacgctgtaggtatctcagttcggtgtaggtcgttcgctccaagctgggctgtgtgcacgaaccccccgttcagcccgaccgctgcgccttatccggtaactatcgtcttgagtccaacccggtaagacacgacttatcgccactggcagcagccactggtaacaggattagcagagcgaggtatgtaggcggtgctacagagttcttgaagtggtggcctaactacggctacactagaagaacagtatttggtatctgcgctctgctgaagccagttaccttcggaaaaagagttggtagctcttgatccggcaaacaaaccaccgctggtagcggtggtttttttgtttgcaagcagcagattacgcgcagaaaaaaaggatctcaagaagatcctttgatcttttctacggggtctgacgctcagtggaacgaaaactcacgttaagggattttggtcatgagattatcaaaaaggatcttcacctagatccttttaaattaaaaatgaagttttaaatcaatctaaagtatatatgagtaaacttggtctgacagttaccaatgcttaatcagtgaggcacctatctcagcgatctgtctatttcgttcatccatagttgcctgactccccgtcgtgtagataactacgatacgggagggcttaccatctggccccagtgctgcaatgataccgcgtgacccacgctcaccggctccagatttatcagcaataaaccagccagccggaagggccgagcgcagaagtggtcctgcaactttatccgcctccatccagtctattaattgttgccgggaagctagagtaagtagttcgccagttaatagtttgcgcaacgttgttgccattgctacaggcatcgtggtgtcacgctcgtcgtttggtatggcttcattcagctccggttcccaacgatcaaggcgagttacatgatcccccatgttgtgcaaaaaagcggttagctccttcggtcctccgatcgttgtcagaagtaagttggccgcagtgttatcactcatggttatggcagcactgcataattctcttactgtcatgccatccgtaagatgcttttctgtgactggtgagtactcaaccaagtcattctgagaatagtgtatgcggcgaccgagttgctcttgcccggcgtcaatacgggataataccgcgccacatagcagaactttaaaagtgctcatcattggaaaacgttcttcggggcgaaaactctcaaggatcttaccgctgttgagatccagttcgatgtaacccactcgtgcacccaactgatcttcagcatcttttactttcaccagcgtttctgggtgagcaaaaacaggaaggcaaaatgccgcaaaaaagggaataagggcgacacggaaatgttgaatactcatactcttcctttttcaatattattgaagcatttatcagggttattgtctcatgagcggatacatatttgaatgtatttagaaaaataaacaaataggggttccgcgcatatttccccgaaaagtgccacctgacgtcgacggatcgggagatctcccgatcccctatggtgcactctcagtacaatctgctctgatgccgcatagttaagccagtatctgctccctgcttgtgtgttggaggtcgctgagtagtgcgcgagcaaaatttaagctacaacaaggcaaggcttgaccgagcaaacaaactctttctgtgttgtaaaacgacggccagtcttaagctcgggccccctgggcggttctgataacgagtaatcgttaatccgcaaataacgtaaaaacccgcttcggcgggtttttttatggggggagtttagggaaagagcatttgtcagaatatttaagggcgcctgtcactttgcttgatatatgagaattatttaaccttataaatgagaaaaaagcaacgcactttaaataagatacgttgctttttcgattgatgaacacctataattaaactattcatctattatttatgattttttgtatatacaatatttctagtttgttaaagagaattaagaaaataaatctcgaaaataataaagggaaaatcagtttttgatatcaaaattatacatgtcaacgataatacaaaatataatacaaactataagatgttatcagtatttattatgcatttagaataaattttgtgtcgcccttattcgactcactatagaagttcctattctctagaaagtagaggaacttcacttcattttgctagcgtgtgagggcctatttcccatgattccttcatatttgcatatacgatacaaggctgttagagagataattggaattaatttgactgtaaacacaaagatattagtacaaaatacgtgacgtagaaagtaataatttcttgggtagtttgcagttttaaaattatgttttaaaatggactatcatatgcttaccgtaacttgaaagtatttcgatttcttggctttatatatcttgtggaaaggacgaaacaccgttagctataggctaataagatagttgtgtcaagtgcttcggagacctaacacgtctccagtcacaacggctaaaaatagcca

SEQ ID NO: 154 - DNA, 3364 bp, synthetic construct
  misc_feature 1..3364: note = plasmid including the sequence for B-Gen.1 human albumin target 32
  source 1..3364: mol_type = other DNA
gcactctaagtttgaatataaggctatttttttgttttcaacaccggtaccgcgttacaatgataagtcgactgaataagtgaactcgagatcagcctcgactgtgccttctagttgccagccatctgttgtttgcccctcccccgtgccttccttgaccctggaaggtgccactcccactgtcctttcctaataaaatgaggaaattgcatccccacttcagaagttcctatactttctagtgaatgagtgagctaactcacattaattgcgttgcgctcactgcccgctttccagtcgggaaacctgtcgtgccagctgcattaatgaatcggccaacgcgcggggagaggcggtttgcgtattgggcgctcttgcgcttcctcgctcactgactcgctgcgctcggtcgttcggctgcggcgagcggtatcagctcactcaaaggcggtaatacggttatccacagaatcaggggataacgcaggaaagaacatgtgagcaaaaggccagcaaaaggccaggaaccgtaaaaaggccgcgttgctggcgtttttccataggctccgcccccctgacgagcatcacaaaaatcgacgctcaagtcagaggtggcgaaacccgacaggactataaagataccaggcgtttccccctggaagctccctcgtgcgctctcctgttccgaccctgccgcttaccggatacctgtccgcctttctcccttcgggaagcgtggcgctttctcatagctcacgctgtaggtatctcagttcggtgtaggtcgttcgctccaagctgggctgtgtgcacgaaccccccgttcagcccgaccgctgcgccttatccggtaactatcgtcttgagtccaacccggtaagacacgacttatcgccactggcagcagccactggtaacaggattagcagagcgaggtatgtaggcggtgctacagagttcttgaagtggtggcctaactacggctacactagaagaacagtatttggtatctgcgctctgctgaagccagttaccttcggaaaaagagttggtagctcttgatccggcaaacaaaccaccgctggtagcggtggtttttttgtttgcaagcagcagattacgcgcagaaaaaaaggatctcaagaagatcctttgatcttttctacggggtctgacgctcagtggaacgaaaactcacgttaagggattttggtcatgagattatcaaaaaggatcttcacctagatccttttaaattaaaaatgaagttttaaatcaatctaaagtatatatgagtaaacttggtctgacagttaccaatgcttaatcagtgaggcacctatctcagcgatctgtctatttcgttcatccatagttgcctgactccccgtcgtgtagataactacgatacgggagggcttaccatctggccccagtgctgcaatgataccgcgtgacccacgctcaccggctccagatttatcagcaataaaccagccagccggaagggccgagcgcagaagtggtcctgcaactttatccgcctccatccagtctattaattgttgccgggaagctagagtaagtagttcgccagttaatagtttgcgcaacgttgttgccattgctacaggcatcgtggtgtcacgctcgtcgtttggtatggcttcattcagctccggttcccaacgatcaaggcgagttacatgatcccccatgttgtgcaaaaaagcggttagctccttcggtcctccgatcgttgtcagaagtaagttggccgcagtgttatcactcatggttatggcagcactgcataattctcttactgtcatgccatccgtaagatgcttttctgtgactggtgagtactcaaccaagtcattctgagaatagtgtatgcggcgaccgagttgctcttgcccggcgtcaatacgggataataccgcgccacatagcagaactttaaaagtgctcatcattggaaaacgttcttcggggcgaaaactctcaaggatcttaccgctgttgagatccagttcgatgtaacccactcgtgcacccaactgatcttcagcatcttttactttcaccagcgtttctgggtgagcaaaaacaggaaggcaaaatgccgcaaaaaagggaataagggcgacacggaaatgttgaatactcatactcttcctttttcaatattattgaagcatttatcagggttattgtctcatgagcggatacatatttgaatgtatttagaaaaataaacaaataggggttccgcgcatatttccccgaaaagtgccacctgacgtcgacggatcgggagatctcccgatcccctatggtgcactctcagtacaatctgctctgatgccgcatagttaagccagtatctgctccctgcttgtgtgttggaggtcgctgagtagtgcgcgagcaaaatttaagctacaacaaggcaaggcttgaccgagcaaacaaactctttctgtgttgtaaaacgacggccagtcttaagctcgggccccctgggcggttctgataacgagtaatcgttaatccgcaaataacgtaaaaacccgcttcggcgggtttttttatggggggagtttagggaaagagcatttgtcagaatatttaagggcgcctgtcactttgcttgatatatgagaattatttaaccttataaatgagaaaaaagcaacgcactttaaataagatacgttgctttttcgattgatgaacacctataattaaactattcatctattatttatgattttttgtatatacaatatttctagtttgttaaagagaattaagaaaataaatctcgaaaataataaagggaaaatcagtttttgatatcaaaattatacatgtcaacgataatacaaaatataatacaaactataagatgttatcagtatttattatgcatttagaataaattttgtgtcgcccttattcgactcactatagaagttcctattctctagaaagtagaggaacttcacttcattttgctagcgtgtgagggcctatttcccatgattccttcatatttgcatatacgatacaaggctgttagagagataattggaattaatttgactgtaaacacaaagatattagtacaaaatacgtgacgtagaaagtaataatttcttgggtagtttgcagttttaaaattatgttttaaaatggactatcatatgcttaccgtaacttgaaagtatttcgatttcttggctttatatatcttgtggaaaggacgaaacaccgttagctataggctaataagatagttgtgtcaagtgcttcggagacctaacacgtctccagtcacaacggctaaaaatagcca

SEQ ID NO: 155 - DNA, 3364 bp, synthetic construct
  misc_feature 1..3364: note = plasmid including the sequence for B-Gen.1 human albumin target 33
  source 1..3364: mol_type = other DNA
gcacatagccttatattcaaacttagattttttgttttcaacaccggtaccgcgttacaatgataagtcgactgaataagtgaactcgagatcagcctcgactgtgccttctagttgccagccatctgttgtttgcccctcccccgtgccttccttgaccctggaaggtgccactcccactgtcctttcctaataaaatgaggaaattgcatccccacttcagaagttcctatactttctagtgaatgagtgagctaactcacattaattgcgttgcgctcactgcccgctttccagtcgggaaacctgtcgtgccagctgcattaatgaatcggccaacgcgcggggagaggcggtttgcgtattgggcgctcttgcgcttcctcgctcactgactcgctgcgctcggtcgttcggctgcggcgagcggtatcagctcactcaaaggcggtaatacggttatccacagaatcaggggataacgcaggaaagaacatgtgagcaaaaggccagcaaaaggccaggaaccgtaaaaaggccgcgttgctggcgtttttccataggctccgcccccctgacgagcatcacaaaaatcgacgctcaagtcagaggtggcgaaacccgacaggactataaagataccaggcgtttccccctggaagctccctcgtgcgctctcctgttccgaccctgccgcttaccggatacctgtccgcctttctcccttcgggaagcgtggcgctttctcatagctcacgctgtaggtatctcagttcggtgtaggtcgttcgctccaagctgggctgtgtgcacgaaccccccgttcagcccgaccgctgcgccttatccggtaactatcgtcttgagtccaacccggtaagacacgacttatcgccactggcagcagccactggtaacaggattagcagagcgaggtatgtaggcggtgctacagagttcttgaagtggtggcctaactacggctacactagaagaacagtatttggtatctgcgctctgctgaagccagttaccttcggaaaaagagttggtagctcttgatccggcaaacaaaccaccgctggtagcggtggtttttttgtttgcaagcagcagattacgcgcagaaaaaaaggatctcaagaagatcctttgatcttttctacggggtctgacgctcagtggaacgaaaactcacgttaagggattttggtcatgagattatcaaaaaggatcttcacctagatccttttaaattaaaaatgaagttttaaatcaatctaaagtatatatgagtaaacttggtctgacagttaccaatgcttaatcagtgaggcacctatctcagcgatctgtctatttcgttcatccatagttgcctgactccccgtcgtgtagataactacgatacgggagggcttaccatctggccccagtgctgcaatgataccgcgtgacccacgctcaccggctccagatttatcagcaataaaccagccagccggaagggccgagcgcagaagtggtcctgcaactttatccgcctccatccagtctattaattgttgccgggaagctagagtaagtagttcgccagttaatagtttgcgcaacgttgttgccattgctacaggcatcgtggtgtcacgctcgtcgtttggtatggcttcattcagctccggttcccaacgatcaaggcgagttacatgatcccccatgttgtgcaaaaaagcggttagctccttcggtcctccgatcgttgtcagaagtaagttggccgcagtgttatcactcatggttatggcagcactgcataattctcttactgtcatgccatccgtaagatgcttttctgtgactggtgagtactcaaccaagtcattctgagaatagtgtatgcggcgaccgagttgctcttgcccggcgtcaatacgggataataccgcgccacatagcagaactttaaaagtgctcatcattggaaaacgttcttcggggcgaaaactctcaaggatcttaccgctgttgagatccagttcgatgtaacccactcgtgcacccaactgatcttcagcatcttttactttcaccagcgtttctgggtgagcaaaaacaggaaggcaaaatgccgcaaaaaagggaataagggcgacacggaaatgttgaatactcatactcttcctttttcaatattattgaagcatttatcagggttattgtctcatgagcggatacatatttgaatgtatttagaaaaataaacaaataggggttccgcgcatatttccccgaaaagtgccacctgacgtcgacggatcgggagatctcccgatcccctatggtgcactctcagtacaatctgctctgatgccgcatagttaagccagtatctgctccctgcttgtgtgttggaggtcgctgagtagtgcgcgagcaaaatttaagctacaacaaggcaaggcttgaccgagcaaacaaactctttctgtgttgtaaaacgacggccagtcttaagctcgggccccctgggcggttctgataacgagtaatcgttaatccgcaaataacgtaaaaacccgcttcggcgggtttttttatggggggagtttagggaaagagcatttgtcagaatatttaagggcgcctgtcactttgcttgatatatgagaattatttaaccttataaatgagaaaaaagcaacgcactttaaataagatacgttgctttttcgattgatgaacacctataattaaactattcatctattatttatgattttttgtatatacaatatttctagtttgttaaagagaattaagaaaataaatctcgaaaataataaagggaaaatcagtttttgatatcaaaattatacatgtcaacgataatacaaaatataatacaaactataagatgttatcagtatttattatgcatttagaataaattttgtgtcgcccttattcgactcactatagaagttcctattctctagaaagtagaggaacttcacttcattttgctagcgtgtgagggcctatttcccatgattccttcatatttgcatatacgatacaaggctgttagagagataattggaattaatttgactgtaaacacaaagatattagtacaaaatacgtgacgtagaaagtaataatttcttgggtagtttgcagttttaaaattatgttttaaaatggactatcatatgcttaccgtaacttgaaagtatttcgatttcttggctttatatatcttgtggaaaggacgaaacaccgttagctataggctaataagatagttgtgtcaagtgcttcggagacctaacacgtctccagtcacaacggctaaaaatagcca

SEQ ID NO: 156 - DNA, 3364 bp, synthetic construct
  misc_feature 1..3364: note = plasmid including the sequence for B-Gen.1 human albumin target 34
  source 1..3364: mol_type = other DNA
gcacaataatttttaaaatagtattctttttttgttttcaacaccggtaccgcgttacaatgataagtcgactgaataagtgaactcgagatcagcctcgactgtgccttctagttgccagccatctgttgtttgcccctcccccgtgccttccttgaccctggaaggtgccactcccactgtcctttcctaataaaatgaggaaattgcatccccacttcagaagttcctatactttctagtgaatgagtgagctaactcacattaattgcgttgcgctcactgcccgctttccagtcgggaaacctgtcgtgccagctgcattaatgaatcggccaacgcgcggggagaggcggtttgcgtattgggcgctcttgcgcttcctcgctcactgactcgctgcgctcggtcgttcggctgcggcgagcggtatcagctcactcaaaggcggtaatacggttatccacagaatcaggggataacgcaggaaagaacatgtgagcaaaaggccagcaaaaggccaggaaccgtaaaaaggccgcgttgctggcgtttttccataggctccgcccccctgacgagcatcacaaaaatcgacgctcaagtcagaggtggcgaaacccgacaggactataaagataccaggcgtttccccctggaagctccctcgtgcgctctcctgttccgaccctgccgcttaccggatacctgtccgcctttctcccttcgggaagcgtggcgctttctcatagctcacgctgtaggtatctcagttcggtgtaggtcgttcgctccaagctgggctgtgtgcacgaaccccccgttcagcccgaccgctgcgccttatccggtaactatcgtcttgagtccaacccggtaagacacgacttatcgccactggcagcagccactggtaacaggattagcagagcgaggtatgtaggcggtgctacagagttcttgaagtggtggcctaactacggctacactagaagaacagtatttggtatctgcgctctgctgaagccagttaccttcggaaaaagagttggtagctcttgatccggcaaacaaaccaccgctggtagcggtggtttttttgtttgcaagcagcagattacgcgcagaaaaaaaggatctcaagaagatcctttgatcttttctacggggtctgacgctcagtggaacgaaaactcacgttaagggattttggtcatgagattatcaaaaaggatcttcacctagatccttttaaattaaaaatgaagttttaaatcaatctaaagtatatatgagtaaacttggtctgacagttaccaatgcttaatcagtgaggcacctatctcagcgatctgtctatttcgttcatccatagttgcctgactccccgtcgtgtagataactacgatacgggagggcttaccatctggccccagtgctgcaatgataccgcgtgacccacgctcaccggctccagatttatcagcaataaaccagccagccggaagggccgagcgcagaagtggtcctgcaactttatccgcctccatccagtctattaattgttgccgggaagctagagtaagtagttcgccagttaatagtttgcgcaacgttgttgccattgctacaggcatcgtggtgtcacgctcgtcgtttggtatggcttcattcagctccggttcccaacgatcaaggcgagttacatgatcccccatgttgtgcaaaaaagcggttagctccttcggtcctccgatcgttgtcagaagtaagttggccgcagtgttatcactcatggttatggcagcactgcataattctcttactgtcatgccatccgtaagatgcttttctgtgactggtgagtactcaaccaagtcattctgagaatagtgtatgcggcgaccgagttgctcttgcccggcgtcaatacgggataataccgcgccacatagcagaactttaaaagtgctcatcattggaaaacgttcttcggggcgaaaactctcaaggatcttaccgctgttgagatccagttcgatgtaacccactcgtgcacccaactgatcttcagcatcttttactttcaccagcgtttctgggtgagcaaaaacaggaaggcaaaatgccgcaaaaaagggaataagggcgacacggaaatgttgaatactcatactcttcctttttcaatattattgaagcatttatcagggttattgtctcatgagcggatacatatttgaatgtatttagaaaaataaacaaataggggttccgcgcatatttccccgaaaagtgccacctgacgtcgacggatcgggagatctcccgatcccctatggtgcactctcagtacaatctgctctgatgccgcatagttaagccagtatctgctccctgcttgtgtgttggaggtcgctgagtagtgcgcgagcaaaatttaagctacaacaaggcaaggcttgaccgagcaaacaaactctttctgtgttgtaaaacgacggccagtcttaagctcgggccccctgggcggttctgataacgagtaatcgttaatccgcaaataacgtaaaaacccgcttcggcgggtttttttatggggggagtttagggaaagagcatttgtcagaatatttaagggcgcctgtcactttgcttgatatatgagaattatttaaccttataaatgagaaaaaagcaacgcactttaaataagatacgttgctttttcgattgatgaacacctataattaaactattcatctattatttatgattttttgtatatacaatatttctagtttgttaaagagaattaagaaaataaatctcgaaaataataaagggaaaatcagtttttgatatcaaaattatacatgtcaacgataatacaaaatataatacaaactataagatgttatcagtatttattatgcatttagaataaattttgtgtcgcccttattcgactcactatagaagttcctattctctagaaagtagaggaacttcacttcattttgctagcgtgtgagggcctatttcccatgattccttcatatttgcatatacgatacaaggctgttagagagataattggaattaatttgactgtaaacacaaagatattagtacaaaatacgtgacgtagaaagtaataatttcttgggtagtttgcagttttaaaattatgttttaaaatggactatcatatgcttaccgtaacttgaaagtatttcgatttcttggctttatatatcttgtggaaaggacgaaacaccgttagctataggctaataagatagttgtgtcaagtgcttcggagacctaacacgtctccagtcacaacggctaaaaatagcca

SEQ ID NO: 157 - DNA, 3364 bp, synthetic construct
  misc_feature 1..3364: note = plasmid including the sequence for B-Gen.1 human albumin target 35
  source 1..3364: mol_type = other DNA
gcacaatatttatagccttatattcaattttttgttttcaacaccggtaccgcgttacaatgataagtcgactgaataagtgaactcgagatcagcctcgactgtgccttctagttgccagccatctgttgtttgcccctcccccgtgccttccttgaccctggaaggtgccactcccactgtcctttcctaataaaatgaggaaattgcatccccacttcagaagttcctatactttctagtgaatgagtgagctaactcacattaattgcgttgcgctcactgcccgctttccagtcgggaaacctgtcgtgccagctgcattaatgaatcggccaacgcgcggggagaggcggtttgcgtattgggcgctcttgcgcttcctcgctcactgactcgctgcgctcggtcgttcggctgcggcgagcggtatcagctcactcaaaggcggtaatacggttatccacagaatcaggggataacgcaggaaagaacatgtgagcaaaaggccagcaaaaggccaggaaccgtaaaaaggccgcgttgctggcgtttttccataggctccgcccccctgacgagcatcacaaaaatcgacgctcaagtcagaggtggcgaaacccgacaggactataaagataccaggcgtttccccctggaagctccctcgtgcgctctcctgttccgaccctgccgcttaccggatacctgtccgcctttctcccttcgggaagcgtggcgctttctcatagctcacgctgtaggtatctcagttcggtgtaggtcgttcgctccaagctgggctgtgtgcacgaaccccccgttcagcccgaccgctgcgccttatccggtaactatcgtcttgagtccaacccggtaagacacgacttatcgccactggcagcagccactggtaacaggattagcagagcgaggtatgtaggcggtgctacagagttcttgaagtggtggcctaactacggctacactagaagaacagtatttggtatctgcgctctgctgaagccagttaccttcggaaaaagagttggtagctcttgatccggcaaacaaaccaccgctggtagcggtggtttttttgtttgcaagcagcagattacgcgcagaaaaaaaggatctcaagaagatcctttgatcttttctacggggtctgacgctcagtggaacgaaaactcacgttaagggattttggtcatgagattatcaaaaaggatcttcacctagatccttttaaattaaaaatgaagttttaaatcaatctaaagtatatatgagtaaacttggtctgacagttaccaatgcttaatcagtgaggcacctatctcagcgatctgtctatttcgttcatccatagttgcctgactccccgtcgtgtagataactacgatacgggagggcttaccatctggccccagtgctgcaatgataccgcgtgacccacgctcaccggctccagatttatcagcaataaaccagccagccggaagggccgagcgcagaagtggtcctgcaactttatccgcctccatccagtctattaattgttgccgggaagctagagtaagtagttcgccagttaatagtttgcgcaacgttgttgccattgctacaggcatcgtggtgtcacgctcgtcgtttggtatggcttcattcagctccggttcccaacgatcaaggcgagttacatgatcccccatgttgtgcaaaaaagcggttagctccttcggtcctccgatcgttgtcagaagtaagttggccgcagtgttatcactcatggttatggcagcactgcataattctcttactgtcatgccatccgtaagatgcttttctgtgactggtgagtactcaaccaagtcattctgagaatagtgtatgcggcgaccgagttgctcttgcccggcgtcaatacgggataataccgcgccacatagcagaactttaaaagtgctcatcattggaaaacgttcttcggggcgaaaactctcaaggatcttaccgctgttgagatccagttcgatgtaacccactcgtgcacccaactgatcttcagcatcttttactttcaccagcgtttctgggtgagcaaaaacaggaaggcaaaatgccgcaaaaaagggaataagggcgacacggaaatgttgaatactcatactcttcctttttcaatattattgaagcatttatcagggttattgtctcatgagcggatacatatttgaatgtatttagaaaaataaacaaataggggttccgcgcatatttccccgaaaagtgccacctgacgtcgacggatcgggagatctcccgatcccctatggtgcactctcagtacaatctgctctgatgccgcatagttaagccagtatctgctccctgcttgtgtgttggaggtcgctgagtagtgcgcgagcaaaatttaagctacaacaaggcaaggcttgaccgagcaaacaaactctttctgtgttgtaaaacgacggccagtcttaagctcgggccccctgggcggttctgataacgagtaatcgttaatccgcaaataacgtaaaaacccgcttcggcgggtttttttatggggggagtttagggaaagagcatttgtcagaatatttaagggcgcctgtcactttgcttgatatatgagaattatttaaccttataaatgagaaaaaagcaacgcactttaaataagatacgttgctttttcgattgatgaacacctataattaaactattcatctattatttatgattttttgtatatacaatatttctagtttgttaaagagaattaagaaaataaatctcgaaaataataaagggaaaatcagtttttgatatcaaaattatacatgtcaacgataatacaaaatataatacaaactataagatgttatcagtatttattatgcatttagaataaattttgtgtcgcccttattcgactcactatagaagttcctattctctagaaagtagaggaacttcacttcattttgctagcgtgtgagggcctatttcccatgattccttcatatttgcatatacgatacaaggctgttagagagataattggaattaatttgactgtaaacacaaagatattagtacaaaatacgtgacgtagaaagtaataatttcttgggtagtttgcagttttaaaattatgttttaaaatggactatcatatgcttaccgtaacttgaaagtatttcgatttcttggctttatatatcttgtggaaaggacgaaacaccgttagctataggctaataagatagttgtgtcaagtgcttcggagacctaacacgtctccagtcacaacggctaaaaatagcca

SEQ ID NO: 158 - DNA, 3364 bp, synthetic construct
  misc_feature 1..3364: note = plasmid including the sequence for B-Gen.1 human albumin target 36
  source 1..3364: mol_type = other DNA
gcacttaaatatttatagccttatattttttttgttttcaacaccggtaccgcgttacaatgataagtcgactgaataagtgaactcgagatcagcctcgactgtgccttctagttgccagccatctgttgtttgcccctcccccgtgccttccttgaccctggaaggtgccactcccactgtcctttcctaataaaatgaggaaattgcatccccacttcagaagttcctatactttctagtgaatgagtgagctaactcacattaattgcgttgcgctcactgcccgctttccagtcgggaaacctgtcgtgccagctgcattaatgaatcggccaacgcgcggggagaggcggtttgcgtattgggcgctcttgcgcttcctcgctcactgactcgctgcgctcggtcgttcggctgcggcgagcggtatcagctcactcaaaggcggtaatacggttatccacagaatcaggggataacgcaggaaagaacatgtgagcaaaaggccagcaaaaggccaggaaccgtaaaaaggccgcgttgctggcgtttttccataggctccgcccccctgacgagcatcacaaaaatcgacgctcaagtcagaggtggcgaaacccgacaggactataaagataccaggcgtttccccctggaagctccctcgtgcgctctcctgttccgaccctgccgcttaccggatacctgtccgcctttctcccttcgggaagcgtggcgctttctcatagctcacgctgtaggtatctcagttcggtgtaggtcgttcgctccaagctgggctgtgtgcacgaaccccccgttcagcccgaccgctgcgccttatccggtaactatcgtcttgagtccaacccggtaagacacgacttatcgccactggcagcagccactggtaacaggattagcagagcgaggtatgtaggcggtgctacagagttcttgaagtggtggcctaactacggctacactagaagaacagtatttggtatctgcgctctgctgaagccagttaccttcggaaaaagagttggtagctcttgatccggcaaacaaaccaccgctggtagcggtggtttttttgtttgcaagcagcagattacgcgcagaaaaaaaggatctcaagaagatcctttgatcttttctacggggtctgacgctcagtggaacgaaaactcacgttaagggattttggtcatgagattatcaaaaaggatcttcacctagatccttttaaattaaaaatgaagttttaaatcaatctaaagtatatatgagtaaacttggtctgacagttaccaatgcttaatcagtgaggcacctatctcagcgatctgtctatttcgttcatccatagttgcctgactccccgtcgtgtagataactacgatacgggagggcttaccatctggccccagtgctgcaatgataccgcgtgacccacgctcaccggctccagatttatcagcaataaaccagccagccggaagggccgagcgcagaagtggtcctgcaactttatccgcctccatccagtctattaattgttgccgggaagctagagtaagtagttcgccagttaatagtttgcgcaacgttgttgccattgctacaggcatcgtggtgtcacgctcgtcgtttggtatggcttcattcagctccggttcccaacgatcaaggcgagttacatgatcccccatgttgtgcaaaaaagcggttagctccttcggtcctccgatcgttgtcagaagtaagttggccgcagtgttatcactcatggttatggcagcactgcataattctcttactgtcatgccatccgtaagatgcttttctgtgactggtgagtactcaaccaagtcattctgagaatagtgtatgcggcgaccgagttgctcttgcccggcgtcaatacgggataataccgcgccacatagcagaactttaaaagtgctcatcattggaaaacgttcttcggggcgaaaactctcaaggatcttaccgctgttgagatccagttcgatgtaacccactcgtgcacccaactgatcttcagcatcttttactttcaccagcgtttctgggtgagcaaaaacaggaaggcaaaatgccgcaaaaaagggaataagggcgacacggaaatgttgaatactcatactcttcctttttcaatattattgaagcatttatcagggttattgtctcatgagcggatacatatttgaatgtatttagaaaaataaacaaataggggttccgcgcatatttccccgaaaagtgccacctgacgtcgacggatcgggagatctcccgatcccctatggtgcactctcagtacaatctgctctgatgccgcatagttaagccagtatctgctccctgcttgtgtgttggaggtcgctgagtagtgcgcgagcaaaatttaagctacaacaaggcaaggcttgaccgagcaaacaaactctttctgtgttgtaaaacgacggccagtcttaagctcgggccccctgggcggttctgataacgagtaatcgttaatccgcaaataacgtaaaaacccgcttcggcgggtttttttatggggggagtttagggaaagagcatttgtcagaatatttaagggcgcctgtcactttgcttgatatatgagaattatttaaccttataaatgagaaaaaagcaacgcactttaaataagatacgttgctttttcgattgatgaacacctataattaaactattcatctattatttatgattttttgtatatacaatatttctagtttgttaaagagaattaagaaaataaatctcgaaaataataaagggaaaatcagtttttgatatcaaaattatacatgtcaacgataatacaaaatataatacaaactataagatgttatcagtatttattatgcatttagaataaattttgtgtcgcccttattcgactcactatagaagttcctattctctagaaagtagaggaacttcacttcattttgctagcgtgtgagggcctatttcccatgattccttcatatttgcatatacgatacaaggctgttagagagataattggaattaatttgactgtaaacacaaagatattagtacaaaatacgtgacgtagaaagtaataatttcttgggtagtttgcagttttaaaattatgttttaaaatggactatcatatgcttaccgtaacttgaaagtatttcgatttcttggctttatatatcttgtggaaaggacgaaacaccgttagctataggctaataagatagttgtgtcaagtgcttcggagacctaacacgtctccagtcacaacggctaaaaatagcca

SEQ ID NO: 159 - DNA, 3364 bp, synthetic construct
  misc_feature 1..3364: note = plasmid including the sequence for B-Gen.1 human albumin target 37
  source 1..3364: mol_type = other DNA
gcacttaaaatagtattcttggtaattttttttgttttcaacaccggtaccgcgttacaatgataagtcgactgaataagtgaactcgagatcagcctcgactgtgccttctagttgccagccatctgttgtttgcccctcccccgtgccttccttgaccctggaaggtgccactcccactgtcctttcctaataaaatgaggaaattgcatccccacttcagaagttcctatactttctagtgaatgagtgagctaactcacattaattgcgttgcgctcactgcccgctttccagtcgggaaacctgtcgtgccagctgcattaatgaatcggccaacgcgcggggagaggcggtttgcgtattgggcgctcttgcgcttcctcgctcactgactcgctgcgctcggtcgttcggctgcggcgagcggtatcagctcactcaaaggcggtaatacggttatccacagaatcaggggataacgcaggaaagaacatgtgagcaaaaggccagcaaaaggccaggaaccgtaaaaaggccgcgttgctggcgtttttccataggctccgcccccctgacgagcatcacaaaaatcgacgctcaagtcagaggtggcgaaacccgacaggactataaagataccaggcgtttccccctggaagctccctcgtgcgctctcctgttccgaccctgccgcttaccggatacctgtccgcctttctcccttcgggaagcgtggcgctttctcatagctcacgctgtaggtatctcagttcggtgtaggtcgttcgctccaagctgggctgtgtgcacgaaccccccgttcagcccgaccgctgcgccttatccggtaactatcgtcttgagtccaacccggtaagacacgacttatcgccactggcagcagccactggtaacaggattagcagagcgaggtatgtaggcggtgctacagagttcttgaagtggtggcctaactacggctacactagaagaacagtatttggtatctgcgctctgctgaagccagttaccttcggaaaaagagttggtagctcttgatccggcaaacaaaccaccgctggtagcggtggtttttttgtttgcaagcagcagattacgcgcagaaaaaaaggatctcaagaagatcctttgatcttttctacggggtctgacgctcagtggaacgaaaactcacgttaagggattttggtcatgagattatcaaaaaggatcttcacctagatccttttaaattaaaaatgaagttttaaatcaatctaaagtatatatgagtaaacttggtctgacagttaccaatgcttaatcagtgaggcacctatctcagcgatctgtctatttcgttcatccatagttgcctgactccccgtcgtgtagataactacgatacgggagggcttaccatctggccccagtgctgcaatgataccgcgtgacccacgctcaccggctccagatttatcagcaataaaccagccagccggaagggccgagcgcagaagtggtcctgcaactttatccgcctccatccagtctattaattgttgccgggaagctagagtaagtagttcgccagttaatagtttgcgcaacgttgttgccattgctacaggcatcgtggtgtcacgctcgtcgtttggtatggcttcattcagctccggttcccaacgatcaaggcgagttacatgatcccccatgttgtgcaaaaaagcggttagctccttcggtcctccgatcgttgtcagaagtaagttggccgcagtgttatcactcatggttatggcagcactgcataattctcttactgtcatgccatccgtaagatgcttttctgtgactggtgagtactcaaccaagtcattctgagaatagtgtatgcggcgaccgagttgctcttgcccggcgtcaatacgggataataccgcgccacatagcagaactttaaaagtgctcatcattggaaaacgttcttcggggcgaaaactctcaaggatcttaccgctgttgagatccagttcgatgtaacccactcgtgcacccaactgatcttcagcatcttttactttcaccagcgtttctgggtgagcaaaaacaggaaggcaaaatgccgcaaaaaagggaataagggcgacacggaaatgttgaatactcatactcttcctttttcaatattattgaagcatttatcagggttattgtctcatgagcggatacatatttgaatgtatttagaaaaataaacaaataggggttccgcgcatatttccccgaaaagtgccacctgacgtcgacggatcgggagatctcccgatcccctatggtgcactctcagtacaatctgctctgatgccgcatagttaagccagtatctgctccctgcttgtgtgttggaggtcgctgagtagtgcgcgagcaaaatttaagctacaacaaggcaaggcttgaccgagcaaacaaactctttctgtgttgtaaaacgacggccagtcttaagctcgggccccctgggcggttctgataacgagtaatcgttaatccgcaaataacgtaaaaacccgcttcggcgggtttttttatggggggagtttagggaaagagcatttgtcagaatatttaagggcgcctgtcactttgcttgatatatgagaattatttaaccttataaatgagaaaaaagcaacgcactttaaataagatacgttgctttttcgattgatgaacacctataattaaactattcatctattatttatgattttttgtatatacaatatttctagtttgttaaagagaattaagaaaataaatctcgaaaataataaagggaaaatcagtttttgatatcaaaattatacatgtcaacgataatacaaaatataatacaaactataagatgttatcagtatttattatgcatttagaataaattttgtgtcgcccttattcgactcactatagaagttcctattctctagaaagtagaggaacttcacttcattttgctagcgtgtgagggcctatttcccatgattccttcatatttgcatatacgatacaaggctgttagagagataattggaattaatttgactgtaaacacaaagatattagtacaaaatacgtgacgtagaaagtaataatttcttgggtagtttgcagttttaaaattatgttttaaaatggactatcatatgcttaccgtaacttgaaagtatttcgatttcttggctttatatatcttgtggaaaggacgaaacaccgttagctataggctaataagatagttgtgtcaagtgcttcggagacctaacacgtctccagtcacaacggctaaaaatagcca

SEQ ID NO: 160 - DNA, 3364 bp, synthetic construct
  misc_feature 1..3364: note = plasmid including the sequence for B-Gen.1 human albumin target 38
  source 1..3364: mol_type = other DNA
gcactaaaaattattaaatatttatagttttttgttttcaacaccggtaccgcgttacaatgataagtcgactgaataagtgaactcgagatcagcctcgactgtgccttctagttgccagccatctgttgtttgcccctcccccgtgccttccttgaccctggaaggtgccactcccactgtcctttcctaataaaatgaggaaattgcatccccacttcagaagttcctatactttctagtgaatgagtgagctaactcacattaattgcgttgcgctcactgcccgctttccagtcgggaaacctgtcgtgccagctgcattaatgaatcggccaacgcgcggggagaggcggtttgcgtattgggcgctcttgcgcttcctcgctcactgactcgctgcgctcggtcgttcggctgcggcgagcggtatcagctcactcaaaggcggtaatacggttatccacagaatcaggggataacgcaggaaagaacatgtgagcaaaaggccagcaaaaggccaggaaccgtaaaaaggccgcgttgctggcgtttttccataggctccgcccccctgacgagcatcacaaaaatcgacgctcaagtcagaggtggcgaaacccgacaggactataaagataccaggcgtttccccctggaagctccctcgtgcgctctcctgttccgaccctgccgcttaccggatacctgtccgcctttctcccttcgggaagcgtggcgctttctcatagctcacgctgtaggtatctcagttcggtgtaggtcgttcgctccaagctgggctgtgtgcacgaaccccccgttcagcccgaccgctgcgccttatccggtaactatcgtcttgagtccaacccggtaagacacgacttatcgccactggcagcagccactggtaacaggattagcagagcgaggtatgtaggcggtgctacagagttcttgaagtggtggcctaactacggctacactagaagaacagtatttggtatctgcgctctgctgaagccagttaccttcggaaaaagagttggtagctcttgatccggcaaacaaaccaccgctggtagcggtggtttttttgtttgcaagcagcagattacgcgcagaaaaaaaggatctcaagaagatcctttgatcttttctacggggtctgacgctcagtggaacgaaaactcacgttaagggattttggtcatgagattatcaaaaaggatcttcacctagatccttttaaattaaaaatgaagttttaaatcaatctaaagtatatatgagtaaacttggtctgacagttaccaatgcttaatcagtgaggcacctatctcagcgatctgtctatttcgttcatccatagttgcctgactccccgtcgtgtagataactacgatacgggagggcttaccatctggccccagtgctgcaatgataccgcgtgacccacgctcaccggctccagatttatcagcaataaaccagccagccggaagggccgagcgcagaagtggtcctgcaactttatccgcctccatccagtctattaattgttgccgggaagctagagtaagtagttcgccagttaatagtttgcgcaacgttgttgccattgctacaggcatcgtggtgtcacgctcgtcgtttggtatggcttcattcagctccggttcccaacgatcaaggcgagttacatgatcccccatgttgtgcaaaaaagcggttagctccttcggtcctccgatcgttgtcagaagtaagttggccgcagtgttatcactcatggttatggcagcactgcataattctcttactgtcatgccatccgtaagatgcttttctgtgactggtgagtactcaaccaagtcattctgagaatagtgtatgcggcgaccgagttgctcttgcccggcgtcaatacgggataataccgcgccacatagcagaactttaaaagtgctcatcattggaaaacgttcttcggggcgaaaactctcaaggatcttaccgctgttgagatccagttcgatgtaacccactcgtgcacccaactgatcttcagcatcttttactttcaccagcgtttctgggtgagcaaaaacaggaaggcaaaatgccgcaaaaaagggaataagggcgacacggaaatgttgaatactcatactcttcctttttcaatattattgaagcatttatcagggttattgtctcatgagcggatacatatttgaatgtatttagaaaaataaacaaataggggttccgcgcatatttccccgaaaagtgccacctgacgtcgacggatcgggagatctcccgatcccctatggtgcactctcagtacaatctgctctgatgccgcatagttaagccagtatctgctccctgcttgtgtgttggaggtcgctgagtagtgcgcgagcaaaatttaagctacaacaaggcaaggcttgaccgagcaaacaaactctttctgtgttgtaaaacgacggccagtcttaagctcgggccccctgggcggttctgataacgagtaatcgttaatccgcaaataacgtaaaaacccgcttcggcgggtttttttatggggggagtttagggaaagagcatttgtcagaatatttaagggcgcctgtcactttgcttgatatatgagaattatttaaccttataaatgagaaaaaagcaacgcactttaaataagatacgttgctttttcgattgatgaacacctataattaaactattcatctattatttatgattttttgtatatacaatatttctagtttgttaaagagaattaagaaaataaatctcgaaaataataaagggaaaatcagtttttgatatcaaaattatacatgtcaacgataatacaaaatataatacaaactataagatgttatcagtatttattatgcatttagaataaattttgtgtcgcccttattcgactcactatagaagttcctattctctagaaagtagaggaacttcacttcattttgctagcgtgtgagggcctatttcccatgattccttcatatttgcatatacgatacaaggctgttagagagataattggaattaatttgactgtaaacacaaagatattagtacaaaatacgtgacgtagaaagtaataatttcttgggtagtttgcagttttaaaattatgttttaaaatggactatcatatgcttaccgtaacttgaaagtatttcgatttcttggctttatatatcttgtggaaaggacgaaacaccgttagctataggctaataagatagttgtgtcaagtgcttcggagacctaacacgtctccagtcacaacggctaaaaatagcca

SEQ ID NO: 161 - DNA, 3364 bp, synthetic construct
  misc_feature 1..3364: note = plasmid including the sequence for B-Gen.1 human albumin target 39
  source 1..3364: mol_type = other DNA
gcacttggtaattgaattattcttctgttttttgttttcaacaccggtaccgcgttacaatgataagtcgactgaataagtgaactcgagatcagcctcgactgtgccttctagttgccagccatctgttgtttgcccctcccccgtgccttccttgaccctggaaggtgccactcccactgtcctttcctaataaaatgaggaaattgcatccccacttcagaagttcctatactttctagtgaatgagtgagctaactcacattaattgcgttgcgctcactgcccgctttccagtcgggaaacctgtcgtgccagctgcattaatgaatcggccaacgcgcggggagaggcggtttgcgtattgggcgctcttgcgcttcctcgctcactgactcgctgcgctcggtcgttcggctgcggcgagcggtatcagctcactcaaaggcggtaatacggttatccacagaatcaggggataacgcaggaaagaacatgtgagcaaaaggccagcaaaaggccaggaaccgtaaaaaggccgcgttgctggcgtttttccataggctccgcccccctgacgagcatcacaaaaatcgacgctcaagtcagaggtggcgaaacccgacaggactataaagataccaggcgtttccccctggaagctccctcgtgcgctctcctgttccgaccctgccgcttaccggatacctgtccgcctttctcccttcgggaagcgtggcgctttctcatagctcacgctgtaggtatctcagttcggtgtaggtcgttcgctccaagctgggctgtgtgcacgaaccccccgttcagcccgaccgctgcgccttatccggtaactatcgtcttgagtccaacccggtaagacacgacttatcgccactggcagcagccactggtaacaggattagcagagcgaggtatgtaggcggtgctacagagttcttgaagtggtggcctaactacggctacactagaagaacagtatttggtatctgcgctctgctgaagccagttaccttcggaaaaagagttggtagctcttgatccggcaaacaaaccaccgctggtagcggtggtttttttgtttgcaagcagcagattacgcgcagaaaaaaaggatctcaagaagatcctttgatcttttctacggggtctgacgctcagtggaacgaaaactcacgttaagggattttggtcatgagattatcaaaaaggatcttcacctagatccttttaaattaaaaatgaagttttaaatcaatctaaagtatatatgagtaaacttggtctgacagttaccaatgcttaatcagtgaggcacctatctcagcgatctgtctatttcgttcatccatagttgcctgactccccgtcgtgtagataactacgatacgggagggcttaccatctggccccagtgctgcaatgataccgcgtgacccacgctcaccggctccagatttatcagcaataaaccagccagccggaagggccgagcgcagaagtggtcctgcaactttatccgcctccatccagtctattaattgttgccgggaagctagagtaagtagttcgccagttaatagtttgcgcaacgttgttgccattgctacaggcatcgtggtgtcacgctcgtcgtttggtatggcttcattcagctccggttcccaacgatcaaggcgagttacatgatcccccatgttgtgcaaaaaagcggttagctccttcggtcctccgatcgttgtcagaagtaagttggccgcagtgttatcactcatggttatggcagcactgcataattctcttactgtcatgccatccgtaagatgcttttctgtgactggtgagtactcaaccaagtcattctgagaatagtgtatgcggcgaccgagttgctcttgcccggcgtcaatacgggataataccgcgccacatagcagaactttaaaagtgctcatcattggaaaacgttcttcggggcgaaaactctcaaggatcttaccgctgttgagatccagttcgatgtaacccactcgtgcacccaactgatcttcagcatcttttactttcaccagcgtttctgggtgagcaaaaacaggaaggcaaaatgccgcaaaaaagggaataagggcgacacggaaatgttgaatactcatactcttcctttttcaatattattgaagcatttatcagggttattgtctcatgagcggatacatatttgaatgtatttagaaaaataaacaaataggggttccgcgcatatttccccgaaaagtgccacctgacgtcgacggatcgggagatctcccgatcccctatggtgcactctcagtacaatctgctctgatgccgcatagttaagccagtatctgctccctgcttgtgtgttggaggtcgctgagtagtgcgcgagcaaaatttaagctacaacaaggcaaggcttgaccgagcaaacaaactctttctgtgttgtaaaacgacggccagtcttaagctcgggccccctgggcggttctgataacgagtaatcgttaatccgcaaataacgtaaaaacccgcttcggcgggtttttttatggggggagtttagggaaagagcatttgtcagaatatttaagggcgcctgtcactttgcttgatatatgagaattatttaaccttataaatgagaaaaaagcaacgcactttaaataagatacgttgctttttcgattgatgaacacctataattaaactattcatctattatttatgattttttgtatatacaatatttctagtttgttaaagagaattaagaaaataaatctcgaaaataataaagggaaaatcagtttttgatatcaaaattatacatgtcaacgataatacaaaatataatacaaactataagatgttatcagtatttattatgcatttagaataaattttgtgtcgcccttattcgactcactatagaagttcctattctctagaaagtagaggaacttcacttcattttgctagcgtgtgagggcctatttcccatgattccttcatatttgcatatacgatacaaggctgttagagagataattggaattaatttgactgtaaacacaaagatattagtacaaaatacgtgacgtagaaagtaataatttcttgggtagtttgcagttttaaaattatgttttaaaatggactatcatatgcttaccgtaacttgaaagtatttcgatttcttggctttatatatcttgtggaaaggacgaaacaccgttagctataggctaataagatagttgtgtcaagtgcttcggagacctaacacgtctccagtcacaacggctaaaaatagcca

SEQ ID NO: 162 - DNA, 3364 bp, synthetic construct
  misc_feature 1..3364: note = plasmid including the sequence for B-Gen.1 human albumin target 40
  source 1..3364: mol_type = other DNA
gcacccaagaatactattttaaaaattttttttgttttcaacaccggtaccgcgttacaatgataagtcgactgaataagtgaactcgagatcagcctcgactgtgccttctagttgccagccatctgttgtttgcccctcccccgtgccttccttgaccctggaaggtgccactcccactgtcctttcctaataaaatgaggaaattgcatccccacttcagaagttcctatactttctagtgaatgagtgagctaactcacattaattgcgttgcgctcactgcccgctttccagtcgggaaacctgtcgtgccagctgcattaatgaatcggccaacgcgcggggagaggcggtttgcgtattgggcgctcttgcgcttcctcgctcactgactcgctgcgctcggtcgttcggctgcggcgagcggtatcagctcactcaaaggcggtaatacggttatccacagaatcaggggataacgcaggaaagaacatgtgagcaaaaggccagcaaaaggccaggaaccgtaaaaaggccgcgttgctggcgtttttccataggctccgcccccctgacgagcatcacaaaaatcgacgctcaagtcagaggtggcgaaacccgacaggactataaagataccaggcgtttccccctggaagctccctcgtgcgctctcctgttccgaccctgccgcttaccggatacctgtccgcctttctcccttcgggaagcgtggcgctttctcatagctcacgctgtaggtatctcagttcggtgtaggtcgttcgctccaagctgggctgtgtgcacgaaccccccgttcagcccgaccgctgcgccttatccggtaactatcgtcttgagtccaacccggtaagacacgacttatcgccactggcagcagccactggtaacaggattagcagagcgaggtatgtaggcggtgctacagagttcttgaagtggtggcctaactacggctacactagaagaacagtatttggtatctgcgctctgctgaagccagttaccttcggaaaaagagttggtagctcttgatccggcaaacaaaccaccgctggtagcggtggtttttttgtttgcaagcagcagattacgcgcagaaaaaaaggatctcaagaagatcctttgatcttttctacggggtctgacgctcagtggaacgaaaactcacgttaagggattttggtcatgagattatcaaaaaggatcttcacctagatccttttaaattaaaaatgaagttttaaatcaatctaaagtatatatgagtaaacttggtctgacagttaccaatgcttaatcagtgaggcacctatctcagcgatctgtctatttcgttcatccatagttgcctgactccccgtcgtgtagataactacgatacgggagggcttaccatctggccccagtgctgcaatgataccgcgtgacccacgctcaccggctccagatttatcagcaataaaccagccagccggaagggccgagcgcagaagtggtcctgcaactttatccgcctccatccagtctattaattgttgccgggaagctagagtaagtagttcgccagttaatagtttgcgcaacgttgttgccattgctacaggcatcgtggtgtcacgctcgtcgtttggtatggcttcattcagctccggttcccaacgatcaaggcgagttacatgatcccccatgttgtgcaaaaaagcggttagctccttcggtcctccgatcgttgtcagaagtaagttggccgcagtgttatcactcatggttatggcagcactgcataattctcttactgtcatgccatccgtaagatgcttttctgtgactggtgagtactcaaccaagtcattctgagaatagtgtatgcggcgaccgagttgctcttgcccggcgtcaatacgggataataccgcgccacatagcagaactttaaaagtgctcatcattggaaaacgttcttcggggcgaaaactctcaaggatcttaccgctgttgagatccagttcgatgtaacccactcgtgcacccaactgatcttcagcatcttttactttcaccagcgtttctgggtgagcaaaaacaggaaggcaaaatgccgcaaaaaagggaataagggcgacacggaaatgttgaatactcatactcttcctttttcaatattattgaagcatttatcagggttattgtctcatgagcggatacatatttgaatgtatttagaaaaataaacaaataggggttccgcgcatatttccccgaaaagtgccacctgacgtcgacggatcgggagatctcccgatcccctatggtgcactctcagtacaatctgctctgatgccgcatagttaagccagtatctgctccctgcttgtgtgttggaggtcgctgagtagtgcgcgagcaaaatttaagctacaacaaggcaaggcttgaccgagcaaacaaactctttctgtgttgtaaaacgacggccagtcttaagctcgggccccctgggcggttctgataacgagtaatcgttaatccgcaaataacgtaaaaacccgcttcggcgggtttttttatggggggagtttagggaaagagcatttgtcagaatatttaagggcgcctgtcactttgcttgatatatgagaattatttaaccttataaatgagaaaaaagcaacgcactttaaataagatacgttgctttttcgattgatgaacacctataattaaactattcatctattatttatgattttttgtatatacaatatttctagtttgttaaagagaattaagaaaataaatctcgaaaataataaagggaaaatcagtttttgatatcaaaattatacatgtcaacgataatacaaaatataatacaaactataagatgttatcagtatttattatgcatttagaataaattttgtgtcgcccttattcgactcactatagaagttcctattctctagaaagtagaggaacttcacttcattttgctagcgtgtgagggcctatttcccatgattccttcatatttgcatatacgatacaaggctgttagagagataattggaattaatttgactgtaaacacaaagatattagtacaaaatacgtgacgtagaaagtaataatttcttgggtagtttgcagttttaaaattatgttttaaaatggactatcatatgcttaccgtaacttgaaagtatttcgatttcttggctttatatatcttgtggaaaggacgaaacaccgttagctataggctaataagatagttgtgtcaagtgcttcggagacctaacacgtctccagtcacaacggctaaaaatagcca

SEQ ID NO: 163 - DNA, 3364 bp, synthetic construct
  misc_feature 1..3364: note = plasmid including the sequence for B-Gen.1 human albumin target 41
  source 1..3364: mol_type = other DNA
gcacaattattcttctgtttaaaggcattttttgttttcaacaccggtaccgcgttacaatgataagtcgactgaataagtgaactcgagatcagcctcgactgtgccttctagttgccagccatctgttgtttgcccctcccccgtgccttccttgaccctggaaggtgccactcccactgtcctttcctaataaaatgaggaaattgcatccccacttcagaagttcctatactttctagtgaatgagtgagctaactcacattaattgcgttgcgctcactgcccgctttccagtcgggaaacctgtcgtgccagctgcattaatgaatcggccaacgcgcggggagaggcggtttgcgtattgggcgctcttgcgcttcctcgctcactgactcgctgcgctcggtcgttcggctgcggcgagcggtatcagctcactcaaaggcggtaatacggttatccacagaatcaggggataacgcaggaaagaacatgtgagcaaaaggccagcaaaaggccaggaaccgtaaaaaggccgcgttgctggcgtttttccataggctccgcccccctgacgagcatcacaaaaatcgacgctcaagtcagaggtggcgaaacccgacaggactataaagataccaggcgtttccccctggaagctccctcgtgcgctctcctgttccgaccctgccgcttaccggatacctgtccgcctttctcccttcgggaagcgtggcgctttctcatagctcacgctgtaggtatctcagttcggtgtaggtcgttcgctccaagctgggctgtgtgcacgaaccccccgttcagcccgaccgctgcgccttatccggtaactatcgtcttgagtccaacccggtaagacacgacttatcgccactggcagcagccactggtaacaggattagcagagcgaggtatgtaggcggtgctacagagttcttgaagtggtggcctaactacggctacactagaagaacagtatttggtatctgcgctctgctgaagccagttaccttcggaaaaagagttggtagctcttgatccggcaaacaaaccaccgctggtagcggtggtttttttgtttgcaagcagcagattacgcgcagaaaaaaaggatctcaagaagatcctttgatcttttctacggggtctgacgctcagtggaacgaaaactcacgttaagggattttggtcatgagattatcaaaaaggatcttcacctagatccttttaaattaaaaatgaagttttaaatcaatctaaagtatatatgagtaaacttggtctgacagttaccaatgcttaatcagtgaggcacctatctcagcgatctgtctatttcgttcatccatagttgcctgactccccgtcgtgtagataactacgatacgggagggcttaccatctggccccagtgctgcaatgataccgcgtgacccacgctcaccggctccagatttatcagcaataaaccagccagccggaagggccgagcgcagaagtggtcctgcaactttatccgcctccatccagtctattaattgttgccgggaagctagagtaagtagttcgccagttaatagtttgcgcaacgttgttgccattgctacaggcatcgtggtgtcacgctcgtcgtttggtatggcttcattcagctccggttcccaacgatcaaggcgagttacatgatcccccatgttgtgcaaaaaagcggttagctccttcggtcctccgatcgttgtcagaagtaagttggccgcagtgttatcactcatggttatggcagcactgcataattctcttactgtcatgccatccgtaagatgcttttctgtgactggtgagtactcaaccaagtcattctgagaatagtgtatgcggcgaccgagttgctcttgcccggcgtcaatacgggataataccgcgccacatagcagaactttaaaagtgctcatcattggaaaacgttcttcggggcgaaaactctcaaggatcttaccgctgttgagatccagttcgatgtaacccactcgtgcacccaactgatcttcagcatcttttactttcaccagcgtttctgggtgagcaaaaacaggaaggcaaaatgccgcaaaaaagggaataagggcgacacggaaatgttgaatactcatactcttcctttttcaatattattgaagcatttatcagggttattgtctcatgagcggatacatatttgaatgtatttagaaaaataaacaaataggggttccgcgcatatttccccgaaaagtgccacctgacgtcgacggatcgggagatctcccgatcccctatggtgcactctcagtacaatctgctctgatgccgcatagttaagccagtatctgctccctgcttgtgtgttggaggtcgctgagtagtgcgcgagcaaaatttaagctacaacaaggcaaggcttgaccgagcaaacaaactctttctgtgttgtaaaacgacggccagtcttaagctcgggccccctgggcggttctgataacgagtaatcgttaatccgcaaataacgtaaaaacccgcttcggcgggtttttttatggggggagtttagggaaagagcatttgtcagaatatttaagggcgcctgtcactttgcttgatatatgagaattatttaaccttataaatgagaaaaaagcaacgcactttaaataagatacgttgctttttcgattgatgaacacctataattaaactattcatctattatttatgattttttgtatatacaatatttctagtttgttaaagagaattaagaaaataaatctcgaaaataataaagggaaaatcagtttttgatatcaaaattatacatgtcaacgataatacaaaatataatacaaactataagatgttatcagtatttattatgcatttagaataaattttgtgtcgcccttattcgactcactatagaagttcctattctctagaaagtagaggaacttcacttcattttgctagcgtgtgagggcctatttcccatgattccttcatatttgcatatacgatacaaggctgttagagagataattggaattaatttgactgtaaacacaaagatattagtacaaaatacgtgacgtagaaagtaataatttcttgggtagtttgcagttttaaaattatgttttaaaatggactatcatatgcttaccgtaacttgaaagtatttcgatttcttggctttatatatcttgtggaaaggacgaaacaccgttagctataggctaataagatagttgtgtcaagtgcttcggagacctaacacgtctccagtcacaacggctaaaaatagcca

SEQ ID NO: 164 - DNA, 3364 bp, synthetic construct
  misc_feature 1..3364: note = plasmid including the sequence for B-Gen.1 human albumin target 42
  source 1..3364: mol_type = other DNA
gcacaattaccaagaatactattttaattttttgttttcaacaccggtaccgcgttacaatgataagtcgactgaataagtgaactcgagatcagcctcgactgtgccttctagttgccagccatctgttgtttgcccctcccccgtgccttccttgaccctggaaggtgccactcccactgtcctttcctaataaaatgaggaaattgcatccccacttcagaagttcctatactttctagtgaatgagtgagctaactcacattaattgcgttgcgctcactgcccgctttccagtcgggaaacctgtcgtgccagctgcattaatgaatcggccaacgcgcggggagaggcggtttgcgtattgggcgctcttgcgcttcctcgctcactgactcgctgcgctcggtcgttcggctgcggcgagcggtatcagctcactcaaaggcggtaatacggttatccacagaatcaggggataacgcaggaaagaacatgtgagcaaaaggccagcaaaaggccaggaaccgtaaaaaggccgcgttgctggcgtttttccataggctccgcccccctgacgagcatcacaaaaatcgacgctcaagtcagaggtggcgaaacccgacaggactataaagataccaggcgtttccccctggaagctccctcgtgcgctctcctgttccgaccctgccgcttaccggatacctgtccgcctttctcccttcgggaagcgtggcgctttctcatagctcacgctgtaggtatctcagttcggtgtaggtcgttcgctccaagctgggctgtgtgcacgaaccccccgttcagcccgaccgctgcgccttatccggtaactatcgtcttgagtccaacccggtaagacacgacttatcgccactggcagcagccactggtaacaggattagcagagcgaggtatgtaggcggtgctacagagttcttgaagtggtggcctaactacggctacactagaagaacagtatttggtatctgcgctctgctgaagccagttaccttcggaaaaagagttggtagctcttgatccggcaaacaaaccaccgctggtagcggtggtttttttgtttgcaagcagcagattacgcgcagaaaaaaaggatctcaagaagatcctttgatcttttctacggggtctgacgctcagtggaacgaaaactcacgttaagggattttggtcatgagattatcaaaaaggatcttcacctagatccttttaaattaaaaatgaagttttaaatcaatctaaagtatatatgagtaaacttggtctgacagttaccaatgcttaatcagtgaggcacctatctcagcgatctgtctatttcgttcatccatagttgcctgactccccgtcgtgtagataactacgatacgggagggcttaccatctggccccagtgctgcaatgataccgcgtgacccacgctcaccggctccagatttatcagcaataaaccagccagccggaagggccgagcgcagaagtggtcctgcaactttatccgcctccatccagtctattaattgttgccgggaagctagagtaagtagttcgccagttaatagtttgcgcaacgttgttgccattgctacaggcatcgtggtgtcacgctcgtcgtttggtatggcttcattcagctccggttcccaacgatcaaggcgagttacatgatcccccatgttgtgcaaaaaagcggttagctccttcggtcctccgatcgttgtcagaagtaagttggccgcagtgttatcactcatggttatggcagcactgcataattctcttactgtcatgccatccgtaagatgcttttctgtgactggtgagtactcaaccaagtcattctgagaatagtgtatgcggcgaccgagttgctcttgcccggcgtcaatacgggataataccgcgccacatagcagaactttaaaagtgctcatcattggaaaacgttcttcggggcgaaaactctcaaggatcttaccgctgttgagatccagttcgatgtaacccactcgtgcacccaactgatcttcagcatcttttactttcaccagcgtttctgggtgagcaaaaacaggaaggcaaaatgccgcaaaaaagggaataagggcgacacggaaatgttgaatactcatactcttcctttttcaatattattgaagcatttatcagggttattgtctcatgagcggatacatatttgaatgtatttagaaaaataaacaaataggggttccgcgcatatttccccgaaaagtgccacctgacgtcgacggatcgggagatctcccgatcccctatggtgcactctcagtacaatctgctctgatgccgcatagttaagccagtatctgctccctgcttgtgtgttggaggtcgctgagtagtgcgcgagcaaaatttaagctacaacaaggcaaggcttgaccgagcaaacaaactctttctgtgttgtaaaacgacggccagtcttaagctcgggccccctgggcggttctgataacgagtaatcgttaatccgcaaataacgtaaaaacccgcttcggcgggtttttttatggggggagtttagggaaagagcatttgtcagaatatttaagggcgcctgtcactttgcttgatatatgagaattatttaaccttataaatgagaaaaaagcaacgcactttaaataagatacgttgctttttcgattgatgaacacctataattaaactattcatctattatttatgattttttgtatatacaatatttctagtttgttaaagagaattaagaaaataaatctcgaaaataataaagggaaaatcagtttttgatatcaaaattatacatgtcaacgataatacaaaatataatacaaactataagatgttatcagtatttattatgcatttagaataaattttgtgtcgcccttattcgactcactatagaagttcctattctctagaaagtagaggaacttcacttcattttgctagcgtgtgagggcctatttcccatgattccttcatatttgcatatacgatacaaggctgttagagagataattggaattaatttgactgtaaacacaaagatattagtacaaaatacgtgacgtagaaagtaataatttcttgggtagtttgcagttttaaaattatgttttaaaatggactatcatatgcttaccgtaacttgaaagtatttcgatttcttggctttatatatcttgtggaaaggacgaaacaccgttagctataggctaataagatagttgtgtcaagtgcttcggagacctaacacgtctccagtcacaacggctaaaaatagcca

SEQ ID NO: 165 - DNA, 3364 bp, synthetic construct
  misc_feature 1..3364: note = plasmid including the sequence for B-Gen.1 human albumin target 43
  source 1..3364: mol_type = other DNA
gcacttcttctgtttaaaggcagaagattttttgttttcaacaccggtaccgcgttacaatgataagtcgactgaataagtgaactcgagatcagcctcgactgtgccttctagttgccagccatctgttgtttgcccctcccccgtgccttccttgaccctggaaggtgccactcccactgtcctttcctaataaaatgaggaaattgcatccccacttcagaagttcctatactttctagtgaatgagtgagctaactcacattaattgcgttgcgctcactgcccgctttccagtcgggaaacctgtcgtgccagctgcattaatgaatcggccaacgcgcggggagaggcggtttgcgtattgggcgctcttgcgcttcctcgctcactgactcgctgcgctcggtcgttcggctgcggcgagcggtatcagctcactcaaaggcggtaatacggttatccacagaatcaggggataacgcaggaaagaacatgtgagcaaaaggccagcaaaaggccaggaaccgtaaaaaggccgcgttgctggcgtttttccataggctccgcccccctgacgagcatcacaaaaatcgacgctcaagtcagaggtggcgaaacccgacaggactataaagataccaggcgtttccccctggaagctccctcgtgcgctctcctgttccgaccctgccgcttaccggatacctgtccgcctttctcccttcgggaagcgtggcgctttctcatagctcacgctgtaggtatctcagttcggtgtaggtcgttcgctccaagctgggctgtgtgcacgaaccccccgttcagcccgaccgctgcgccttatccggtaactatcgtcttgagtccaacccggtaagacacgacttatcgccactggcagcagccactggtaacaggattagcagagcgaggtatgtaggcggtgctacagagttcttgaagtggtggcctaactacggctacactagaagaacagtatttggtatctgcgctctgctgaagccagttaccttcggaaaaagagttggtagctcttgatccggcaaacaaaccaccgctggtagcggtggtttttttgtttgcaagcagcagattacgcgcagaaaaaaaggatctcaagaagatcctttgatcttttctacggggtctgacgctcagtggaacgaaaactcacgttaagggattttggtcatgagattatcaaaaaggatcttcacctagatccttttaaattaaaaatgaagttttaaatcaatctaaagtatatatgagtaaacttggtctgacagttaccaatgcttaatcagtgaggcacctatctcagcgatctgtctatttcgttcatccatagttgcctgactccccgtcgtgtagataactacgatacgggagggcttaccatctggccccagtgctgcaatgataccgcgtgacccacgctcaccggctccagatttatcagcaataaaccagccagccggaagggccgagcgcagaagtggtcctgcaactttatccgcctccatccagtctattaattgttgccgggaagctagagtaagtagttcgccagttaatagtttgcgcaacgttgttgccattgctacaggcatcgtggtgtcacgctcgtcgtttggtatggcttcattcagctccggttcccaacgatcaaggcgagttacatgatcccccatgttgtgcaaaaaagcggttagctccttcggtcctccgatcgttgtcagaagtaagttggccgcagtgttatcactcatggttatggcagcactgcataattctcttactgtcatgccatccgtaagatgcttttctgtgactggtgagtactcaaccaagtcattctgagaatagtgtatgcggcgaccgagttgctcttgcccggcgtcaatacgggataataccgcgccacatagcagaactttaaaagtgctcatcattggaaaacgttcttcggggcgaaaactctcaaggatcttaccgctgttgagatccagttcgatgtaacccactcgtgcacccaactgatcttcagcatcttttactttcaccagcgtttctgggtgagcaaaaacaggaaggcaaaatgccgcaaaaaagggaataagggcgacacggaaatgttgaatactcatactcttcctttttcaatattattgaagcatttatcagggttattgtctcatgagcggatacatatttgaatgtatttagaaaaataaacaaataggggttccgcgcatatttccccgaaaagtgccacctgacgtcgacggatcgggagatctcccgatcccctatggtgcactctcagtacaatctgctctgatgccgcatagttaagccagtatctgctccctgcttgtgtgttggaggtcgctgagtagtgcgcgagcaaaatttaagctacaacaaggcaaggcttgaccgagcaaacaaactctttctgtgttgtaaaacgacggccagtcttaagctcgggccccctgggcggttctgataacgagtaatcgttaatccgcaaataacgtaaaaacccgcttcggcgggtttttttatggggggagtttagggaaagagcatttgtcagaatatttaagggcgcctgtcactttgcttgatatatgagaattatttaaccttataaatgagaaaaaagcaacgcactttaaataagatacgttgctttttcgattgatgaacacctataattaaactattcatctattatttatgattttttgtatatacaatatttctagtttgttaaagagaattaagaaaataaatctcgaaaataataaagggaaaatcagtttttgatatcaaaattatacatgtcaacgataatacaaaatataatacaaactataagatgttatcagtatttattatgcatttagaataaattttgtgtcgcccttattcgactcactatagaagttcctattctctagaaagtagaggaacttcacttcattttgctagcgtgtgagggcctatttcccatgattccttcatatttgcatatacgatacaaggctgttagagagataattggaattaatttgactgtaaacacaaagatattagtacaaaatacgtgacgtagaaagtaataatttcttgggtagtttgcagttttaaaattatgttttaaaatggactatcatatgcttaccgtaacttgaaagtatttcgatttcttggctttatatatcttgtggaaaggacgaaacaccgttagctataggctaataagatagttgtgtcaagtgcttcggagacctaacacgtctccagtcacaacggctaaaaatagcca

SEQ ID NO: 166 - DNA, 3364 bp, synthetic construct
  misc_feature 1..3364: note = plasmid including the sequence for B-Gen.1 human albumin target 44
  source 1..3364: mol_type = other DNA
gcacttctgtttaaaggcagaagaaatttttttgttttcaacaccggtaccgcgttacaatgataagtcgactgaataagtgaactcgagatcagcctcgactgtgccttctagttgccagccatctgttgtttgcccctcccccgtgccttccttgaccctggaaggtgccactcccactgtcctttcctaataaaatgaggaaattgcatccccacttcagaagttcctatactttctagtgaatgagtgagctaactcacattaattgcgttgcgctcactgcccgctttccagtcgggaaacctgtcgtgccagctgcattaatgaatcggccaacgcgcggggagaggcggtttgcgtattgggcgctcttgcgcttcctcgctcactgactcgctgcgctcggtcgttcggctgcggcgagcggtatcagctcactcaaaggcggtaatacggttatccacagaatcaggggataacgcaggaaagaacatgtgagcaaaaggccagcaaaaggccaggaaccgtaaaaaggccgcgttgctggcgtttttccataggctccgcccccctgacgagcatcacaaaaatcgacgctcaagtcagaggtggcgaaacccgacaggactataaagataccaggcgtttccccctggaagctccctcgtgcgctctcctgttccgaccctgccgcttaccggatacctgtccgcctttctcccttcgggaagcgtggcgctttctcatagctcacgctgtaggtatctcagttcggtgtaggtcgttcgctccaagctgggctgtgtgcacgaaccccccgttcagcccgaccgctgcgccttatccggtaactatcgtcttgagtccaacccggtaagacacgacttatcgccactggcagcagccactggtaacaggattagcagagcgaggtatgtaggcggtgctacagagttcttgaagtggtggcctaactacggctacactagaagaacagtatttggtatctgcgctctgctgaagccagttaccttcggaaaaagagttggtagctcttgatccggcaaacaaaccaccgctggtagcggtggtttttttgtttgcaagcagcagattacgcgcagaaaaaaaggatctcaagaagatcctttgatcttttctacggggtctgacgctcagtggaacgaaaactcacgttaagggattttggtcatgagattatcaaaaaggatcttcacctagatccttttaaattaaaaatgaagttttaaatcaatctaaagtatatatgagtaaacttggtctgacagttaccaatgcttaatcagtgaggcacctatctcagcgatctgtctatttcgttcatccatagttgcctgactccccgtcgtgtagataactacgatacgggagggcttaccatctggccccagtgctgcaatgataccgcgtgacccacgctcaccggctccagatttatcagcaataaaccagccagccggaagggccgagcgcagaagtggtcctgcaactttatccgcctccatccagtctattaattgttgccgggaagctagagtaagtagttcgccagttaatagtttgcgcaacgttgttgccattgctacaggcatcgtggtgtcacgctcgtcgtttggtatggcttcattcagctccggttcccaacgatcaaggcgagttacatgatcccccatgttgtgcaaaaaagcggttagctccttcggtcctccgatcgttgtcagaagtaagttggccgcagtgttatcactcatggttatggcagcactgcataattctcttactgtcatgccatccgtaagatgcttttctgtgactggtgagtactcaaccaagtcattctgagaatagtgtatgcggcgaccgagttgctcttgcccggcgtcaatacgggataataccgcgccacatagcagaactttaaaagtgctcatcattggaaaacgttcttcggggcgaaaactctcaaggatcttaccgctgttgagatccagttcgatgtaacccactcgtgcacccaactgatcttcagcatcttttactttcaccagcgtttctgggtgagcaaaaacaggaaggcaaaatgccgcaaaaaagggaataagggcgacacggaaatgttgaatactcatactcttcctttttcaatattattgaagcatttatcagggttattgtctcatgagcggatacatatttgaatgtatttagaaaaataaacaaataggggttccgcgcatatttccccgaaaagtgccacctgacgtcgacggatcgggagatctcccgatcccctatggtgcactctcagtacaatctgctctgatgccgcatagttaagccagtatctgctccctgcttgtgtgttggaggtcgctgagtagtgcgcgagcaaaatttaagctacaacaaggcaaggcttgaccgagcaaacaaactctttctgtgttgtaaaacgacggccagtcttaagctcgggccccctgggcggttctgataacgagtaatcgttaatccgcaaataacgtaaaaacccgcttcggcgggtttttttatggggggagtttagggaaagagcatttgtcagaatatttaagggcgcctgtcactttgcttgatatatgagaattatttaaccttataaatgagaaaaaagcaacgcactttaaataagatacgttgctttttcgattgatgaacacctataattaaactattcatctattatttatgattttttgtatatacaatatttctagtttgttaaagagaattaagaaaataaatctcgaaaataataaagggaaaatcagtttttgatatcaaaattatacatgtcaacgataatacaaaatataatacaaactataagatgttatcagtatttattatgcatttagaataaattttgtgtcgcccttattcgactcactatagaagttcctattctctagaaagtagaggaacttcacttcattttgctagcgtgtgagggcctatttcccatgattccttcatatttgcatatacgatacaaggctgttagagagataattggaattaatttgactgtaaacacaaagatattagtacaaaatacgtgacgtagaaagtaataatttcttgggtagtttgcagttttaaaattatgttttaaaatggactatcatatgcttaccgtaacttgaaagtatttcgatttcttggctttatatatcttgtggaaaggacgaaacaccgttagctataggctaataagatagttgtgtcaagtgcttcggagacctaacacgtctccagtcacaacggctaaaaatagcca

SEQ ID NO: 167 - DNA, 3364 bp, synthetic construct
  misc_feature 1..3364: note = plasmid including the sequence for B-Gen.1 human albumin target 45
  source 1..3364: mol_type = other DNA
gcaccttctgcctttaaacagaagaatttttttgttttcaacaccggtaccgcgttacaatgataagtcgactgaataagtgaactcgagatcagcctcgactgtgccttctagttgccagccatctgttgtttgcccctcccccgtgccttccttgaccctggaaggtgccactcccactgtcctttcctaataaaatgaggaaattgcatccccacttcagaagttcctatactttctagtgaatgagtgagctaactcacattaattgcgttgcgctcactgcccgctttccagtcgggaaacctgtcgtgccagctgcattaatgaatcggccaacgcgcggggagaggcggtttgcgtattgggcgctcttgcgcttcctcgctcactgactcgctgcgctcggtcgttcggctgcggcgagcggtatcagctcactcaaaggcggtaatacggttatccacagaatcaggggataacgcaggaaagaacatgtgagcaaaaggccagcaaaaggccaggaaccgtaaaaaggccgcgttgctggcgtttttccataggctccgcccccctgacgagcatcacaaaaatcgacgctcaagtcagaggtggcgaaacccgacaggactataaagataccaggcgtttccccctggaagctccctcgtgcgctctcctgttccgaccctgccgcttaccggatacctgtccgcctttctcccttcgggaagcgtggcgctttctcatagctcacgctgtaggtatctcagttcggtgtaggtcgttcgctccaagctgggctgtgtgcacgaaccccccgttcagcccgaccgctgcgccttatccggtaactatcgtcttgagtccaacccggtaagacacgacttatcgccactggcagcagccactggtaacaggattagcagagcgaggtatgtaggcggtgctacagagttcttgaagtggtggcctaactacggctacactagaagaacagtatttggtatctgcgctctgctgaagccagttaccttcggaaaaagagttggtagctcttgatccggcaaacaaaccaccgctggtagcggtggtttttttgtttgcaagcagcagattacgcgcagaaaaaaaggatctcaagaagatcctttgatcttttctacggggtctgacgctcagtggaacgaaaactcacgttaagggattttggtcatgagattatcaaaaaggatcttcacctagatccttttaaattaaaaatgaagttttaaatcaatctaaagtatatatgagtaaacttggtctgacagttaccaatgcttaatcagtgaggcacctatctcagcgatctgtctatttcgttcatccatagttgcctgactccccgtcgtgtagataactacgatacgggagggcttaccatctggccccagtgctgcaatgataccgcgtgacccacgctcaccggctccagatttatcagcaataaaccagccagccggaagggccgagcgcagaagtggtcctgcaactttatccgcctccatccagtctattaattgttgccgggaagctagagtaagtagttcgccagttaatagtttgcgcaacgttgttgccattgctacaggcatcgtggtgtcacgctcgtcgtttggtatggcttcattcagctccggttcccaacgatcaaggcgagttacatgatcccccatgttgtgcaaaaaagcggttagctccttcggtcctccgatcgttgtcagaagtaagttggccgcagtgttatcactcatggttatggcagcactgcataattctcttactgtcatgccatccgtaagatgcttttctgtgactggtgagtactcaaccaagtcattctgagaatagtgtatgcggcgaccgagttgctcttgcccggcgtcaatacgggataataccgcgccacatagcagaactttaaaagtgctcatcattggaaaacgttcttcggggcgaaaactctcaaggatcttaccgctgttgagatccagttcgatgtaacccactcgtgcacccaactgatcttcagcatcttttactttcaccagcgtttctgggtgagcaaaaacaggaaggcaaaatgccgcaaaaaagggaataagggcgacacggaaatgttgaatactcatactcttcctttttcaatattattgaagcatttatcagggttattgtctcatgagcggatacatatttgaatgtatttagaaaaataaacaaataggggttccgcgcatatttccccgaaaagtgccacctgacgtcgacggatcgggagatctcccgatcccctatggtgcactctcagtacaatctgctctgatgccgcatagttaagccagtatctgctccctgcttgtgtgttggaggtcgctgagtagtgcgcgagcaaaatttaagctacaacaaggcaaggcttgaccgagcaaacaaactctttctgtgttgtaaaacgacggccagtcttaagctcgggccccctgggcggttctgataacgagtaatcgttaatccgcaaataacgtaaaaacccgcttcggcgggtttttttatggggggagtttagggaaagagcatttgtcagaatatttaagggcgcctgtcactttgcttgatatatgagaattatttaaccttataaatgagaaaaaagcaacgcactttaaataagatacgttgctttttcgattgatgaacacctataattaaactattcatctattatttatgattttttgtatatacaatatttctagtttgttaaagagaattaagaaaataaatctcgaaaataataaagggaaaatcagtttttgatatcaaaattatacatgtcaacgataatacaaaatataatacaaactataagatgttatcagtatttattatgcatttagaataaattttgtgtcgcccttattcgactcactatagaagttcctattctctagaaagtagaggaacttcacttcattttgctagcgtgtgagggcctatttcccatgattccttcatatttgcatatacgatacaaggctgttagagagataattggaattaatttgactgtaaacacaaagatattagtacaaaatacgtgacgtagaaagtaataatttcttgggtagtttgcagttttaaaattatgttttaaaatggactatcatatgcttaccgtaacttgaaagtatttcgatttcttggctttatatatcttgtggaaaggacgaaacaccgttagctataggctaataagatagttgtgtcaagtgcttcggagacctaacacgtctccagtcacaacggctaaaaatagcca

SEQ ID NO: 168 - DNA, 3364 bp, synthetic construct
  misc_feature 1..3364: note = plasmid including the sequence for B-Gen.1 human albumin target 46
  source 1..3364: mol_type = other DNA
gcactttcttctgcctttaaacagaagttttttgttttcaacaccggtaccgcgttacaatgataagtcgactgaataagtgaactcgagatcagcctcgactgtgccttctagttgccagccatctgttgtttgcccctcccccgtgccttccttgaccctggaaggtgccactcccactgtcctttcctaataaaatgaggaaattgcatccccacttcagaagttcctatactttctagtgaatgagtgagctaactcacattaattgcgttgcgctcactgcccgctttccagtcgggaaacctgtcgtgccagctgcattaatgaatcggccaacgcgcggggagaggcggtttgcgtattgggcgctcttgcgcttcctcgctcactgactcgctgcgctcggtcgttcggctgcggcgagcggtatcagctcactcaaaggcggtaatacggttatccacagaatcaggggataacgcaggaaagaacatgtgagcaaaaggccagcaaaaggccaggaaccgtaaaaaggccgcgttgctggcgtttttccataggctccgcccccctgacgagcatcacaaaaatcgacgctcaagtcagaggtggcgaaacccgacaggactataaagataccaggcgtttccccctggaagctccctcgtgcgctctcctgttccgaccctgccgcttaccggatacctgtccgcctttctcccttcgggaagcgtggcgctttctcatagctcacgctgtaggtatctcagttcggtgtaggtcgttcgctccaagctgggctgtgtgcacgaaccccccgttcagcccgaccgctgcgccttatccggtaactatcgtcttgagtccaacccggtaagacacgacttatcgccactggcagcagccactggtaacaggattagcagagcgaggtatgtaggcggtgctacagagttcttgaagtggtggcctaactacggctacactagaagaacagtatttggtatctgcgctctgctgaagccagttaccttcggaaaaagagttggtagctcttgatccggcaaacaaaccaccgctggtagcggtggtttttttgtttgcaagcagcagattacgcgcagaaaaaaaggatctcaagaagatcctttgatcttttctacggggtctgacgctcagtggaacgaaaactcacgttaagggattttggtcatgagattatcaaaaaggatcttcacctagatccttttaaattaaaaatgaagttttaaatcaatctaaagtatatatgagtaaacttggtctgacagttaccaatgcttaatcagtgaggcacctatctcagcgatctgtctatttcgttcatccatagttgcctgactccccgtcgtgtagataactacgatacgggagggcttaccatctggccccagtgctgcaatgataccgcgtgacccacgctcaccggctccagatttatcagcaataaaccagccagccggaagggccgagcgcagaagtggtcctgcaactttatccgcctccatccagtctattaattgttgccgggaagctagagtaagtagttcgccagttaatagtttgcgcaacgttgttgccattgctacaggcatcgtggtgtcacgctcgtcgtttggtatggcttcattcagctccggttcccaacgatcaaggcgagttacatgatcccccatgttgtgcaaaaaagcggttagctccttcggtcctccgatcgttgtcagaagtaagttggccgcagtgttatcactcatggttatggcagcactgcataattctcttactgtcatgccatccgtaagatgcttttctgtgactggtgagtactcaaccaagtcattctgagaatagtgtatgcggcgaccgagttgctcttgcccggcgtcaatacgggataataccgcgccacatagcagaactttaaaagtgctcatcattggaaaacgttcttcggggcgaaaactctcaaggatcttaccgctgttgagatccagttcgatgtaacccactcgtgcacccaactgatcttcagcatcttttactttcaccagcgtttctgggtgagcaaaaacaggaaggcaaaatgccgcaaaaaagggaataagggcgacacggaaatgttgaatactcatactcttcctttttcaatattattgaagcatttatcagggttattgtctcatgagcggatacatatttgaatgtatttagaaaaataaacaaataggggttccgcgcatatttccccgaaaagtgccacctgacgtcgacggatcgggagatctcccgatcccctatggtgcactctcagtacaatctgctctgatgccgcatagttaagccagtatctgctccctgcttgtgtgttggaggtcgctgagtagtgcgcgagcaaaatttaagctacaacaaggcaaggcttgaccgagcaaacaaactctttctgtgttgtaaaacgacggccagtcttaagctcgggccccctgggcggttctgataacgagtaatcgttaatccgcaaataacgtaaaaacccgcttcggcgggtttttttatggggggagtttagggaaagagcatttgtcagaatatttaagggcgcctgtcactttgcttgatatatgagaattatttaaccttataaatgagaaaaaagcaacgcactttaaataagatacgttgctttttcgattgatgaacacctataattaaactattcatctattatttatgattttttgtatatacaatatttctagtttgttaaagagaattaagaaaataaatctcgaaaataataaagggaaaatcagtttttgatatcaaaattatacatgtcaacgataatacaaaatataatacaaactataagatgttatcagtatttattatgcatttagaataaattttgtgtcgcccttattcgactcactatagaagttcctattctctagaaagtagaggaacttcacttcattttgctagcgtgtgagggcctatttcccatgattccttcatatttgcatatacgatacaaggctgttagagagataattggaattaatttgactgtaaacacaaagatattagtacaaaatacgtgacgtagaaagtaataatttcttgggtagtttgcagttttaaaattatgttttaaaatggactatcatatgcttaccgtaacttgaaagtatttcgatttcttggctttatatatcttgtggaaaggacgaaacaccgttagctataggctaataagatagttgtgtcaagtgcttcggagacctaacacgtctccagtcacaacggctaaaaatagcca

SEQ ID NO: 169 - DNA, 3364 bp, synthetic construct
  misc_feature 1..3364: note = plasmid including the sequence for B-Gen.1 human albumin target 47
  source 1..3364: mol_type = other DNA
gcacaacatcatcctgagtttttctgtttttttgttttcaacaccggtaccgcgttacaatgataagtcgactgaataagtgaactcgagatcagcctcgactgtgccttctagttgccagccatctgttgtttgcccctcccccgtgccttccttgaccctggaaggtgccactcccactgtcctttcctaataaaatgaggaaattgcatccccacttcagaagttcctatactttctagtgaatgagtgagctaactcacattaattgcgttgcgctcactgcccgctttccagtcgggaaacctgtcgtgccagctgcattaatgaatcggccaacgcgcggggagaggcggtttgcgtattgggcgctcttgcgcttcctcgctcactgactcgctgcgctcggtcgttcggctgcggcgagcggtatcagctcactcaaaggcggtaatacggttatccacagaatcaggggataacgcaggaaagaacatgtgagcaaaaggccagcaaaaggccaggaaccgtaaaaaggccgcgttgctggcgtttttccataggctccgcccccctgacgagcatcacaaaaatcgacgctcaagtcagaggtggcgaaacccgacaggactataaagataccaggcgtttccccctggaagctccctcgtgcgctctcctgttccgaccctgccgcttaccggatacctgtccgcctttctcccttcgggaagcgtggcgctttctcatagctcacgctgtaggtatctcagttcggtgtaggtcgttcgctccaagctgggctgtgtgcacgaaccccccgttcagcccgaccgctgcgccttatccggtaactatcgtcttgagtccaacccggtaagacacgacttatcgccactggcagcagccactggtaacaggattagcagagcgaggtatgtaggcggtgctacagagttcttgaagtggtggcctaactacggctacactagaagaacagtatttggtatctgcgctctgctgaagccagttaccttcggaaaaagagttggtagctcttgatccggcaaacaaaccaccgctggtagcggtggtttttttgtttgcaagcagcagattacgcgcagaaaaaaaggatctcaagaagatcctttgatcttttctacggggtctgacgctcagtggaacgaaaactcacgttaagggattttggtcatgagattatcaaaaaggatcttcacctagatccttttaaattaaaaatgaagttttaaatcaatctaaagtatatatgagtaaacttggtctgacagttaccaatgcttaatcagtgaggcacctatctcagcgatctgtctatttcgttcatccatagttgcctgactccccgtcgtgtagataactacgatacgggagggcttaccatctggccccagtgctgcaatgataccgcgtgacccacgctcaccggctccagatttatcagcaataaaccagccagccggaagggccgagcgcagaagtggtcctgcaactttatccgcctccatccagtctattaattgttgccgggaagctagagtaagtagttcgccagttaatagtttgcgcaacgttgttgccattgctacaggcatcgtggtgtcacgctcgtcgtttggtatggcttcattcagctccggttcccaacgatcaaggcgagttacatgatcccccatgttgtgcaaaaaagcggttagctccttcggtcctccgatcgttgtcagaagtaagttggccgcagtgttatcactcatggttatggcagcactgcataattctcttactgtcatgccatccgtaagatgcttttctgtgactggtgagtactcaaccaagtcattctgagaatagtgtatgcggcgaccgagttgctcttgcccggcgtcaatacgggataataccgcgccacatagcagaactttaaaagtgctcatcattggaaaacgttcttcggggcgaaaactctcaaggatcttaccgctgttgagatccagttcgatgtaacccactcgtgcacccaactgatcttcagcatcttttactttcaccagcgtttctgggtgagcaaaaacaggaaggcaaaatgccgcaaaaaagggaataagggcgacacggaaatgttgaatactcatactcttcctttttcaatattattgaagcatttatcagggttattgtctcatgagcggatacatatttgaatgtatttagaaaaataaacaaataggggttccgcgcatatttccccgaaaagtgccacctgacgtcgacggatcgggagatctcccgatcccctatggtgcactctcagtacaatctgctctgatgccgcatagttaagccagtatctgctccctgcttgtgtgttggaggtcgctgagtagtgcgcgagcaaaatttaagctacaacaaggcaaggcttgaccgagcaaacaaactctttctgtgttgtaaaacgacggccagtcttaagctcgggccccctgggcggttctgataacgagtaatcgttaatccgcaaataacgtaaaaacccgcttcggcgggtttttttatggggggagtttagggaaagagcatttgtcagaatatttaagggcgcctgtcactttgcttgatatatgagaattatttaaccttataaatgagaaaaaagcaacgcactttaaataagatacgttgctttttcgattgatgaacacctataattaaactattcatctattatttatgattttttgtatatacaatatttctagtttgttaaagagaattaagaaaataaatctcgaaaataataaagggaaaatcagtttttgatatcaaaattatacatgtcaacgataatacaaaatataatacaaactataagatgttatcagtatttattatgcatttagaataaattttgtgtcgcccttattcgactcactatagaagttcctattctctagaaagtagaggaacttcacttcattttgctagcgtgtgagggcctatttcccatgattccttcatatttgcatatacgatacaaggctgttagagagataattggaattaatttgactgtaaacacaaagatattagtacaaaatacgtgacgtagaaagtaataatttcttgggtagtttgcagttttaaaattatgttttaaaatggactatcatatgcttaccgtaacttgaaagtatttcgatttcttggctttatatatcttgtggaaaggacgaaacaccgttagctataggctaataagatagttgtgtcaagtgcttcggagacctaacacgtctccagtcacaacggctaaaaatagcca

SEQ ID NO: 170 - DNA, 3364 bp, synthetic construct
  misc_feature 1..3364: note = plasmid including the sequence for B-Gen.1 human albumin target 48
  source 1..3364: mol_type = other DNA
gcacctacagaaaaactcaggatgatgttttttgttttcaacaccggtaccgcgttacaatgataagtcgactgaataagtgaactcgagatcagcctcgactgtgccttctagttgccagccatctgttgtttgcccctcccccgtgccttccttgaccctggaaggtgccactcccactgtcctttcctaataaaatgaggaaattgcatccccacttcagaagttcctatactttctagtgaatgagtgagctaactcacattaattgcgttgcgctcactgcccgctttccagtcgggaaacctgtcgtgccagctgcattaatgaatcggccaacgcgcggggagaggcggtttgcgtattgggcgctcttgcgcttcctcgctcactgactcgctgcgctcggtcgttcggctgcggcgagcggtatcagctcactcaaaggcggtaatacggttatccacagaatcaggggataacgcaggaaagaacatgtgagcaaaaggccagcaaaaggccaggaaccgtaaaaaggccgcgttgctggcgtttttccataggctccgcccccctgacgagcatcacaaaaatcgacgctcaagtcagaggtggcgaaacccgacaggactataaagataccaggcgtttccccctggaagctccctcgtgcgctctcctgttccgaccctgccgcttaccggatacctgtccgcctttctcccttcgggaagcgtggcgctttctcatagctcacgctgtaggtatctcagttcggtgtaggtcgttcgctccaagctgggctgtgtgcacgaaccccccgttcagcccgaccgctgcgccttatccggtaactatcgtcttgagtccaacccggtaagacacgacttatcgccactggcagcagccactggtaacaggattagcagagcgaggtatgtaggcggtgctacagagttcttgaagtggtggcctaactacggctacactagaagaacagtatttggtatctgcgctctgctgaagccagttaccttcggaaaaagagttggtagctcttgatccggcaaacaaaccaccgctggtagcggtggtttttttgtttgcaagcagcagattacgcgcagaaaaaaaggatctcaagaagatcctttgatcttttctacggggtctgacgctcagtggaacgaaaactcacgttaagggattttggtcatgagattatcaaaaaggatcttcacctagatccttttaaattaaaaatgaagttttaaatcaatctaaagtatatatgagtaaacttggtctgacagttaccaatgcttaatcagtgaggcacctatctcagcgatctgtctatttcgttcatccatagttgcctgactccccgtcgtgtagataactacgatacgggagggcttaccatctggccccagtgctgcaatgataccgcgtgacccacgctcaccggctccagatttatcagcaataaaccagccagccggaagggccgagcgcagaagtggtcctgcaactttatccgcctccatccagtctattaattgttgccgggaagctagagtaagtagttcgccagttaatagtttgcgcaacgttgttgccattgctacaggcatcgtggtgtcacgctcgtcgtttggtatggcttcattcagctccggttcccaacgatcaaggcgagttacatgatcccccatgttgtgcaaaaaagcggttagctccttcggtcctccgatcgttgtcagaagtaagttggccgcagtgttatcactcatggttatggcagcactgcataattctcttactgtcatgccatccgtaagatgcttttctgtgactggtgagtactcaaccaagtcattctgagaatagtgtatgcggcgaccgagttgctcttgcccggcgtcaatacgggataataccgcgccacatagcagaactttaaaagtgctcatcattggaaaacgttcttcggggcgaaaactctcaaggatcttaccgctgttgagatccagttcgatgtaacccactcgtgcacccaactgatcttcagcatcttttactttcaccagcgtttctgggtgagcaaaaacaggaaggcaaaatgccgcaaaaaagggaataagggcgacacggaaatgttgaatactcatactcttcctttttcaatattattgaagcatttatcagggttattgtctcatgagcggatacatatttgaatgtatttagaaaaataaacaaataggggttccgcgcatatttccccgaaaagtgccacctgacgtcgacggatcgggagatctcccgatcccctatggtgcactctcagtacaatctgctctgatgccgcatagttaagccagtatctgctccctgcttgtgtgttggaggtcgctgagtagtgcgcgagcaaaatttaagctacaacaaggcaaggcttgaccgagcaaacaaactctttctgtgttgtaaaacgacggccagtcttaagctcgggccccctgggcggttctgataacgagtaatcgttaatccgcaaataacgtaaaaacccgcttcggcgggtttttttatggggggagtttagggaaagagcatttgtcagaatatttaagggcgcctgtcactttgcttgatatatgagaattatttaaccttataaatgagaaaaaagcaacgcactttaaataagatacgttgctttttcgattgatgaacacctataattaaactattcatctattatttatgattttttgtatatacaatatttctagtttgttaaagagaattaagaaaataaatctcgaaaataataaagggaaaatcagtttttgatatcaaaattatacatgtcaacgataatacaaaatataatacaaactataagatgttatcagtatttattatgcatttagaataaattttgtgtcgcccttattcgactcactatagaagttcctattctctagaaagtagaggaacttcacttcattttgctagcgtgtgagggcctatttcccatgattccttcatatttgcatatacgatacaaggctgttagagagataattggaattaatttgactgtaaacacaaagatattagtacaaaatacgtgacgtagaaagtaataatttcttgggtagtttgcagttttaaaattatgttttaaaatggactatcatatgcttaccgtaacttgaaagtatttcgatttcttggctttatatatcttgtggaaaggacgaaacaccgttagctataggctaataagatagttgtgtcaagtgcttcggagacctaacacgtctccagtcacaacggctaaaaatagcca

SEQ ID NO: 171 - DNA, 3364 bp, synthetic construct
  misc_feature 1..3364: note = plasmid including the sequence for B-Gen.1 human albumin target 49
  source 1..3364: mol_type = other DNA
gcacggctctgattcctacagaaaaacttttttgttttcaacaccggtaccgcgttacaatgataagtcgactgaataagtgaactcgagatcagcctcgactgtgccttctagttgccagccatctgttgtttgcccctcccccgtgccttccttgaccctggaaggtgccactcccactgtcctttcctaataaaatgaggaaattgcatccccacttcagaagttcctatactttctagtgaatgagtgagctaactcacattaattgcgttgcgctcactgcccgctttccagtcgggaaacctgtcgtgccagctgcattaatgaatcggccaacgcgcggggagaggcggtttgcgtattgggcgctcttgcgcttcctcgctcactgactcgctgcgctcggtcgttcggctgcggcgagcggtatcagctcactcaaaggcggtaatacggttatccacagaatcaggggataacgcaggaaagaacatgtgagcaaaaggccagcaaaaggccaggaaccgtaaaaaggccgcgttgctggcgtttttccataggctccgcccccctgacgagcatcacaaaaatcgacgctcaagtcagaggtggcgaaacccgacaggactataaagataccaggcgtttccccctggaagctccctcgtgcgctctcctgttccgaccctgccgcttaccggatacctgtccgcctttctcccttcgggaagcgtggcgctttctcatagctcacgctgtaggtatctcagttcggtgtaggtcgttcgctccaagctgggctgtgtgcacgaaccccccgttcagcccgaccgctgcgccttatccggtaactatcgtcttgagtccaacccggtaagacacgacttatcgccactggcagcagccactggtaacaggattagcagagcgaggtatgtaggcggtgctacagagttcttgaagtggtggcctaactacggctacactagaagaacagtatttggtatctgcgctctgctgaagccagttaccttcggaaaaagagttggtagctcttgatccggcaaacaaaccaccgctggtagcggtggtttttttgtttgcaagcagcagattacgcgcagaaaaaaaggatctcaagaagatcctttgatcttttctacggggtctgacgctcagtggaacgaaaactcacgttaagggattttggtcatgagattatcaaaaaggatcttcacctagatccttttaaattaaaaatgaagttttaaatcaatctaaagtatatatgagtaaacttggtctgacagttaccaatgcttaatcagtgaggcacctatctcagcgatctgtctatttcgttcatccatagttgcctgactccccgtcgtgtagataactacgatacgggagggcttaccatctggccccagtgctgcaatgataccgcgtgacccacgctcaccggctccagatttatcagcaataaaccagccagccggaagggccgagcgcagaagtggtcctgcaactttatccgcctccatccagtctattaattgttgccgggaagctagagtaagtagttcgccagttaatagtttgcgcaacgttgttgccattgctacaggcatcgtggtgtcacgctcgtcgtttggtatggcttcattcagctccggttcccaacgatcaaggcgagttacatgatcccccatgttgtgcaaaaaagcggttagctccttcggtcctccgatcgttgtcagaagtaagttggccgcagtgttatcactcatggttatggcagcactgcataattctcttactgtcatgccatccgtaagatgcttttctgtgactggtgagtactcaaccaagtcattctgagaatagtgtatgcggcgaccgagttgctcttgcccggcgtcaatacgggataataccgcgccacatagcagaactttaaaagtgctcatcattggaaaacgttcttcggggcgaaaactctcaaggatcttaccgctgttgagatccagttcgatgtaacccactcgtgcacccaactgatcttcagcatcttttactttcaccagcgtttctgggtgagcaaaaacaggaaggcaaaatgccgcaaaaaagggaataagggcgacacggaaatgttgaatactcatactcttcctttttcaatattattgaagcatttatcagggttattgtctcatgagcggatacatatttgaatgtatttagaaaaataaacaaataggggttccgcgcatatttccccgaaaagtgccacctgacgtcgacggatcgggagatctcccgatcccctatggtgcactctcagtacaatctgctctgatgccgcatagttaagccagtatctgctccctgcttgtgtgttggaggtcgctgagtagtgcgcgagcaaaatttaagctacaacaaggcaaggcttgaccgagcaaacaaactctttctgtgttgtaaaacgacggccagtcttaagctcgggccccctgggcggttctgataacgagtaatcgttaatccgcaaataacgtaaaaacccgcttcggcgggtttttttatggggggagtttagggaaagagcatttgtcagaatatttaagggcgcctgtcactttgcttgatatatgagaattatttaaccttataaatgagaaaaaagcaacgcactttaaataagatacgttgctttttcgattgatgaacacctataattaaactattcatctattatttatgattttttgtatatacaatatttctagtttgttaaagagaattaagaaaataaatctcgaaaataataaagggaaaatcagtttttgatatcaaaattatacatgtcaacgataatacaaaatataatacaaactataagatgttatcagtatttattatgcatttagaataaattttgtgtcgcccttattcgactcactatagaagttcctattctctagaaagtagaggaacttcacttcattttgctagcgtgtgagggcctatttcccatgattccttcatatttgcatatacgatacaaggctgttagagagataattggaattaatttgactgtaaacacaaagatattagtacaaaatacgtgacgtagaaagtaataatttcttgggtagtttgcagttttaaaattatgttttaaaatggactatcatatgcttaccgtaacttgaaagtatttcgatttcttggctttatatatcttgtggaaaggacgaaacaccgttagctataggctaataagatagttgtgtcaagtgcttcggagacctaacacgtctccagtcacaacggctaaaaatagcca

SEQ ID NO: 172 - DNA, 3364 bp, synthetic construct
  misc_feature 1..3364: note = plasmid including the sequence for B-Gen.1 human albumin target 50
  source 1..3364: mol_type = other DNA
gcactgaaacaaatgcataatctaagtttttttgttttcaacaccggtaccgcgttacaatgataagtcgactgaataagtgaactcgagatcagcctcgactgtgccttctagttgccagccatctgttgtttgcccctcccccgtgccttccttgaccctggaaggtgccactcccactgtcctttcctaataaaatgaggaaattgcatccccacttcagaagttcctatactttctagtgaatgagtgagctaactcacattaattgcgttgcgctcactgcccgctttccagtcgggaaacctgtcgtgccagctgcattaatgaatcggccaacgcgcggggagaggcggtttgcgtattgggcgctcttgcgcttcctcgctcactgactcgctgcgctcggtcgttcggctgcggcgagcggtatcagctcactcaaaggcggtaatacggttatccacagaatcaggggataacgcaggaaagaacatgtgagcaaaaggccagcaaaaggccaggaaccgtaaaaaggccgcgttgctggcgtttttccataggctccgcccccctgacgagcatcacaaaaatcgacgctcaagtcagaggtggcgaaacccgacaggactataaagataccaggcgtttccccctggaagctccctcgtgcgctctcctgttccgaccctgccgcttaccggatacctgtccgcctttctcccttcgggaagcgtggcgctttctcatagctcacgctgtaggtatctcagttcggtgtaggtcgttcgctccaagctgggctgtgtgcacgaaccccccgttcagcccgaccgctgcgccttatccggtaactatcgtcttgagtccaacccggtaagacacgacttatcgccactggcagcagccactggtaacaggattagcagagcgaggtatgtaggcggtgctacagagttcttgaagtggtggcctaactacggctacactagaagaacagtatttggtatctgcgctctgctgaagccagttaccttcggaaaaagagttggtagctcttgatccggcaaacaaaccaccgctggtagcggtggtttttttgtttgcaagcagcagattacgcgcagaaaaaaaggatctcaagaagatcctttgatcttttctacggggtctgacgctcagtggaacgaaaactcacgttaagggattttggtcatgagattatcaaaaaggatcttcacctagatccttttaaattaaaaatgaagttttaaatcaatctaaagtatatatgagtaaacttggtctgacagttaccaatgcttaatcagtgaggcacctatctcagcgatctgtctatttcgttcatccatagttgcctgactccccgtcgtgtagataactacgatacgggagggcttaccatctggccccagtgctgcaatgataccgcgtgacccacgctcaccggctccagatttatcagcaataaaccagccagccggaagggccgagcgcagaagtggtcctgcaactttatccgcctccatccagtctattaattgttgccgggaagctagagtaagtagttcgccagttaatagtttgcgcaacgttgttgccattgctacaggcatcgtggtgtcacgctcgtcgtttggtatggcttcattcagctccggttcccaacgatcaaggcgagttacatgatcccccatgttgtgcaaaaaagcggttagctccttcggtcctccgatcgttgtcagaagtaagttggccgcagtgttatcactcatggttatggcagcactgcataattctcttactgtcatgccatccgtaagatgcttttctgtgactggtgagtactcaaccaagtcattctgagaatagtgtatgcggcgaccgagttgctcttgcccggcgtcaatacgggataataccgcgccacatagcagaactttaaaagtgctcatcattggaaaacgttcttcggggcgaaaactctcaaggatcttaccgctgttgagatccagttcgatgtaacccactcgtgcacccaactgatcttcagcatcttttactttcaccagcgtttctgggtgagcaaaaacaggaaggcaaaatgccgcaaaaaagggaataagggcgacacggaaatgttgaatactcatactcttcctttttcaatattattgaagcatttatcagggttattgtctcatgagcggatacatatttgaatgtatttagaaaaataaacaaataggggttccgcgcatatttccccgaaaagtgccacctgacgtcgacggatcgggagatctcccgatcccctatggtgcactctcagtacaatctgctctgatgccgcatagttaagccagtatctgctccctgcttgtgtgttggaggtcgctgagtagtgcgcgagcaaaatttaagctacaacaaggcaaggcttgaccgagcaaacaaactctttctgtgttgtaaaacgacggccagtcttaagctcgggccccctgggcggttctgataacgagtaatcgttaatccgcaaataacgtaaaaacccgcttcggcgggtttttttatggggggagtttagggaaagagcatttgtcagaatatttaagggcgcctgtcactttgcttgatatatgagaattatttaaccttataaatgagaaaaaagcaacgcactttaaataagatacgttgctttttcgattgatgaacacctataattaaactattcatctattatttatgattttttgtatatacaatatttctagtttgttaaagagaattaagaaaataaatctcgaaaataataaagggaaaatcagtttttgatatcaaaattatacatgtcaacgataatacaaaatataatacaaactataagatgttatcagtatttattatgcatttagaataaattttgtgtcgcccttattcgactcactatagaagttcctattctctagaaagtagaggaacttcacttcattttgctagcgtgtgagggcctatttcccatgattccttcatatttgcatatacgatacaaggctgttagagagataattggaattaatttgactgtaaacacaaagatattagtacaaaatacgtgacgtagaaagtaataatttcttgggtagtttgcagttttaaaattatgttttaaaatggactatcatatgcttaccgtaacttgaaagtatttcgatttcttggctttatatatcttgtggaaaggacgaaacaccgttagctataggctaataagatagttgtgtcaagtgcttcggagacctaacacgtctccagtcacaacggctaaaaatagcca

SEQ ID NO: 173 - DNA, 3364 bp, synthetic construct
  misc_feature 1..3364: note = plasmid including the sequence for B-Gen.1 human albumin target 51
  source 1..3364: mol_type = other DNA
gcacgtttcaaaatattgggctctgatttttttgttttcaacaccggtaccgcgttacaatgataagtcgactgaataagtgaactcgagatcagcctcgactgtgccttctagttgccagccatctgttgtttgcccctcccccgtgccttccttgaccctggaaggtgccactcccactgtcctttcctaataaaatgaggaaattgcatccccacttcagaagttcctatactttctagtgaatgagtgagctaactcacattaattgcgttgcgctcactgcccgctttccagtcgggaaacctgtcgtgccagctgcattaatgaatcggccaacgcgcggggagaggcggtttgcgtattgggcgctcttgcgcttcctcgctcactgactcgctgcgctcggtcgttcggctgcggcgagcggtatcagctcactcaaaggcggtaatacggttatccacagaatcaggggataacgcaggaaagaacatgtgagcaaaaggccagcaaaaggccaggaaccgtaaaaaggccgcgttgctggcgtttttccataggctccgcccccctgacgagcatcacaaaaatcgacgctcaagtcagaggtggcgaaacccgacaggactataaagataccaggcgtttccccctggaagctccctcgtgcgctctcctgttccgaccctgccgcttaccggatacctgtccgcctttctcccttcgggaagcgtggcgctttctcatagctcacgctgtaggtatctcagttcggtgtaggtcgttcgctccaagctgggctgtgtgcacgaaccccccgttcagcccgaccgctgcgccttatccggtaactatcgtcttgagtccaacccggtaagacacgacttatcgccactggcagcagccactggtaacaggattagcagagcgaggtatgtaggcggtgctacagagttcttgaagtggtggcctaactacggctacactagaagaacagtatttggtatctgcgctctgctgaagccagttaccttcggaaaaagagttggtagctcttgatccggcaaacaaaccaccgctggtagcggtggtttttttgtttgcaagcagcagattacgcgcagaaaaaaaggatctcaagaagatcctttgatcttttctacggggtctgacgctcagtggaacgaaaactcacgttaagggattttggtcatgagattatcaaaaaggatcttcacctagatccttttaaattaaaaatgaagttttaaatcaatctaaagtatatatgagtaaacttggtctgacagttaccaatgcttaatcagtgaggcacctatctcagcgatctgtctatttcgttcatccatagttgcctgactccccgtcgtgtagataactacgatacgggagggcttaccatctggccccagtgctgcaatgataccgcgtgacccacgctcaccggctccagatttatcagcaataaaccagccagccggaagggccgagcgcagaagtggtcctgcaactttatccgcctccatccagtctattaattgttgccgggaagctagagtaagtagttcgccagttaatagtttgcgcaacgttgttgccattgctacaggcatcgtggtgtcacgctcgtcgtttggtatggcttcattcagctccggttcccaacgatcaaggcgagttacatgatcccccatgttgtgcaaaaaagcggttagctccttcggtcctccgatcgttgtcagaagtaagttggccgcagtgttatcactcatggttatggcagcactgcataattctcttactgtcatgccatccgtaagatgcttttctgtgactggtgagtactcaaccaagtcattctgagaatagtgtatgcggcgaccgagttgctcttgcccggcgtcaatacgggataataccgcgccacatagcagaactttaaaagtgctcatcattggaaaacgttcttcggggcgaaaactctcaaggatcttaccgctgttgagatccagttcgatgtaacccactcgtgcacccaactgatcttcagcatcttttactttcaccagcgtttctgggtgagcaaaaacaggaaggcaaaatgccgcaaaaaagggaataagggcgacacggaaatgttgaatactcatactcttcctttttcaatattattgaagcatttatcagggttattgtctcatgagcggatacatatttgaatgtatttagaaaaataaacaaataggggttccgcgcatatttccccgaaaagtgccacctgacgtcgacggatcgggagatctcccgatcccctatggtgcactctcagtacaatctgctctgatgccgcatagttaagccagtatctgctccctgcttgtgtgttggaggtcgctgagtagtgcgcgagcaaaatttaagctacaacaaggcaaggcttgaccgagcaaacaaactctttctgtgttgtaaaacgacggccagtcttaagctcgggccccctgggcggttctgataacgagtaatcgttaatccgcaaataacgtaaaaacccgcttcggcgggtttttttatggggggagtttagggaaagagcatttgtcagaatatttaagggcgcctgtcactttgcttgatatatgagaattatttaaccttataaatgagaaaaaagcaacgcactttaaataagatacgttgctttttcgattgatgaacacctataattaaactattcatctattatttatgattttttgtatatacaatatttctagtttgttaaagagaattaagaaaataaatctcgaaaataataaagggaaaatcagtttttgatatcaaaattatacatgtcaacgataatacaaaatataatacaaactataagatgttatcagtatttattatgcatttagaataaattttgtgtcgcccttattcgactcactatagaagttcctattctctagaaagtagaggaacttcacttcattttgctagcgtgtgagggcctatttcccatgattccttcatatttgcatatacgatacaaggctgttagagagataattggaattaatttgactgtaaacacaaagatattagtacaaaatacgtgacgtagaaagtaataatttcttgggtagtttgcagttttaaaattatgttttaaaatggactatcatatgcttaccgtaacttgaaagtatttcgatttcttggctttatatatcttgtggaaaggacgaaacaccgttagctataggctaataagatagttgtgtcaagtgcttcggagacctaacacgtctccagtcacaacggctaaaaatagcca

SEQ ID NO: 174 - DNA, 3364 bp, synthetic construct
  misc_feature 1..3364: note = plasmid including the sequence for B-Gen.1 human albumin target 52
  source 1..3364: mol_type = other DNA
gcactgcatttgtttcaaaatattgggttttttgttttcaacaccggtaccgcgttacaatgataagtcgactgaataagtgaactcgagatcagcctcgactgtgccttctagttgccagccatctgttgtttgcccctcccccgtgccttccttgaccctggaaggtgccactcccactgtcctttcctaataaaatgaggaaattgcatccccacttcagaagttcctatactttctagtgaatgagtgagctaactcacattaattgcgttgcgctcactgcccgctttccagtcgggaaacctgtcgtgccagctgcattaatgaatcggccaacgcgcggggagaggcggtttgcgtattgggcgctcttgcgcttcctcgctcactgactcgctgcgctcggtcgttcggctgcggcgagcggtatcagctcactcaaaggcggtaatacggttatccacagaatcaggggataacgcaggaaagaacatgtgagcaaaaggccagcaaaaggccaggaaccgtaaaaaggccgcgttgctggcgtttttccataggctccgcccccctgacgagcatcacaaaaatcgacgctcaagtcagaggtggcgaaacccgacaggactataaagataccaggcgtttccccctggaagctccctcgtgcgctctcctgttccgaccctgccgcttaccggatacctgtccgcctttctcccttcgggaagcgtggcgctttctcatagctcacgctgtaggtatctcagttcggtgtaggtcgttcgctccaagctgggctgtgtgcacgaaccccccgttcagcccgaccgctgcgccttatccggtaactatcgtcttgagtccaacccggtaagacacgacttatcgccactggcagcagccactggtaacaggattagcagagcgaggtatgtaggcggtgctacagagttcttgaagtggtggcctaactacggctacactagaagaacagtatttggtatctgcgctctgctgaagccagttaccttcggaaaaagagttggtagctcttgatccggcaaacaaaccaccgctggtagcggtggtttttttgtttgcaagcagcagattacgcgcagaaaaaaaggatctcaagaagatcctttgatcttttctacggggtctgacgctcagtggaacgaaaactcacgttaagggattttggtcatgagattatcaaaaaggatcttcacctagatccttttaaattaaaaatgaagttttaaatcaatctaaagtatatatgagtaaacttggtctgacagttaccaatgcttaatcagtgaggcacctatctcagcgatctgtctatttcgttcatccatagttgcctgactccccgtcgtgtagataactacgatacgggagggcttaccatctggccccagtgctgcaatgataccgcgtgacccacgctcaccggctccagatttatcagcaataaaccagccagccggaagggccgagcgcagaagtggtcctgcaactttatccgcctccatccagtctattaattgttgccgggaagctagagtaagtagttcgccagttaatagtttgcgcaacgttgttgccattgctacaggcatcgtggtgtcacgctcgtcgtttggtatggcttcattcagctccggttcccaacgatcaaggcgagttacatgatcccccatgttgtgcaaaaaagcggttagctccttcggtcctccgatcgttgtcagaagtaagttggccgcagtgttatcactcatggttatggcagcactgcataattctcttactgtcatgccatccgtaagatgcttttctgtgactggtgagtactcaaccaagtcattctgagaatagtgtatgcggcgaccgagttgctcttgcccggcgtcaatacgggataataccgcgccacatagcagaactttaaaagtgctcatcattggaaaacgttcttcggggcgaaaactctcaaggatcttaccgctgttgagatccagttcgatgtaacccactcgtgcacccaactgatcttcagcatcttttactttcaccagcgtttctgggtgagcaaaaacaggaaggcaaaatgccgcaaaaaagggaataagggcgacacggaaatgttgaatactcatactcttcctttttcaatattattgaagcatttatcagggttattgtctcatgagcggatacatatttgaatgtatttagaaaaataaacaaataggggttccgcgcatatttccccgaaaagtgccacctgacgtcgacggatcgggagatctcccgatcccctatggtgcactctcagtacaatctgctctgatgccgcatagttaagccagtatctgctccctgcttgtgtgttggaggtcgctgagtagtgcgcgagcaaaatttaagctacaacaaggcaaggcttgaccgagcaaacaaactctttctgtgttgtaaaacgacggccagtcttaagctcgggccccctgggcggttctgataacgagtaatcgttaatccgcaaataacgtaaaaacccgcttcggcgggtttttttatggggggagtttagggaaagagcatttgtcagaatatttaagggcgcctgtcactttgcttgatatatgagaattatttaaccttataaatgagaaaaaagcaacgcactttaaataagatacgttgctttttcgattgatgaacacctataattaaactattcatctattatttatgattttttgtatatacaatatttctagtttgttaaagagaattaagaaaataaatctcgaaaataataaagggaaaatcagtttttgatatcaaaattatacatgtcaacgataatacaaaatataatacaaactataagatgttatcagtatttattatgcatttagaataaattttgtgtcgcccttattcgactcactatagaagttcctattctctagaaagtagaggaacttcacttcattttgctagcgtgtgagggcctatttcccatgattccttcatatttgcatatacgatacaaggctgttagagagataattggaattaatttgactgtaaacacaaagatattagtacaaaatacgtgacgtagaaagtaataatttcttgggtagtttgcagttttaaaattatgttttaaaatggactatcatatgcttaccgtaacttgaaagtatttcgatttcttggctttatatatcttgtggaaaggacgaaacaccgttagctataggctaataagatagttgtgtcaagtgcttcggagacctaacacgtctccagtcacaacggctaaaaatagcca

SEQ ID NO: 175 - DNA, 3364 bp, synthetic construct
  misc_feature 1..3364: note = plasmid including the sequence for B-Gen.1 human albumin target 53
  source 1..3364: mol_type = other DNA
gcacctttccatttgacttagattatgttttttgttttcaacaccggtaccgcgttacaatgataagtcgactgaataagtgaactcgagatcagcctcgactgtgccttctagttgccagccatctgttgtttgcccctcccccgtgccttccttgaccctggaaggtgccactcccactgtcctttcctaataaaatgaggaaattgcatccccacttcagaagttcctatactttctagtgaatgagtgagctaactcacattaattgcgttgcgctcactgcccgctttccagtcgggaaacctgtcgtgccagctgcattaatgaatcggccaacgcgcggggagaggcggtttgcgtattgggcgctcttgcgcttcctcgctcactgactcgctgcgctcggtcgttcggctgcggcgagcggtatcagctcactcaaaggcggtaatacggttatccacagaatcaggggataacgcaggaaagaacatgtgagcaaaaggccagcaaaaggccaggaaccgtaaaaaggccgcgttgctggcgtttttccataggctccgcccccctgacgagcatcacaaaaatcgacgctcaagtcagaggtggcgaaacccgacaggactataaagataccaggcgtttccccctggaagctccctcgtgcgctctcctgttccgaccctgccgcttaccggatacctgtccgcctttctcccttcgggaagcgtggcgctttctcatagctcacgctgtaggtatctcagttcggtgtaggtcgttcgctccaagctgggctgtgtgcacgaaccccccgttcagcccgaccgctgcgccttatccggtaactatcgtcttgagtccaacccggtaagacacgacttatcgccactggcagcagccactggtaacaggattagcagagcgaggtatgtaggcggtgctacagagttcttgaagtggtggcctaactacggctacactagaagaacagtatttggtatctgcgctctgctgaagccagttaccttcggaaaaagagttggtagctcttgatccggcaaacaaaccaccgctggtagcggtggtttttttgtttgcaagcagcagattacgcgcagaaaaaaaggatctcaagaagatcctttgatcttttctacggggtctgacgctcagtggaacgaaaactcacgttaagggattttggtcatgagattatcaaaaaggatcttcacctagatccttttaaattaaaaatgaagttttaaatcaatctaaagtatatatgagtaaacttggtctgacagttaccaatgcttaatcagtgaggcacctatctcagcgatctgtctatttcgttcatccatagttgcctgactccccgtcgtgtagataactacgatacgggagggcttaccatctggccccagtgctgcaatgataccgcgtgacccacgctcaccggctccagatttatcagcaataaaccagccagccggaagggccgagcgcagaagtggtcctgcaactttatccgcctccatccagtctattaattgttgccgggaagctagagtaagtagttcgccagttaatagtttgcgcaacgttgttgccattgctacaggcatcgtggtgtcacgctcgtcgtttggtatggcttcattcagctccggttcccaacgatcaaggcgagttacatgatcccccatgttgtgcaaaaaagcggttagctccttcggtcctccgatcgttgtcagaagtaagttggccgcagtgttatcactcatggttatggcagcactgcataattctcttactgtcatgccatccgtaagatgcttttctgtgactggtgagtactcaaccaagtcattctgagaatagtgtatgcggcgaccgagttgctcttgcccggcgtcaatacgggataataccgcgccacatagcagaactttaaaagtgctcatcattggaaaacgttcttcggggcgaaaactctcaaggatcttaccgctgttgagatccagttcgatgtaacccactcgtgcacccaactgatcttcagcatcttttactttcaccagcgtttctgggtgagcaaaaacaggaaggcaaaatgccgcaaaaaagggaataagggcgacacggaaatgttgaatactcatactcttcctttttcaatattattgaagcatttatcagggttattgtctcatgagcggatacatatttgaatgtatttagaaaaataaacaaataggggttccgcgcatatttccccgaaaagtgccacctgacgtcgacggatcgggagatctcccgatcccctatggtgcactctcagtacaatctgctctgatgccgcatagttaagccagtatctgctccctgcttgtgtgttggaggtcgctgagtagtgcgcgagcaaaatttaagctacaacaaggcaaggcttgaccgagcaaacaaactctttctgtgttgtaaaacgacggccagtcttaagctcgggccccctgggcggttctgataacgagtaatcgttaatccgcaaataacgtaaaaacccgcttcggcgggtttttttatggggggagtttagggaaagagcatttgtcagaatatttaagggcgcctgtcactttgcttgatatatgagaattatttaaccttataaatgagaaaaaagcaacgcactttaaataagatacgttgctttttcgattgatgaacacctataattaaactattcatctattatttatgattttttgtatatacaatatttctagtttgttaaagagaattaagaaaataaatctcgaaaataataaagggaaaatcagtttttgatatcaaaattatacatgtcaacgataatacaaaatataatacaaactataagatgttatcagtatttattatgcatttagaataaattttgtgtcgcccttattcgactcactatagaagttcctattctctagaaagtagaggaacttcacttcattttgctagcgtgtgagggcctatttcccatgattccttcatatttgcatatacgatacaaggctgttagagagataattggaattaatttgactgtaaacacaaagatattagtacaaaatacgtgacgtagaaagtaataatttcttgggtagtttgcagttttaaaattatgttttaaaatggactatcatatgcttaccgtaacttgaaagtatttcgatttcttggctttatatatcttgtggaaaggacgaaacaccgttagctataggctaataagatagttgtgtcaagtgcttcggagacctaacacgtctccagtcacaacggctaaaaatagcca

SEQ ID NO: 176 - DNA, 3364 bp, synthetic construct
  misc_feature 1..3364: note = plasmid including the sequence for B-Gen.1 human albumin target 54
  source 1..3364: mol_type = other DNA
gcacttacttcttgttttcttcagtatttttttgttttcaacaccggtaccgcgttacaatgataagtcgactgaataagtgaactcgagatcagcctcgactgtgccttctagttgccagccatctgttgtttgcccctcccccgtgccttccttgaccctggaaggtgccactcccactgtcctttcctaataaaatgaggaaattgcatccccacttcagaagttcctatactttctagtgaatgagtgagctaactcacattaattgcgttgcgctcactgcccgctttccagtcgggaaacctgtcgtgccagctgcattaatgaatcggccaacgcgcggggagaggcggtttgcgtattgggcgctcttgcgcttcctcgctcactgactcgctgcgctcggtcgttcggctgcggcgagcggtatcagctcactcaaaggcggtaatacggttatccacagaatcaggggataacgcaggaaagaacatgtgagcaaaaggccagcaaaaggccaggaaccgtaaaaaggccgcgttgctggcgtttttccataggctccgcccccctgacgagcatcacaaaaatcgacgctcaagtcagaggtggcgaaacccgacaggactataaagataccaggcgtttccccctggaagctccctcgtgcgctctcctgttccgaccctgccgcttaccggatacctgtccgcctttctcccttcgggaagcgtggcgctttctcatagctcacgctgtaggtatctcagttcggtgtaggtcgttcgctccaagctgggctgtgtgcacgaaccccccgttcagcccgaccgctgcgccttatccggtaactatcgtcttgagtccaacccggtaagacacgacttatcgccactggcagcagccactggtaacaggattagcagagcgaggtatgtaggcggtgctacagagttcttgaagtggtggcctaactacggctacactagaagaacagtatttggtatctgcgctctgctgaagccagttaccttcggaaaaagagttggtagctcttgatccggcaaacaaaccaccgctggtagcggtggtttttttgtttgcaagcagcagattacgcgcagaaaaaaaggatctcaagaagatcctttgatcttttctacggggtctgacgctcagtggaacgaaaactcacgttaagggattttggtcatgagattatcaaaaaggatcttcacctagatccttttaaattaaaaatgaagttttaaatcaatctaaagtatatatgagtaaacttggtctgacagttaccaatgcttaatcagtgaggcacctatctcagcgatctgtctatttcgttcatccatagttgcctgactccccgtcgtgtagataactacgatacgggagggcttaccatctggccccagtgctgcaatgataccgcgtgacccacgctcaccggctccagatttatcagcaataaaccagccagccggaagggccgagcgcagaagtggtcctgcaactttatccgcctccatccagtctattaattgttgccgggaagctagagtaagtagttcgccagttaatagtttgcgcaacgttgttgccattgctacaggcatcgtggtgtcacgctcgtcgtttggtatggcttcattcagctccggttcccaacgatcaaggcgagttacatgatcccccatgttgtgcaaaaaagcggttagctccttcggtcctccgatcgttgtcagaagtaagttggccgcagtgttatcactcatggttatggcagcactgcataattctcttactgtcatgccatccgtaagatgcttttctgtgactggtgagtactcaaccaagtcattctgagaatagtgtatgcggcgaccgagttgctcttgcccggcgtcaatacgggataataccgcgccacatagcagaactttaaaagtgctcatcattggaaaacgttcttcggggcgaaaactctcaaggatcttaccgctgttgagatccagttcgatgtaacccactcgtgcacccaactgatcttcagcatcttttactttcaccagcgtttctgggtgagcaaaaacaggaaggcaaaatgccgcaaaaaagggaataagggcgacacggaaatgttgaatactcatactcttcctttttcaatattattgaagcatttatcagggttattgtctcatgagcggatacatatttgaatgtatttagaaaaataaacaaataggggttccgcgcatatttccccgaaaagtgccacctgacgtcgacggatcgggagatctcccgatcccctatggtgcactctcagtacaatctgctctgatgccgcatagttaagccagtatctgctccctgcttgtgtgttggaggtcgctgagtagtgcgcgagcaaaatttaagctacaacaaggcaaggcttgaccgagcaaacaaactctttctgtgttgtaaaacgacggccagtcttaagctcgggccccctgggcggttctgataacgagtaatcgttaatccgcaaataacgtaaaaacccgcttcggcgggtttttttatggggggagtttagggaaagagcatttgtcagaatatttaagggcgcctgtcactttgcttgatatatgagaattatttaaccttataaatgagaaaaaagcaacgcactttaaataagatacgttgctttttcgattgatgaacacctataattaaactattcatctattatttatgattttttgtatatacaatatttctagtttgttaaagagaattaagaaaataaatctcgaaaataataaagggaaaatcagtttttgatatcaaaattatacatgtcaacgataatacaaaatataatacaaactataagatgttatcagtatttattatgcatttagaataaattttgtgtcgcccttattcgactcactatagaagttcctattctctagaaagtagaggaacttcacttcattttgctagcgtgtgagggcctatttcccatgattccttcatatttgcatatacgatacaaggctgttagagagataattggaattaatttgactgtaaacacaaagatattagtacaaaatacgtgacgtagaaagtaataatttcttgggtagtttgcagttttaaaattatgttttaaaatggactatcatatgcttaccgtaacttgaaagtatttcgatttcttggctttatatatcttgtggaaaggacgaaacaccgttagctataggctaataagatagttgtgtcaagtgcttcggagacctaacacgtctccagtcacaacggctaaaaatagcca

SEQ ID NO: 177 - DNA, 3364 bp, synthetic construct
  misc_feature 1..3364: note = plasmid including the sequence for B-Gen.1 human albumin target 55
  source 1..3364: mol_type = other DNA
gcaccttcttgttttcttcagtatttattttttgttttcaacaccggtaccgcgttacaatgataagtcgactgaataagtgaactcgagatcagcctcgactgtgccttctagttgccagccatctgttgtttgcccctcccccgtgccttccttgaccctggaaggtgccactcccactgtcctttcctaataaaatgaggaaattgcatccccacttcagaagttcctatactttctagtgaatgagtgagctaactcacattaattgcgttgcgctcactgcccgctttccagtcgggaaacctgtcgtgccagctgcattaatgaatcggccaacgcgcggggagaggcggtttgcgtattgggcgctcttgcgcttcctcgctcactgactcgctgcgctcggtcgttcggctgcggcgagcggtatcagctcactcaaaggcggtaatacggttatccacagaatcaggggataacgcaggaaagaacatgtgagcaaaaggccagcaaaaggccaggaaccgtaaaaaggccgcgttgctggcgtttttccataggctccgcccccctgacgagcatcacaaaaatcgacgctcaagtcagaggtggcgaaacccgacaggactataaagataccaggcgtttccccctggaagctccctcgtgcgctctcctgttccgaccctgccgcttaccggatacctgtccgcctttctcccttcgggaagcgtggcgctttctcatagctcacgctgtaggtatctcagttcggtgtaggtcgttcgctccaagctgggctgtgtgcacgaaccccccgttcagcccgaccgctgcgccttatccggtaactatcgtcttgagtccaacccggtaagacacgacttatcgccactggcagcagccactggtaacaggattagcagagcgaggtatgtaggcggtgctacagagttcttgaagtggtggcctaactacggctacactagaagaacagtatttggtatctgcgctctgctgaagccagttaccttcggaaaaagagttggtagctcttgatccggcaaacaaaccaccgctggtagcggtggtttttttgtttgcaagcagcagattacgcgcagaaaaaaaggatctcaagaagatcctttgatcttttctacggggtctgacgctcagtggaacgaaaactcacgttaagggattttggtcatgagattatcaaaaaggatcttcacctagatccttttaaattaaaaatgaagttttaaatcaatctaaagtatatatgagtaaacttggtctgacagttaccaatgcttaatcagtgaggcacctatctcagcgatctgtctatttcgttcatccatagttgcctgactccccgtcgtgtagataactacgatacgggagggcttaccatctggccccagtgctgcaatgataccgcgtgacccacgctcaccggctccagatttatcagcaataaaccagccagccggaagggccgagcgcagaagtggtcctgcaactttatccgcctccatccagtctattaattgttgccgggaagctagagtaagtagttcgccagttaatagtttgcgcaacgttgttgccattgctacaggcatcgtggtgtcacgctcgtcgtttggtatggcttcattcagctccggttcccaacgatcaaggcgagttacatgatcccccatgttgtgcaaaaaagcggttagctccttcggtcctccgatcgttgtcagaagtaagttggccgcagtgttatcactcatggttatggcagcactgcataattctcttactgtcatgccatccgtaagatgcttttctgtgactggtgagtactcaaccaagtcattctgagaatagtgtatgcggcgaccgagttgctcttgcccggcgtcaatacgggataataccgcgccacatagcagaactttaaaagtgctcatcattggaaaacgttcttcggggcgaaaactctcaaggatcttaccgctgttgagatccagttcgatgtaacccactcgtgcacccaactgatcttcagcatcttttactttcaccagcgtttctgggtgagcaaaaacaggaaggcaaaatgccgcaaaaaagggaataagggcgacacggaaatgttgaatactcatactcttcctttttcaatattattgaagcatttatcagggttattgtctcatgagcggatacatatttgaatgtatttagaaaaataaacaaataggggttccgcgcatatttccccgaaaagtgccacctgacgtcgacggatcgggagatctcccgatcccctatggtgcactctcagtacaatctgctctgatgccgcatagttaagccagtatctgctccctgcttgtgtgttggaggtcgctgagtagtgcgcgagcaaaatttaagctacaacaaggcaaggcttgaccgagcaaacaaactctttctgtgttgtaaaacgacggccagtcttaagctcgggccccctgggcggttctgataacgagtaatcgttaatccgcaaataacgtaaaaacccgcttcggcgggtttttttatggggggagtttagggaaagagcatttgtcagaatatttaagggcgcctgtcactttgcttgatatatgagaattatttaaccttataaatgagaaaaaagcaacgcactttaaataagatacgttgctttttcgattgatgaacacctataattaaactattcatctattatttatgattttttgtatatacaatatttctagtttgttaaagagaattaagaaaataaatctcgaaaataataaagggaaaatcagtttttgatatcaaaattatacatgtcaacgataatacaaaatataatacaaactataagatgttatcagtatttattatgcatttagaataaattttgtgtcgcccttattcgactcactatagaagttcctattctctagaaagtagaggaacttcacttcattttgctagcgtgtgagggcctatttcccatgattccttcatatttgcatatacgatacaaggctgttagagagataattggaattaatttgactgtaaacacaaagatattagtacaaaatacgtgacgtagaaagtaataatttcttgggtagtttgcagttttaaaattatgttttaaaatggactatcatatgcttaccgtaacttgaaagtatttcgatttcttggctttatatatcttgtggaaaggacgaaacaccgttagctataggctaataagatagttgtgtcaagtgcttcggagacctaacacgtctccagtcacaacggctaaaaatagcca

SEQ ID NO: 178 - DNA, 3364 bp, synthetic construct
  misc_feature 1..3364: note = plasmid including the sequence for B-Gen.1 human albumin target 56
  source 1..3364: mol_type = other DNA
gcacaacaatccttttttttcttccctttttttgttttcaacaccggtaccgcgttacaatgataagtcgactgaataagtgaactcgagatcagcctcgactgtgccttctagttgccagccatctgttgtttgcccctcccccgtgccttccttgaccctggaaggtgccactcccactgtcctttcctaataaaatgaggaaattgcatccccacttcagaagttcctatactttctagtgaatgagtgagctaactcacattaattgcgttgcgctcactgcccgctttccagtcgggaaacctgtcgtgccagctgcattaatgaatcggccaacgcgcggggagaggcggtttgcgtattgggcgctcttgcgcttcctcgctcactgactcgctgcgctcggtcgttcggctgcggcgagcggtatcagctcactcaaaggcggtaatacggttatccacagaatcaggggataacgcaggaaagaacatgtgagcaaaaggccagcaaaaggccaggaaccgtaaaaaggccgcgttgctggcgtttttccataggctccgcccccctgacgagcatcacaaaaatcgacgctcaagtcagaggtggcgaaacccgacaggactataaagataccaggcgtttccccctggaagctccctcgtgcgctctcctgttccgaccctgccgcttaccggatacctgtccgcctttctcccttcgggaagcgtggcgctttctcatagctcacgctgtaggtatctcagttcggtgtaggtcgttcgctccaagctgggctgtgtgcacgaaccccccgttcagcccgaccgctgcgccttatccggtaactatcgtcttgagtccaacccggtaagacacgacttatcgccactggcagcagccactggtaacaggattagcagagcgaggtatgtaggcggtgctacagagttcttgaagtggtggcctaactacggctacactagaagaacagtatttggtatctgcgctctgctgaagccagttaccttcggaaaaagagttggtagctcttgatccggcaaacaaaccaccgctggtagcggtggtttttttgtttgcaagcagcagattacgcgcagaaaaaaaggatctcaagaagatcctttgatcttttctacggggtctgacgctcagtggaacgaaaactcacgttaagggattttggtcatgagattatcaaaaaggatcttcacctagatccttttaaattaaaaatgaagttttaaatcaatctaaagtatatatgagtaaacttggtctgacagttaccaatgcttaatcagtgaggcacctatctcagcgatctgtctatttcgttcatccatagttgcctgactccccgtcgtgtagataactacgatacgggagggcttaccatctggccccagtgctgcaatgataccgcgtgacccacgctcaccggctccagatttatcagcaataaaccagccagccggaagggccgagcgcagaagtggtcctgcaactttatccgcctccatccagtctattaattgttgccgggaagctagagtaagtagttcgccagttaatagtttgcgcaacgttgttgccattgctacaggcatcgtggtgtcacgctcgtcgtttggtatggcttcattcagctccggttcccaacgatcaaggcgagttacatgatcccccatgttgtgcaaaaaagcggttagctccttcggtcctccgatcgttgtcagaagtaagttggccgcagtgttatcactcatggttatggcagcactgcataattctcttactgtcatgccatccgtaagatgcttttctgtgactggtgagtactcaaccaagtcattctgagaatagtgtatgcggcgaccgagttgctcttgcccggcgtcaatacgggataataccgcgccacatagcagaactttaaaagtgctcatcattggaaaacgttcttcggggcgaaaactctcaaggatcttaccgctgttgagatccagttcgatgtaacccactcgtgcacccaactgatcttcagcatcttttactttcaccagcgtttctgggtgagcaaaaacaggaaggcaaaatgccgcaaaaaagggaataagggcgacacggaaatgttgaatactcatactcttcctttttcaatattattgaagcatttatcagggttattgtctcatgagcggatacatatttgaatgtatttagaaaaataaacaaataggggttccgcgcatatttccccgaaaagtgccacctgacgtcgacggatcgggagatctcccgatcccctatggtgcactctcagtacaatctgctctgatgccgcatagttaagccagtatctgctccctgcttgtgtgttggaggtcgctgagtagtgcgcgagcaaaatttaagctacaacaaggcaaggcttgaccgagcaaacaaactctttctgtgttgtaaaacgacggccagtcttaagctcgggccccctgggcggttctgataacgagtaatcgttaatccgcaaataacgtaaaaacccgcttcggcgggtttttttatggggggagtttagggaaagagcatttgtcagaatatttaagggcgcctgtcactttgcttgatatatgagaattatttaaccttataaatgagaaaaaagcaacgcactttaaataagatacgttgctttttcgattgatgaacacctataattaaactattcatctattatttatgattttttgtatatacaatatttctagtttgttaaagagaattaagaaaataaatctcgaaaataataaagggaaaatcagtttttgatatcaaaattatacatgtcaacgataatacaaaatataatacaaactataagatgttatcagtatttattatgcatttagaataaattttgtgtcgcccttattcgactcactatagaagttcctattctctagaaagtagaggaacttcacttcattttgctagcgtgtgagggcctatttcccatgattccttcatatttgcatatacgatacaaggctgttagagagataattggaattaatttgactgtaaacacaaagatattagtacaaaatacgtgacgtagaaagtaataatttcttgggtagtttgcagttttaaaattatgttttaaaatggactatcatatgcttaccgtaacttgaaagtatttcgatttcttggctttatatatcttgtggaaaggacgaaacaccgttagctataggctaataagatagttgtgtcaagtgcttcggagacctaacacgtctccagtcacaacggctaaaaatagcca

SEQ ID NO: 179 - DNA, 3364 bp, synthetic construct
  misc_feature 1..3364: note = plasmid including the sequence for B-Gen.1 human albumin target 57
  source 1..3364: mol_type = other DNA
gcacttaaatactgaagaaaacaagaattttttgttttcaacaccggtaccgcgttacaatgataagtcgactgaataagtgaactcgagatcagcctcgactgtgccttctagttgccagccatctgttgtttgcccctcccccgtgccttccttgaccctggaaggtgccactcccactgtcctttcctaataaaatgaggaaattgcatccccacttcagaagttcctatactttctagtgaatgagtgagctaactcacattaattgcgttgcgctcactgcccgctttccagtcgggaaacctgtcgtgccagctgcattaatgaatcggccaacgcgcggggagaggcggtttgcgtattgggcgctcttgcgcttcctcgctcactgactcgctgcgctcggtcgttcggctgcggcgagcggtatcagctcactcaaaggcggtaatacggttatccacagaatcaggggataacgcaggaaagaacatgtgagcaaaaggccagcaaaaggccaggaaccgtaaaaaggccgcgttgctggcgtttttccataggctccgcccccctgacgagcatcacaaaaatcgacgctcaagtcagaggtggcgaaacccgacaggactataaagataccaggcgtttccccctggaagctccctcgtgcgctctcctgttccgaccctgccgcttaccggatacctgtccgcctttctcccttcgggaagcgtggcgctttctcatagctcacgctgtaggtatctcagttcggtgtaggtcgttcgctccaagctgggctgtgtgcacgaaccccccgttcagcccgaccgctgcgccttatccggtaactatcgtcttgagtccaacccggtaagacacgacttatcgccactggcagcagccactggtaacaggattagcagagcgaggtatgtaggcggtgctacagagttcttgaagtggtggcctaactacggctacactagaagaacagtatttggtatctgcgctctgctgaagccagttaccttcggaaaaagagttggtagctcttgatccggcaaacaaaccaccgctggtagcggtggtttttttgtttgcaagcagcagattacgcgcagaaaaaaaggatctcaagaagatcctttgatcttttctacggggtctgacgctcagtggaacgaaaactcacgttaagggattttggtcatgagattatcaaaaaggatcttcacctagatccttttaaattaaaaatgaagttttaaatcaatctaaagtatatatgagtaaacttggtctgacagttaccaatgcttaatcagtgaggcacctatctcagcgatctgtctatttcgttcatccatagttgcctgactccccgtcgtgtagataactacgatacgggagggcttaccatctggccccagtgctgcaatgataccgcgtgacccacgctcaccggctccagatttatcagcaataaaccagccagccggaagggccgagcgcagaagtggtcctgcaactttatccgcctccatccagtctattaattgttgccgggaagctagagtaagtagttcgccagttaatagtttgcgcaacgttgttgccattgctacaggcatcgtggtgtcacgctcgtcgtttggtatggcttcattcagctccggttcccaacgatcaaggcgagttacatgatcccccatgttgtgcaaaaaagcggttagctccttcggtcctccgatcgttgtcagaagtaagttggccgcagtgttatcactcatggttatggcagcactgcataattctcttactgtcatgccatccgtaagatgcttttctgtgactggtgagtactcaaccaagtcattctgagaatagtgtatgcggcgaccgagttgctcttgcccggcgtcaatacgggataataccgcgccacatagcagaactttaaaagtgctcatcattggaaaacgttcttcggggcgaaaactctcaaggatcttaccgctgttgagatccagttcgatgtaacccactcgtgcacccaactgatcttcagcatcttttactttcaccagcgtttctgggtgagcaaaaacaggaaggcaaaatgccgcaaaaaagggaataagggcgacacggaaatgttgaatactcatactcttcctttttcaatattattgaagcatttatcagggttattgtctcatgagcggatacatatttgaatgtatttagaaaaataaacaaataggggttccgcgcatatttccccgaaaagtgccacctgacgtcgacggatcgggagatctcccgatcccctatggtgcactctcagtacaatctgctctgatgccgcatagttaagccagtatctgctccctgcttgtgtgttggaggtcgctgagtagtgcgcgagcaaaatttaagctacaacaaggcaaggcttgaccgagcaaacaaactctttctgtgttgtaaaacgacggccagtcttaagctcgggccccctgggcggttctgataacgagtaatcgttaatccgcaaataacgtaaaaacccgcttcggcgggtttttttatggggggagtttagggaaagagcatttgtcagaatatttaagggcgcctgtcactttgcttgatatatgagaattatttaaccttataaatgagaaaaaagcaacgcactttaaataagatacgttgctttttcgattgatgaacacctataattaaactattcatctattatttatgattttttgtatatacaatatttctagtttgttaaagagaattaagaaaataaatctcgaaaataataaagggaaaatcagtttttgatatcaaaattatacatgtcaacgataatacaaaatataatacaaactataagatgttatcagtatttattatgcatttagaataaattttgtgtcgcccttattcgactcactatagaagttcctattctctagaaagtagaggaacttcacttcattttgctagcgtgtgagggcctatttcccatgattccttcatatttgcatatacgatacaaggctgttagagagataattggaattaatttgactgtaaacacaaagatattagtacaaaatacgtgacgtagaaagtaataatttcttgggtagtttgcagttttaaaattatgttttaaaatggactatcatatgcttaccgtaacttgaaagtatttcgatttcttggctttatatatcttgtggaaaggacgaaacaccgttagctataggctaataagatagttgtgtcaagtgcttcggagacctaacacgtctccagtcacaacggctaaaaatagcca

SEQ ID NO: 180 - DNA, 3364 bp, synthetic construct
  misc_feature 1..3364: note = plasmid including the sequence for B-Gen.1 human albumin target 58
  source 1..3364: mol_type = other DNA
gcacaaacatcctaggtaaaaaaaaaattttttgttttcaacaccggtaccgcgttacaatgataagtcgactgaataagtgaactcgagatcagcctcgactgtgccttctagttgccagccatctgttgtttgcccctcccccgtgccttccttgaccctggaaggtgccactcccactgtcctttcctaataaaatgaggaaattgcatccccacttcagaagttcctatactttctagtgaatgagtgagctaactcacattaattgcgttgcgctcactgcccgctttccagtcgggaaacctgtcgtgccagctgcattaatgaatcggccaacgcgcggggagaggcggtttgcgtattgggcgctcttgcgcttcctcgctcactgactcgctgcgctcggtcgttcggctgcggcgagcggtatcagctcactcaaaggcggtaatacggttatccacagaatcaggggataacgcaggaaagaacatgtgagcaaaaggccagcaaaaggccaggaaccgtaaaaaggccgcgttgctggcgtttttccataggctccgcccccctgacgagcatcacaaaaatcgacgctcaagtcagaggtggcgaaacccgacaggactataaagataccaggcgtttccccctggaagctccctcgtgcgctctcctgttccgaccctgccgcttaccggatacctgtccgcctttctcccttcgggaagcgtggcgctttctcatagctcacgctgtaggtatctcagttcggtgtaggtcgttcgctccaagctgggctgtgtgcacgaaccccccgttcagcccgaccgctgcgccttatccggtaactatcgtcttgagtccaacccggtaagacacgacttatcgccactggcagcagccactggtaacaggattagcagagcgaggtatgtaggcggtgctacagagttcttgaagtggtggcctaactacggctacactagaagaacagtatttggtatctgcgctctgctgaagccagttaccttcggaaaaagagttggtagctcttgatccggcaaacaaaccaccgctggtagcggtggtttttttgtttgcaagcagcagattacgcgcagaaaaaaaggatctcaagaagatcctttgatcttttctacggggtctgacgctcagtggaacgaaaactcacgttaagggattttggtcatgagattatcaaaaaggatcttcacctagatccttttaaattaaaaatgaagttttaaatcaatctaaagtatatatgagtaaacttggtctgacagttaccaatgcttaatcagtgaggcacctatctcagcgatctgtctatttcgttcatccatagttgcctgactccccgtcgtgtagataactacgatacgggagggcttaccatctggccccagtgctgcaatgataccgcgtgacccacgctcaccggctccagatttatcagcaataaaccagccagccggaagggccgagcgcagaagtggtcctgcaactttatccgcctccatccagtctattaattgttgccgggaagctagagtaagtagttcgccagttaatagtttgcgcaacgttgttgccattgctacaggcatcgtggtgtcacgctcgtcgtttggtatggcttcattcagctccggttcccaacgatcaaggcgagttacatgatcccccatgttgtgcaaaaaagcggttagctccttcggtcctccgatcgttgtcagaagtaagttggccgcagtgttatcactcatggttatggcagcactgcataattctcttactgtcatgccatccgtaagatgcttttctgtgactggtgagtactcaaccaagtcattctgagaatagtgtatgcggcgaccgagttgctcttgcccggcgtcaatacgggataataccgcgccacatagcagaactttaaaagtgctcatcattggaaaacgttcttcggggcgaaaactctcaaggatcttaccgctgttgagatccagttcgatgtaacccactcgtgcacccaactgatcttcagcatcttttactttcaccagcgtttctgggtgagcaaaaacaggaaggcaaaatgccgcaaaaaagggaataagggcgacacggaaatgttgaatactcatactcttcctttttcaatattattgaagcatttatcagggttattgtctcatgagcggatacatatttgaatgtatttagaaaaataaacaaataggggttccgcgcatatttccccgaaaagtgccacctgacgtcgacggatcgggagatctcccgatcccctatggtgcactctcagtacaatctgctctgatgccgcatagttaagccagtatctgctccctgcttgtgtgttggaggtcgctgagtagtgcgcgagcaaaatttaagctacaacaaggcaaggcttgaccgagcaaacaaactctttctgtgttgtaaaacgacggccagtcttaagctcgggccccctgggcggttctgataacgagtaatcgttaatccgcaaataacgtaaaaacccgcttcggcgggtttttttatggggggagtttagggaaagagcatttgtcagaatatttaagggcgcctgtcactttgcttgatatatgagaattatttaaccttataaatgagaaaaaagcaacgcactttaaataagatacgttgctttttcgattgatgaacacctataattaaactattcatctattatttatgattttttgtatatacaatatttctagtttgttaaagagaattaagaaaataaatctcgaaaataataaagggaaaatcagtttttgatatcaaaattatacatgtcaacgataatacaaaatataatacaaactataagatgttatcagtatttattatgcatttagaataaattttgtgtcgcccttattcgactcactatagaagttcctattctctagaaagtagaggaacttcacttcattttgctagcgtgtgagggcctatttcccatgattccttcatatttgcatatacgatacaaggctgttagagagataattggaattaatttgactgtaaacacaaagatattagtacaaaatacgtgacgtagaaagtaataatttcttgggtagtttgcagttttaaaattatgttttaaaatggactatcatatgcttaccgtaacttgaaagtatttcgatttcttggctttatatatcttgtggaaaggacgaaacaccgttagctataggctaataagatagttgtgtcaagtgcttcggagacctaacacgtctccagtcacaacggctaaaaatagcca

SEQ ID NO: 181 - DNA, 3364 bp, synthetic construct
  misc_feature 1..3364: note = plasmid including the sequence for B-Gen.1 human albumin target 59
  source 1..3364: mol_type = other DNA
gcactattaataagataaccttgtaagttttttgttttcaacaccggtaccgcgttacaatgataagtcgactgaataagtgaactcgagatcagcctcgactgtgccttctagttgccagccatctgttgtttgcccctcccccgtgccttccttgaccctggaaggtgccactcccactgtcctttcctaataaaatgaggaaattgcatccccacttcagaagttcctatactttctagtgaatgagtgagctaactcacattaattgcgttgcgctcactgcccgctttccagtcgggaaacctgtcgtgccagctgcattaatgaatcggccaacgcgcggggagaggcggtttgcgtattgggcgctcttgcgcttcctcgctcactgactcgctgcgctcggtcgttcggctgcggcgagcggtatcagctcactcaaaggcggtaatacggttatccacagaatcaggggataacgcaggaaagaacatgtgagcaaaaggccagcaaaaggccaggaaccgtaaaaaggccgcgttgctggcgtttttccataggctccgcccccctgacgagcatcacaaaaatcgacgctcaagtcagaggtggcgaaacccgacaggactataaagataccaggcgtttccccctggaagctccctcgtgcgctctcctgttccgaccctgccgcttaccggatacctgtccgcctttctcccttcgggaagcgtggcgctttctcatagctcacgctgtaggtatctcagttcggtgtaggtcgttcgctccaagctgggctgtgtgcacgaaccccccgttcagcccgaccgctgcgccttatccggtaactatcgtcttgagtccaacccggtaagacacgacttatcgccactggcagcagccactggtaacaggattagcagagcgaggtatgtaggcggtgctacagagttcttgaagtggtggcctaactacggctacactagaagaacagtatttggtatctgcgctctgctgaagccagttaccttcggaaaaagagttggtagctcttgatccggcaaacaaaccaccgctggtagcggtggtttttttgtttgcaagcagcagattacgcgcagaaaaaaaggatctcaagaagatcctttgatcttttctacggggtctgacgctcagtggaacgaaaactcacgttaagggattttggtcatgagattatcaaaaaggatcttcacctagatccttttaaattaaaaatgaagttttaaatcaatctaaagtatatatgagtaaacttggtctgacagttaccaatgcttaatcagtgaggcacctatctcagcgatctgtctatttcgttcatccatagttgcctgactccccgtcgtgtagataactacgatacgggagggcttaccatctggccccagtgctgcaatgataccgcgtgacccacgctcaccggctccagatttatcagcaataaaccagccagccggaagggccgagcgcagaagtggtcctgcaactttatccgcctccatccagtctattaattgttgccgggaagctagagtaagtagttcgccagttaatagtttgcgcaacgttgttgccattgctacaggcatcgtggtgtcacgctcgtcgtttggtatggcttcattcagctccggttcccaacgatcaaggcgagttacatgatcccccatgttgtgcaaaaaagcggttagctccttcggtcctccgatcgttgtcagaagtaagttggccgcagtgttatcactcatggttatggcagcactgcataattctcttactgtcatgccatccgtaagatgcttttctgtgactggtgagtactcaaccaagtcattctgagaatagtgtatgcggcgaccgagttgctcttgcccggcgtcaatacgggataataccgcgccacatagcagaactttaaaagtgctcatcattggaaaacgttcttcggggcgaaaactctcaaggatcttaccgctgttgagatccagttcgatgtaacccactcgtgcacccaactgatcttcagcatcttttactttcaccagcgtttctgggtgagcaaaaacaggaaggcaaaatgccgcaaaaaagggaataagggcgacacggaaatgttgaatactcatactcttcctttttcaatattattgaagcatttatcagggttattgtctcatgagcggatacatatttgaatgtatttagaaaaataaacaaataggggttccgcgcatatttccccgaaaagtgccacctgacgtcgacggatcgggagatctcccgatcccctatggtgcactctcagtacaatctgctctgatgccgcatagttaagccagtatctgctccctgcttgtgtgttggaggtcgctgagtagtgcgcgagcaaaatttaagctacaacaaggcaaggcttgaccgagcaaacaaactctttctgtgttgtaaaacgacggccagtcttaagctcgggccccctgggcggttctgataacgagtaatcgttaatccgcaaataacgtaaaaacccgcttcggcgggtttttttatggggggagtttagggaaagagcatttgtcagaatatttaagggcgcctgtcactttgcttgatatatgagaattatttaaccttataaatgagaaaaaagcaacgcactttaaataagatacgttgctttttcgattgatgaacacctataattaaactattcatctattatttatgattttttgtatatacaatatttctagtttgttaaagagaattaagaaaataaatctcgaaaataataaagggaaaatcagtttttgatatcaaaattatacatgtcaacgataatacaaaatataatacaaactataagatgttatcagtatttattatgcatttagaataaattttgtgtcgcccttattcgactcactatagaagttcctattctctagaaagtagaggaacttcacttcattttgctagcgtgtgagggcctatttcccatgattccttcatatttgcatatacgatacaaggctgttagagagataattggaattaatttgactgtaaacacaaagatattagtacaaaatacgtgacgtagaaagtaataatttcttgggtagtttgcagttttaaaattatgttttaaaatggactatcatatgcttaccgtaacttgaaagtatttcgatttcttggctttatatatcttgtggaaaggacgaaacaccgttagctataggctaataagatagttgtgtcaagtgcttcggagacctaacacgtctccagtcacaacggctaaaaatagcca

SEQ ID NO: 182 - DNA, 3364 bp, synthetic construct
  misc_feature 1..3364: note = plasmid including the sequence for B-Gen.1 human albumin target 60
  source 1..3364: mol_type = other DNA
gcacaaacttagataatatctaatactttttttgttttcaacaccggtaccgcgttacaatgataagtcgactgaataagtgaactcgagatcagcctcgactgtgccttctagttgccagccatctgttgtttgcccctcccccgtgccttccttgaccctggaaggtgccactcccactgtcctttcctaataaaatgaggaaattgcatccccacttcagaagttcctatactttctagtgaatgagtgagctaactcacattaattgcgttgcgctcactgcccgctttccagtcgggaaacctgtcgtgccagctgcattaatgaatcggccaacgcgcggggagaggcggtttgcgtattgggcgctcttgcgcttcctcgctcactgactcgctgcgctcggtcgttcggctgcggcgagcggtatcagctcactcaaaggcggtaatacggttatccacagaatcaggggataacgcaggaaagaacatgtgagcaaaaggccagcaaaaggccaggaaccgtaaaaaggccgcgttgctggcgtttttccataggctccgcccccctgacgagcatcacaaaaatcgacgctcaagtcagaggtggcgaaacccgacaggactataaagataccaggcgtttccccctggaagctccctcgtgcgctctcctgttccgaccctgccgcttaccggatacctgtccgcctttctcccttcgggaagcgtggcgctttctcatagctcacgctgtaggtatctcagttcggtgtaggtcgttcgctccaagctgggctgtgtgcacgaaccccccgttcagcccgaccgctgcgccttatccggtaactatcgtcttgagtccaacccggtaagacacgacttatcgccactggcagcagccactggtaacaggattagcagagcgaggtatgtaggcggtgctacagagttcttgaagtggtggcctaactacggctacactagaagaacagtatttggtatctgcgctctgctgaagccagttaccttcggaaaaagagttggtagctcttgatccggcaaacaaaccaccgctggtagcggtggtttttttgtttgcaagcagcagattacgcgcagaaaaaaaggatctcaagaagatcctttgatcttttctacggggtctgacgctcagtggaacgaaaactcacgttaagggattttggtcatgagattatcaaaaaggatcttcacctagatccttttaaattaaaaatgaagttttaaatcaatctaaagtatatatgagtaaacttggtctgacagttaccaatgcttaatcagtgaggcacctatctcagcgatctgtctatttcgttcatccatagttgcctgactccccgtcgtgtagataactacgatacgggagggcttaccatctggccccagtgctgcaatgataccgcgtgacccacgctcaccggctccagatttatcagcaataaaccagccagccggaagggccgagcgcagaagtggtcctgcaactttatccgcctccatccagtctattaattgttgccgggaagctagagtaagtagttcgccagttaatagtttgcgcaacgttgttgccattgctacaggcatcgtggtgtcacgctcgtcgtttggtatggcttcattcagctccggttcccaacgatcaaggcgagttacatgatcccccatgttgtgcaaaaaagcggttagctccttcggtcctccgatcgttgtcagaagtaagttggccgcagtgttatcactcatggttatggcagcactgcataattctcttactgtcatgccatccgtaagatgcttttctgtgactggtgagtactcaaccaagtcattctgagaatagtgtatgcggcgaccgagttgctcttgcccggcgtcaatacgggataataccgcgccacatagcagaactttaaaagtgctcatcattggaaaacgttcttcggggcgaaaactctcaaggatcttaccgctgttgagatccagttcgatgtaacccactcgtgcacccaactgatcttcagcatcttttactttcaccagcgtttctgggtgagcaaaaacaggaaggcaaaatgccgcaaaaaagggaataagggcgacacggaaatgttgaatactcatactcttcctttttcaatattattgaagcatttatcagggttattgtctcatgagcggatacatatttgaatgtatttagaaaaataaacaaataggggttccgcgcatatttccccgaaaagtgccacctgacgtcgacggatcgggagatctcccgatcccctatggtgcactctcagtacaatctgctctgatgccgcatagttaagccagtatctgctccctgcttgtgtgttggaggtcgctgagtagtgcgcgagcaaaatttaagctacaacaaggcaaggcttgaccgagcaaacaaactctttctgtgttgtaaaacgacggccagtcttaagctcgggccccctgggcggttctgataacgagtaatcgttaatccgcaaataacgtaaaaacccgcttcggcgggtttttttatggggggagtttagggaaagagcatttgtcagaatatttaagggcgcctgtcactttgcttgatatatgagaattatttaaccttataaatgagaaaaaagcaacgcactttaaataagatacgttgctttttcgattgatgaacacctataattaaactattcatctattatttatgattttttgtatatacaatatttctagtttgttaaagagaattaagaaaataaatctcgaaaataataaagggaaaatcagtttttgatatcaaaattatacatgtcaacgataatacaaaatataatacaaactataagatgttatcagtatttattatgcatttagaataaattttgtgtcgcccttattcgactcactatagaagttcctattctctagaaagtagaggaacttcacttcattttgctagcgtgtgagggcctatttcccatgattccttcatatttgcatatacgatacaaggctgttagagagataattggaattaatttgactgtaaacacaaagatattagtacaaaatacgtgacgtagaaagtaataatttcttgggtagtttgcagttttaaaattatgttttaaaatggactatcatatgcttaccgtaacttgaaagtatttcgatttcttggctttatatatcttgtggaaaggacgaaacaccgttagctataggctaataagatagttgtgtcaagtgcttcggagacctaacacgtctccagtcacaacggctaaaaatagcca

SEQ ID NO: 183 - DNA, 3364 bp, synthetic construct
  misc_feature 1..3364: note = plasmid including the sequence for B-Gen.1 human albumin target 61
  source 1..3364: mol_type = other DNA
gcacgacttagattatgcatttgtttcttttttgttttcaacaccggtaccgcgttacaatgataagtcgactgaataagtgaactcgagatcagcctcgactgtgccttctagttgccagccatctgttgtttgcccctcccccgtgccttccttgaccctggaaggtgccactcccactgtcctttcctaataaaatgaggaaattgcatccccacttcagaagttcctatactttctagtgaatgagtgagctaactcacattaattgcgttgcgctcactgcccgctttccagtcgggaaacctgtcgtgccagctgcattaatgaatcggccaacgcgcggggagaggcggtttgcgtattgggcgctcttgcgcttcctcgctcactgactcgctgcgctcggtcgttcggctgcggcgagcggtatcagctcactcaaaggcggtaatacggttatccacagaatcaggggataacgcaggaaagaacatgtgagcaaaaggccagcaaaaggccaggaaccgtaaaaaggccgcgttgctggcgtttttccataggctccgcccccctgacgagcatcacaaaaatcgacgctcaagtcagaggtggcgaaacccgacaggactataaagataccaggcgtttccccctggaagctccctcgtgcgctctcctgttccgaccctgccgcttaccggatacctgtccgcctttctcccttcgggaagcgtggcgctttctcatagctcacgctgtaggtatctcagttcggtgtaggtcgttcgctccaagctgggctgtgtgcacgaaccccccgttcagcccgaccgctgcgccttatccggtaactatcgtcttgagtccaacccggtaagacacgacttatcgccactggcagcagccactggtaacaggattagcagagcgaggtatgtaggcggtgctacagagttcttgaagtggtggcctaactacggctacactagaagaacagtatttggtatctgcgctctgctgaagccagttaccttcggaaaaagagttggtagctcttgatccggcaaacaaaccaccgctggtagcggtggtttttttgtttgcaagcagcagattacgcgcagaaaaaaaggatctcaagaagatcctttgatcttttctacggggtctgacgctcagtggaacgaaaactcacgttaagggattttggtcatgagattatcaaaaaggatcttcacctagatccttttaaattaaaaatgaagttttaaatcaatctaaagtatatatgagtaaacttggtctgacagttaccaatgcttaatcagtgaggcacctatctcagcgatctgtctatttcgttcatccatagttgcctgactccccgtcgtgtagataactacgatacgggagggcttaccatctggccccagtgctgcaatgataccgcgtgacccacgctcaccggctccagatttatcagcaataaaccagccagccggaagggccgagcgcagaagtggtcctgcaactttatccgcctccatccagtctattaattgttgccgggaagctagagtaagtagttcgccagttaatagtttgcgcaacgttgttgccattgctacaggcatcgtggtgtcacgctcgtcgtttggtatggcttcattcagctccggttcccaacgatcaaggcgagttacatgatcccccatgttgtgcaaaaaagcggttagctccttcggtcctccgatcgttgtcagaagtaagttggccgcagtgttatcactcatggttatggcagcactgcataattctcttactgtcatgccatccgtaagatgcttttctgtgactggtgagtactcaaccaagtcattctgagaatagtgtatgcggcgaccgagttgctcttgcccggcgtcaatacgggataataccgcgccacatagcagaactttaaaagtgctcatcattggaaaacgttcttcggggcgaaaactctcaaggatcttaccgctgttgagatccagttcgatgtaacccactcgtgcacccaactgatcttcagcatcttttactttcaccagcgtttctgggtgagcaaaaacaggaaggcaaaatgccgcaaaaaagggaataagggcgacacggaaatgttgaatactcatactcttcctttttcaatattattgaagcatttatcagggttattgtctcatgagcggatacatatttgaatgtatttagaaaaataaacaaataggggttccgcgcatatttccccgaaaagtgccacctgacgtcgacggatcgggagatctcccgatcccctatggtgcactctcagtacaatctgctctgatgccgcatagttaagccagtatctgctccctgcttgtgtgttggaggtcgctgagtagtgcgcgagcaaaatttaagctacaacaaggcaaggcttgaccgagcaaacaaactctttctgtgttgtaaaacgacggccagtcttaagctcgggccccctgggcggttctgataacgagtaatcgttaatccgcaaataacgtaaaaacccgcttcggcgggtttttttatggggggagtttagggaaagagcatttgtcagaatatttaagggcgcctgtcactttgcttgatatatgagaattatttaaccttataaatgagaaaaaagcaacgcactttaaataagatacgttgctttttcgattgatgaacacctataattaaactattcatctattatttatgattttttgtatatacaatatttctagtttgttaaagagaattaagaaaataaatctcgaaaataataaagggaaaatcagtttttgatatcaaaattatacatgtcaacgataatacaaaatataatacaaactataagatgttatcagtatttattatgcatttagaataaattttgtgtcgcccttattcgactcactatagaagttcctattctctagaaagtagaggaacttcacttcattttgctagcgtgtgagggcctatttcccatgattccttcatatttgcatatacgatacaaggctgttagagagataattggaattaatttgactgtaaacacaaagatattagtacaaaatacgtgacgtagaaagtaataatttcttgggtagtttgcagttttaaaattatgttttaaaatggactatcatatgcttaccgtaacttgaaagtatttcgatttcttggctttatatatcttgtggaaaggacgaaacaccgttagctataggctaataagatagttgtgtcaagtgcttcggagacctaacacgtctccagtcacaacggctaaaaatagcca

SEQ ID NO: 184 - DNA, 8018 bp, synthetic construct
  misc_feature 1..8018: note = AQ23758_9638_contig_22_79 containing G-Gen.1 CRISPR Cas nuclease
  source 1..8018: mol_type = other DNA
aaagtagaggaacttcacttcattttgctagaccggtaccgcgttacataacttacggtaaatggcccgcctggctgaccgcccaacgacccccgcccattgacgtcaatagtaacgccaatagggactttccattgacgtcaatgggtggagtatttacggtaaactgcccacttggcagtacatcaagtgtatcatatgccaagtacgccccctattgacgtcaatgacggtaaatggcccgcctggcattgtgcccagtacatgaccttatgggactttcctacttggcagtacatctacgtattagtcatcgctattaccatggtcgaggtgagccccacgttctgcttcactctccccatctcccccccctccccacccccaattttgtatttatttattttttaattattttgtgcagcgatgggggcgggggggggggggcgcgcgccaggtggggcggggcggggcgaggggcggggcggggcgaggcggagaggtgcggcggcagccaatcagagcggcgcgctccgaaagtttccttttatggcgaggcggcggcggcggcggccctataaaaagcgaagcgcgcggcgggcgggagtcgctgcgcgctgccttcgccccgtgccccgctccgccgccgcctcgcgccgcccgccccggctctgactgaccgcgttactcccacaggtgagcgggcgggacggcccttctcctccgggctgtaattagctgagcaagaggtaagggtttaagggatggttggttggtggggtattaatgtttaattacctggagcacctgcctgaaatcactttttttcaggttggcaaccgcggacacccaagcggccgccaatgaagaggcctgccgccacaaagaaggccggccaggccaagaagaagaagggtggcggtggtagtggtggcggtggttcaggcggtggcggctcaggctccatgcctattcgctcttttaagctgaaacttgtaacccataacggcgatagtacgtacatggataaactgcgccgcggcctgtggaaaactcatgtgataataaaccgcggcatcgcgtactacatgaacaccttggccctcatgaggcaagaaccctacgggtccaagagccgggaagaagtacggttggatctgctttccactctgagagagcagcaacgccggaacaattggtcagaacaaaccgggactgatgatgaattgctttccctgagccgtcgagtttacgagcttcttgtaccatccgctataggtgaaaagggcgatgcgcaaatgctgagccgcaaatttctctcccctctcgtggacccaaacagtgagggcgggcgcgggaccgccaaaagtgggagaaagccacggtggaagaagatgatggaagaaggacaccccgactgggaaaaggagaaggaaaaggatgcggctaagaaggcagaggatccaacagcatctatattggcggatctcgaggcagtgggactgttgccacttttcccgctgttttctgacgaacagaaagaaatccgctggctccccaagaagaagcgtcagtttgtgaggacatgggaccgggatatgttccaacaggcccttgaacgaatgctgagctgggaaagctggaatcgcagagttgccgaggaatacttgaagctccaggcccagcgggacgaggtgtatgccaaataccttgaggatgctggctcctggcttaatgatctgcagactttcgaaaagcagcgcgaagaggaactggcggaagtaagcttcgaacccaactctgagtacctgattactcgccggcagattcgcgggtggaaggaagtgtatgaaaagtggtcaaagaccagcgaaaatgcgagccaggagcagttgtggcggatggtggctgacgtgcagactgccatggccggcgcgttcggagatcccaaagtgtaccagtttctttctcagcctaagcaccaccatatttggagagagcatccaaatagactgttctactacagcaagtacaacgaggtccgggagaagctcaacagggccaagaagcaggcggcctttaccctgccagatcccgtggagcacccactgtggacacgttttgatgcgcgcggcggcaatatccatgactacgagatatccaaggtgggcaagcaataccacgtgacgttcagctctcttatcctgccagaggcccagagttgggtggagattgagaatgttacagtgggtatcgggaacagcctgcagctgaaacgccagattcgcttggacggttacgcagacaagaagcagaaagtcaaatattatgattattccagcaggttcgagctcacaggagtactcggcggagcaaagatccaattcgataggaagcatcttaagaaggctgctcacagactggctgagggcgaaacagggccgatcttcttgaatgttgtggtggatgtagaaccattcttggaagtgaagaatggacgtttgcggactccactcggtcaagtcctgcaggtgaacactagagattggcccaaggtcgtcgactacaaagcaaaggagctgtcagtcttgatggaaaacacgcaaattggcaacgagaatggggtgtctacaatcgaggccggaatgaggattatgtctattgacctgggacagaggaccgctgctgccgtgtctattttcgaggtcatttctaagaaacctgacgaaaaggaaacgaagctgttttatcccatcgcagacacagatctgtatgccgttcacaggcgaagtctcctgctgagattgcccggcgaggagatctctagtaagaaaatgattgagaagcggaaagagcgcgcacgtatccgctccctggtgaggtatcagatcaggctcctctcagaagtcctgcggcttcacacacagggcaccgctgaacagcgtcggtttaagctggacgagctgctcgtgagcatccagaagaagttggagcttgaccagagcgagtggatttcagaactcgagaaactcttcgactatatcgatgagtcagctgagaaatggaaagaggctctggtcgtggctcacagaactctggagcctatcgtggttgaagccgtcagaaactggaagaagtctctgtccaaagaaaacaaggatagacgcaggattgccggaatctccatctggtctatagaggagctcgaggaaacccgcaagctgcttattgcatggtctaaacactccagagaacctggcattccgaaaagacttgagaaagaggaaacatttgctccagaacacctgcagcacatacagaacgtgaaagacgatcgccttaaacagatggctaacttgtttgtgatgaccgccttgggctataagtatgatgaaggcaataagcggtgggtggaagcgtatccagcatgccaggtaatcctgtttgaggatttgtctagatatcggttcgccctggacagacctaggcgggagaacaatcgattgatgaagtgggcccaccgcagtatcccaaggctcacctacatgcaggctgaactgtttggaatccaggtgggcgatgtctattcagcgtacacctctagattccacgccaaaacaggggcccccgggatccgctgtcatgcactgacagaagccgatcttcaatctaatagttacgttgtgaaccagctgataaaggataaatttattcaagacaaccagactgaaatcctcaaggccggccagatagttccttggcagggcggtgagttgtttgttacctttgcagatagatccggcgccagcttggctgttatccacgccgatattaatgcagcgcagaaccttcagaaaaggttttggcagcacaactcagaggtgttccgagtgccttgtaaggtggtgaagggcgggttggtccctgtttatgaaaagatgcgaaagcttttcggaaaaggcctctttgtaaatatagacgacccagaatccaaggaagtctaccgctgggaacattccactaagatgaaatccaagactacaccagttgaccttgaaagcgaagatattgatcacgaggaactcagcgacgagtgggaagatatgcaggaaggatacaaaacactgctgcgtgacccttcaggcttcttctggtcctcagacagttggatccctcagaaggatttctggatcagagtcaagagcagaatcggcaagtctctgcgggagcagattcgcggtggaagcggaggcagcgggggatcaggtccccctaagaaaaagcggaaggtgggcggtggcggcggttcacatcatcatcaccatcatggcggtgaaggacgcggctcccttctgacctgtggtgacgtggaagagaaccccggccctgaattcatgtctggcggcgaggaactgtttgccggaatcgtgcctgtgctgatcgagctggatggggatgtgcacggccacaagtttagcgtcagaggcgaaggcgaaggggacgccgattacggcaagctggaaatcaagttcatctgcaccaccggaaagctgcccgtgccttggcctacactggtcaccacactgtgctacggcatccagtgcttcgccagatatcccgagcatatgaagatgaacgacttcttcaagagcgccatgcctgagggctacatccaagagcggacaatccagttccaggacgacggcaagtacaagaccaggggcgaagtgaagttcgagggcgacaccctggtcaacagaatcgagctgaagggcaaagacttcaaagaggacggcaacatcctgggccacaagcttgagtacagcttcaacagccacaacgtgtacatcagacccgacaaggccaacaacggcctggaagccaacttcaagacccggcacaacatcgaaggtggcggagtgcagctggccgatcactaccagacaaatgtgcccctcggagatggccccgtgctgatccctatcaaccactacctgagcacccagaccaagatcagcaaggacagaaacgaggcccgggaccacatggtgctgctggaaagctttagcgcctgctgtcacacccacggcatggacgagctgtacagataatgactcgagatcagcctcgactgtgccttctagttgccagccatctgttgtttgcccctcccccgtgccttccttgaccctggaaggtgccactcccactgtcctttcctaataaaatgaggaaattgcatccccacttcagaagttcctatactttctaatgagtgagctaactcacattaattgcgttgcgctcactgcccgctttccagtcgggaaacctgtcgtgccagctgcattaatgaatcggccaacgcgcggggagaggcggtttgcgtattgggcgctcttgcgcttcctcgctcactgactcgctgcgctcggtcgttcggctgcggcgagcggtatcagctcactcaaaggcggtaatacggttatccacagaatcaggggataacgcaggaaagaacatgtgagcaaaaggccagcaaaaggccaggaaccgtaaaaaggccgcgttgctggcgtttttccataggctccgcccccctgacgagcatcacaaaaatcgacgctcaagtcagaggtggcgaaacccgacaggactataaagataccaggcgtttccccctggaagctccctcgtgcgctctcctgttccgaccctgccgcttaccggatacctgtccgcctttctcccttcgggaagcgtggcgctttctcatagctcacgctgtaggtatctcagttcggtgtaggtcgttcgctccaagctgggctgtgtgcacgaaccccccgttcagcccgaccgctgcgccttatccggtaactatcgtcttgagtccaacccggtaagacacgacttatcgccactggcagcagccactggtaacaggattagcagagcgaggtatgtaggcggtgctacagagttcttgaagtggtggcctaactacggctacactagaagaacagtatttggtatctgcgctctgctgaagccagttaccttcggaaaaagagttggtagctcttgatccggcaaacaaaccaccgctggtagcggtggtttttttgtttgcaagcagcagattacgcgcagaaaaaaaggatctcaagaagatcctttgatcttttctacggggtctgacgctcagtggaacgaaaactcacgttaagggattttggtcatgagattatcaaaaaggatcttcacctagatccttttaaattaaaaatgaagttttaaatcaatctaaagtatatatgagtaaacttggtctgacagttaccaatgcttaatcagtgaggcacctatctcagcgatctgtctatttcgttcatccatagttgcctgactccccgtcgtgtagataactacgatacgggagggcttaccatctggccccagtgctgcaatgataccgcgtgacccacgctcaccggctccagatttatcagcaataaaccagccagccggaagggccgagcgcagaagtggtcctgcaactttatccgcctccatccagtctattaattgttgccgggaagctagagtaagtagttcgccagttaatagtttgcgcaacgttgttgccattgctacaggcatcgtggtgtcacgctcgtcgtttggtatggcttcattcagctccggttcccaacgatcaaggcgagttacatgatcccccatgttgtgcaaaaaagcggttagctccttcggtcctccgatcgttgtcagaagtaagttggccgcagtgttatcactcatggttatggcagcactgcataattctcttactgtcatgccatccgtaagatgcttttctgtgactggtgagtactcaaccaagtcattctgagaatagtgtatgcggcgaccgagttgctcttgcccggcgtcaatacgggataataccgcgccacatagcagaactttaaaagtgctcatcattggaaaacgttcttcggggcgaaaactctcaaggatcttaccgctgttgagatccagttcgatgtaacccactcgtgcacccaactgatcttcagcatcttttactttcaccagcgtttctgggtgagcaaaaacaggaaggcaaaatgccgcaaaaaagggaataagggcgacacggaaatgttgaatactcatactcttcctttttcaatattattgaagcatttatcagggttattgtctcatgagcggatacatatttgaatgtatttagaaaaataaacaaataggggttccgcgcatatttccccgaaaagtgccacctgacgtcgacggatcgggagatctcccgatcccctatggtgcactctcagtacaatctgctctgatgccgcatagttaagccagtatctgctccctgcttgtgtgttggaggtcgctgagtagtgcgcgagcaaaatttaagctacaacaaggcaaggcttgaccgaacaaactctttctgtgttgtaaaacgacggccagtcttaagctcgggccccctgggcggttctgataacgagtaatcgttaatccgcaaataacgtaaaaacccgcttcggcgggtttttttatggggggagtttagggaaagagcatttgtcagaatatttaagggcgcctgtcactttgcttgatatatgagaattatttaaccttataaatgagaaaaaagcaacgcactttaaataagatacgttgctttttcgattgatgaacacctataattaaactattcatctattatttatgattttttgtatatacaatatttctagtttgttaaagagaattaagaaaataaatctcgaaaataataaagggaaaatcagtttttgatatcaaaattatacatgtcaacgataatacaaaatataatacaaactataagatgttatcagtatttattatgcatttagaataaattttgtgtcgcccttattcgactcactatagaagttcctattctctag

SEQ ID NO: 185 - protein, 1091 aa, synthetic construct
  REGION 1..1091: note = SEQ ID NO: 2 from WO2022/258753 in which this sequence was named B-Gen.2
MPIRSFKLKLVTHNGDSTYMDKLRRGLWKTHVIINRGIAYYMNTLALMRQEPYGSKSREEVRLDLLSTLREQQRRNNWSEQTGTDDELLSLSRRVYELLVPSAIGEKGDAQMLSRKFLSPLVDPNSEGGRGTAKSGRKPRWKKMMEEGHPDWEKEKEKDAAKKAEDPTASILADLEAVGLLPLFPLFSDEQKEIRWLPKKKRQFVRTWDRDMFQQALERMLSWESWNRRVAEEYLKLQAQRDEVYAKYLEDAGSWLNDLQTFEKQREEELAEVSFEPNSEYLITRRQIRGWKEVYEKWSKTSENASQEQLWRMVADVQTAMAGAFGDPKVYQFLSQPKHHHIWREHPNRLFYYSKYNEVREKLNRAKKQAAFTLPDPVEHPLWTRFDARGGNIHDYEISKVGKQYHVTFSSLILPEAQSWVEIENVTVGIGNSLQLKRQIRLDGYADKKQKVKYYDYSSRFELTGVLGGAKIQFDRKHLKKAAHRLAEGETGPIFLNVVVDVEPFLEVKNGRLRTPLGQVLQVNTRDWPKVVDYKAKELSVLMENTQIGNENGVSTIEAGMRIMSIDLGQRTAAAVSIFEVISKKPDEKETKLFYPIADTDLYAVHRRSLLLRLPGEEISSKKMIEKRKERARIRSLVRYQIRLLSEVLRLHTQGTAEQRRFKLDELLVSIQKKLELDQSEWISELEKLFDYIDESAEKWKEALVVAHRTLEPIVVEAVRNWKKSLSKENKDRRRIAGISIWSIEELEETRKLLIAWSKHSREPGIPKRLEKEETFAPEHLQHIQNVKDDRLKQMANLFVMTALGYKYDEGNKRWVEAYPACQVILFEDLSRYRFALDRPRRENNRLMKWAHRSIPRLTYMQAELFGIQVGDVYSAYTSRFHAKTGAPGIRCHALTEADLQSNSYVVNQLIKDKFIQDNQTEILKAGQIVPWQGGELFVTFADRSGASLAVIHADINAAQNLQKRFWQHNSEVFRVPCKVVKGGLVPVYEKMRKLFGKGLFVNIDDPESKEVYRWEHSTKMKSKTTPVDLESEDIDHEELSDEWEDMQEGYKTLLRDPSGFFWSSDSWIPQKDFWIRVKSRIGKSLREQIR

SEQ ID NO: 186 - protein, 1091 aa, synthetic construct
  REGION 1..1091: note = SEQ ID NO: 39 from WO2022/258753, B-Gen.1-2
MPIRSFKLKLVTHNGDSTYMDKLRRGLWKTHVIINRGIAYYMNTLALMRQEPYGSKSREEVRLDLLSTLREQQRRNNWSEQTGTDDELLSLSRRVYELLVPSAIGEKGDAQMLSRKFLSPLVDPNSEGGRGTAKSGRKPRWKKMMEEGHPDWEKEKEKDAAKKAEDPTASILADLEAVGLLPLFPLFSDEQKEIRWLPKKKRQFVRTWDRDMFQQALERMLSWESWNRRVAEEYQKLQAQRDEVYAKYLEDAGSWLNDLQTFEKQREEELAEVSFEPNSEYLITRRQIRGWKEVYEKWSKTSENASQEQLWRMVADVQTAMAGAFGDPKVYQFLSQPKHHHIWREHPNRLFYYSKYNEVREKLNRAKKQAAFTLPDPVEHPLWTRFDARGGNIHDYEISKVGKQYHVTFSSLILPEAQSWVEIENVTVGIGNSLQLKRQIRLDGYADKKQKVKYYDYSSRFELTGVLGGAKIQFDRKHLKKAAHRLAEGETGPIFLNVVVDVEPFLEVKNGRLRTPLGQVLQVNTRDWPKVVDYKAKELSVLMENTQIGNENGVSTIEAGMRIMSIDLGQRTAAAVSIFEVISKKPDEKETKLFYPIADTDLYAVHRRSLLLRLPGEEISSKKMIEKRKERARIRSLVRYQIRLLSEVLRLHTQGTAEQRRFKLDELLVSIQRKLELDQSEWISELEKLFDYIDESAEKWKEALVVAHRTLEPIVVEAVRNWKKSLSKENKDRRRIAGISIWSIEELEETRKLLIAWSKHSREPGIPKRLEKEETFAPEHLQHIQNVKDDRLKQMANLFVMTALGYKYDEGNKRWVEAYPACQVILFEDLSRYRFALDRPRRENNRLMKWAHRSIPRLTYMQAELFGIQVGDVYSAYTSRFHAKTGAPGIRCHALTEADLQSNSYVVNQLIKDKFIQDNQTEILKAGQIVPWQGGELFVTFADRSGASLAVIHADINAAQNLQKRFWQHNSEVFRVPCKVVKGGLVPVYEKMRKLFGKGLFVNIDDPESKEVYRWEHSTKMKSKTTPVDLESEDIEHEELSDEWEDMQEGYKTLLRDPSGFFWSSDSWIPQKDFWIRVKSRIGKSLREQIR